European Patent Application EP 4 116 316 A1, published January 11, 2023. Title: Antigens useful in active immunotherapy against infection with Pseudomonas aeruginosa. Applicant: Evaxion Biotech ApS. The sequence listing filed with the application follows.

SEQUENCE LISTING (90 sequences)

SEQ ID NO: 1 - protein, 66 aa, Pseudomonas aeruginosa
MSQEPHVHGPNCNHDHDHHHDHGHGHVHGPHCNHSHEPVRNPLKAVGRNDPCPCGSEKKFKKCHGA

SEQ ID NO: 2 - protein, 78 aa, Pseudomonas aeruginosa
MKKTVTLALLLAASLGLAACDKKEEDKAAAPAAPATETQPSAPATPPAEPSAPAPSSDTPATPQTPAPTPEQPQQNQQ

SEQ ID NO: 3 - protein, 104 aa, Pseudomonas aeruginosa
MKKISLASSVVGAALLGVASVGAHAAQNPFAVQELSSGYSVAAAEKAKEGSCGEAKCGADKGKREASKAGHEGSCGADRKAKEGSCGGEKKAGEGNCGADKKKS

SEQ ID NO: 4 - protein, 155 aa, Pseudomonas aeruginosa
MSVFDSRQKTSASLLGAVLVGGMLLGGSAFAVEPLGQGLQVAAASAGEGKCGEGKCGSGGSAKTPAKAGAEGKCGEGKCGDASFARTDTDHDGKVSRAEFLAVAKDRAGEFDSIDSDHDGFISEAEAYEHLRKTYEANGKPMPAGLFSKLEQGQH

SEQ ID NO: 5 - protein, 179 aa, Pseudomonas aeruginosa
MRSLSLLLLLSLASTCEAAAVFRCEDASGHVSFTQLGCPAGQAGETVVADNPPPGGRSVTPMAETKTKKASIGRKSVPLAVIGEREDRCGRRLDEKERRKAIVEQRIMAGMTRSDVERALGKPDRVSGNNAEVRYQYKADKRRGARSVSFDQEGCVKGREGTGWSESIPGAKAGPSSYR

SEQ ID NO: 6 - protein, 304 aa, Pseudomonas aeruginosa
MSQPSENRLITSARYALCLLTASGVLLSGCASSGVGSVAQTTRAEYYPSCYEPVSHLRSTDNAVRNSAITGAITGGLLGGLAGGLASDENRGRNAALAAAGGALAGGAAGYYMEKQKQISDDRARIGSYGTDVDRSTVEINRSVAYAKSAQSCYQSQFKALLDGRKNKSINEAEGRKRLAEIVSGLQETNALLVAANGRAGENISNYTQAYEKDLQQVGVPRAEVTKVAEAENRASTTKGGSKPKTGSNPKVPKEAVATEQTIRKAQDAQSEGNKVASQGQGMIREVCNSPDMGDWAPPSCAKA

SEQ ID NO: 7 - protein, 309 aa, Pseudomonas aeruginosa
MAGKKKSEKESSWIGEIEKYSRQIWLAGLGAYSKVSKDGSKLFETLVKDGEKAEKEAKSDVDAQVGAAKASARSAKSKVDEVRDRALGKWSELEEAFDKRLNSAISRLGVPSRNEVKELHSKVDTLTKQIEKLTGVSVKPAAKAAAKPAAKPAAKPAAKTAAAKPAAKPAAKAAAKPAAKPAAKKTAAKTAAAKPAAKPAAKPTAKAAAKPATKPAAKAAAKPAAKPAAAKPAAKPAAKPAAATAAKPAAKPAAKPAAKKPAAKKPAAKPAAAKPAAPAASSSAPAAPAATPAASAPAANAPATPSSQG

SEQ ID NO: 8 - protein, 340 aa, Pseudomonas aeruginosa
MKATMVLTPLALAMAAVLSVSAYAGNEGGWHPPKPNPQSNNKGGATALVVDTQQNYNNKVSNFGTLNNASVSGSIKDASGNVGVNVAAGDNNQQANAAALASADASFVFGTATASTSVLQSGYGNTLNNYSNPNTASLSNSANNVSGNLGVNVAAGNFNQQKNDLAAAVSNGQYSTAGSAASQTSTGNTTVNSANYAYGGTYVSLKLNADGSYKGTSDQIGDVYLDTWEGQTHPGGSNTGHIDVDSQAQGAKDLNHDGGAFAFKEKGDVDLKGTVSGFIPAIVGFKTPVTNNASLSNSLQNVSGNVGVNIAAGGGNQQSNSLSIAAGCSSCPAGGESLGF

SEQ ID NO: 9 - protein, 347 aa, Pseudomonas aeruginosa
MKQQFERSPSESYFWPVVLAVVLHVLIFAMLFVSWAFAPELPPSKPIVQATLYQLKSKSQATTQTNQKIAGEAKKTASKQYEVEQLEQKKLEQQKLEQQKLEQQQVAAAKAAEQKKADEARKAEAQKAAEAKKADEAKKAAEAKAAEQKKQADIAKKRAEDEAKKKAAEDAKKKAAEDAKKKAAEEAKKKAAAEAAKKKAAVEAAKKKAAAAAAAARKAAEDKKARALAELLSDTTERQQALADEVGSEVTGSLDDLIVNLVSQQWRRPPSARNGMSVEVLIEMLPDGTITNASVSRSSGDKPFDSSAVAAVRNVGRIPEMQQLPRATFDSLYRQRRIIFKPEDLSL

SEQ ID NO: 10 - protein, 352 aa, Pseudomonas aeruginosa
MSANKKPVTTPLHLLQQLSHSLVEHLEGACKQALVDSEKLLAKLEKQRGKAQEKLHKARTKLQDAAKAGKTKAQAKARETISDLEEALDTLKARQADTRTYIVGLKRDVQESLKLAQGVGKVKEAAGKALESRKAKPATKPAAKAAAKPAVKTVAAKPAAKPAAKPAAKPAAKPAAKTAAAKPAAKPTAKPAAKPAAKPAAKTAAAKPAAKPAAKPVAKPAAKPAAKTAAAKPAAKPAAKPVAKPTAKPAAKTAAAKPAAKPAAKPAAKPAAKPVAKSAAAKPAAKPAAKPAAKPAAKPAAKPVAAKPAATKPATAPAAKPAATPSAPAAASSAASATPAAGSNGAAPTSAS

SEQ ID NO: 11 - protein, 420 aa, Pseudomonas aeruginosa
MWGLTMKFASLILMLLFATVARAEDYYWKIQSLPERFSSPSAACAAWAKATGRPGEFTFTGSMKARDQTSFWCEFTNNETGKTAAGYGPAGRYGDSCPEGTEYDKATGVCKSPPQECKEGELFPAKGPDSPVVTSGGRNYVGDGGAPTACYQSCEYGGNPSPASCYLVKGSTTTGFCNYILKGTGQNCGADSYTFSQTGDSLNPPDTPNTDPSDPNDPGCPPGWSWSGTTCVKAPTDPTDPTDPTTPGSDGGGDGNGGGNNNGGGNDGGTGNGGDGSGGGDGNGGGDGSGDGDGSGTGGDGNGTCDPAKENCSTGPEGPGGELKEPTPGTWDDAIATWEKKVEDAKQELKTKVKANVDQMKGAFDLNLAEGGGQLPCESMTIWGKSYSLCISDYAGQLSSLRVALLLMAALIAALILLKD

SEQ ID NO: 12 - protein, 427 aa, Pseudomonas aeruginosa
MAVAPGVLLPPTPDVKPKAAAPKSQQKTPEPSNDKTSSFSDMYAKETAKKPAERADGPAKGSRDKPRDAGKDAAEAQPTDAVRQPAVAEDGKPLPADGQAKADGEDKVETPVDPLQLLGLGGAVPLLDENTQATLLPPAVPTASSAPASLTEASSDPTLVKLNGVPAVNMALEQGAQDAAQTAKGGPAKSADPRQANLGDALAGLTSDSLTKAVDGKALEAQLQQTAEPAVASAASESLLESKAEPRGEPFAAKLNGLTQAMAQQALTNRPVNGTVPGQPVAMQQNGWSEAVVDRVMWMSSQNLKSAEIQLDPAELGRLDVRIHMTADQTQVTFASPNAGVRDALESQMHRLRDMFSQQGMNQLDVNVSDQSLARGWQGQQQGEGGSARGRGLAGEASGDEETLAGVSEIRSRPGASAARGLVDYYA

SEQ ID NO: 13 - protein, 428 aa, Pseudomonas aeruginosa
MLRLLPLLLSLACLAPAFADERADTQRQLEQTQKDIGELKKLLDGIQQEKSGVQKQLKSTETEMGDLEKQIKALQDELDKSEAELKRLDGEKKKLQDARIEQQRLLAIQARAAYQSGREEYLKLLLNQEHPEKFSRTLTYYDYINKARLEQLASFNETLRQLANVEQDISAQKAEQLSKQGELDSRREALAATRKERQQALAKLNSDYRERDQKLKSRQQDQAELAKVLRTIEETLARQAREAAAAAERERQRALAAERERARQQQAAPGRVTSPPREPAPGPLVSSTGAVYGGAFGSARGKLPWPVNGRVVARFGSQRGDDPRAKWDGVLISASAGSTVRAVHGGRVVFADWLRGAGLLVILDHGGGYLSLYGHNQSLLKDAGDTVKAGDPIATVGTSGGQSSPAVYFAIRHQGRPADPTTWCRAQG

SEQ ID NO: 14 - protein, 568 aa, Pseudomonas aeruginosa
MQRLSRIGRNTLAVSVSTLLLSACNQGDDAPKPAAVAPQPAAPSMAALSIPLCLNGQCAVIDQDAKLLVPFDNDYDNIVASAYQGTLMAAREERWNLIQAKDGKVLRDDIGEALSLLTPNLYGFVRDGKYGVVDGQGKEVQAPRFDDIYPNSANEFIIYEIDGKRGILDAKGKQLTEALYDTTLVNGSVAEHGGLISAERGEEKWIINLATGEQKAVAYESLGDLHDGVMSASVIGKGSQLVDAKGDVVGDGKSYDYLGTPANGLVAFREKYDSPCGYLDYQGKVAIAAQFAGCGAFGKQGGLAQQRMEDGSSGKYGLIDRSGAWKVQPQYDSADSAGLTALGYTVDVPGLAAVGVSTGLFSADFGIFNLDEGSEWVKPGYAQIGALGNDLFVVAKKGGPQKTVSFMGSESQVPVVGLMDRSGKMLLEPDELISIQSAYDGRFLEGLDGMDNAAHTVLLDRQGRTLVPALWQKLEVNPQQGYILGYEVSGTGDEATETLRALYDLNGKPRFTVATTDCGAEQLLDGNGKAIWPQDPTPYCQSDDEQDDEGEPEQEPAPVEESEETSES

SEQ ID NO: 15 - protein, 579 aa, Pseudomonas aeruginosa
MLRPARSLSLCSALVILLAACGEGEPLLPADARLPDGARYRGELVDGRLEGQGRLDYDNGAWYAGRFEHGLLHGHGTWQGADGSRYSGGFAAGLFDGQGRLAMADGSVYQGGFRQGLFDGEGSLEQQGTRYRGGFRKGLYSGQGTLDGSDGSRYQGSFRQGRLEGEGSFSDSQGNQYAGTFRDGQLNGKGRWSGPDGDRYVGQFKDNQFHGQGRYESASGDVWIGRFSEGALNGPGELLGADGSRYRGGFQFWRFHGQGLLEQLDGTRYEGGFAAGAYAGQGTLDRADGSREQGLWADGKRIRDAAGKALPDTLEVGLLAQGRLLDEELRKIPASTPASELYALSLGGDGRQGVFLREADYAGDLLGQRFAARGVIRLVNHRDHFGDRPLATRESLSRAVRTLAERSGPEDLVFIYLTSHGSSDHQLALDMPGLNLGDLPAAELAELLAPLRQRDKVLVVSACYSGGFIPPLKDERTLILTAARADRVSFGCSDDADFTYFGRALLANALNRTDDLSKAFELAKEEVRQREKEEGFEASEPQAWLPERVLAHWRTLRGQQAERALASREGKTGEGAAGK

SEQ ID NO: 16 - protein, 621 aa, Pseudomonas aeruginosa
MLQNIRDNSQGWIAKTIIGVIIVLLSLTGFDAIIRATDHSNVAAKVNGDDISLNEVQQAVDMQRRQLLQRLGKDFDPSMLDDKLLKEAALKGLIERTLLLQAAKDDKFAFSDQALDQLILQTPEFQVDGKFNADRFDQVIRQMNYSRMQFRQMLGQEMLIGQLRAGLAGTGFVTDNELQSFARLEKQTRDFATLAIKADASKSSVSDDEVKAFYEGHKSEFMTPEQVVVEYVELKKSSFFDQVKVKQEDLEALYQKEIANLSEQRDAAHILIEVNDKVGDEQAKAKIDEIKARLAKGEDFAALAKEFSQDIGSAATGGDLGYAGRGVYDPAFEEALYALKQGEVSAPVKTPYGYHLIKLLGVQAPEVPSLESLKPKLEDELKKQMVEQRFVEATKDLESSAYEAADLSQPAQEMGLKVQTSQPFGRSGGDGIAANRQIVQTAFSAEVLEEAANSGAIELDPDTVVVLRVKEHNKPKEQPLEQVAANIRERLAAEKAAEEAQKRGEALIAELREGRTSSAAGESWKVVEAASRGHEGVDPKLLQAVFRMQRPEAKDKPSFSGVTLANGDYVVIRLNGVSEPEEAISDDEKAMYRRFLASRSGQADFAAFRRQLQDKAEVEKY

SEQ ID NO: 17 - protein, 688 aa, Pseudomonas aeruginosa
MDMTSLMPLLLGVGLVVLLVVGLLALFKAFYIKVPQGTALIVNDMSSTPKVHFTGALVYPVIHLKEFMRISLITLEVDRRGKDGLICRDNMRADITVAFYLRVNETQDDVLKVAKAIGVDRASDRSAVNELFNAKFSEALKTVGKQFDFVQLFENRQDFRDRIIEVIGNDLNGYVLEDVAIDYLEQTAKNSLDPSNILDAEGIRKITELTATQNVITNELERNEELAIKKKNVETREAALALERQQADAEARQKREIETIRAREEAETARVKEEERLKAEQARIQAQQEIDVRTENHQREVEVAQQNRQRAVVIEVEKVTRAKDLEIVAREREVELQKIEKEKALEEQRKNIANVIRERVAVEKTVAQEEERIKEVREVSEAERVKQVILLQAQAEAEQELVRQVKQAEADEARSKHKAVEINTMAQAELEAASKQAEAKKRLAEGIEAERAAPGLADARVLEVTAAAKEKDGLAAARVRAEQLIAEARGDEERGLADARVLEAQAAAKEKDGLAEAKVLAEKLGAQARGEEQLGAAKAKATKDQGSAEAEVLLQRLNAEAEGLGKKFGALDALSDSARQHEEFRMQLEKSFEEAMAAIAANKDIAKDQAEVLATALGKANIEIVGGEGDFFNSFAKSLSVGKAIEGVVGKSPVVQDVLARLLNGRGAAAAVMPERKSGHENEPAAEV

SEQ ID NO: 18 - protein, 742 aa, Pseudomonas aeruginosa
MYPQFRRGHLAAAVLFASSSLLGGQALAEDERLEELDERAESVVQLGDEVVLGTAEQELKQAPGVSIITAEDIRKRPPVNDLSEIIRTMPGVNLTGNSSSGQRGNNRQIDIRGMGPENTLILVDGKPVSSRNSVRYGWRGERDTRGDSNWVPPEEVERIEVLRGPAAARYGSGAAGGVVNIITKRPTDRLRGSMTVFTNIPESSKDGATRRANFSLSGPLTEALSFRAYGSANKTDSDDTDINLGHTVNPSRTVAGREGVRNRDLSGMLSWQVTPDQVVDFEAGFSRQGNIYAGDTQNNNGTANTQGLADDGAETNRMYRENYAITHNGTWSFGTSRFVAQYDSTRNNRLEEGLAGSVEGQIGADRSFSASKLENYRLSGELNLPLHALFEQVLTVGAEWNKETLNDPSSLKQGFVGSDSLPGTPAAGSRSPKSKAEIRALYVEDNIELRPGTMLTPGLRLDDHSDFGLNWSPSLNASQTLGEYFTVKAGIARAFKAPNLYQSNPNYLLYTRGNGCPIQTSSGGCYLVGNENLDAETSVNKELGIEFRRDGWVAGLTYFRNDYKNKIVAPLDVMGQTGTGNNILQWSNAKKAVVEGLEGNLLVPLHEDLSWSTNLTYMLQSKDKDTGNPLSVIPEYTLNSTLDWQASERLSTQLTSTIYGRQEPPKHGTSRNTPVVSRKEVGTYGIWGVSAGYTFSENLSVRGGVSNLFDKRLYRQGNSFDAGAATYNEPGRAYYVSMTTSF

SEQ ID NO: 19 - protein, 746 aa, Pseudomonas aeruginosa
MSSRALPAVPFLLLSSCLLANAVHAAGQGDGSVIELGEQTVVATAQEETKQAPGVSIITAEDIAKRPPSNDLSQIIRTMPGVNLTGNSSSGQRGNNRQIDIRGMGPENTLILVDGKPVSSRNSVRYGWRGERDSRGDTNWVPADQVERIEVIRGPAAARYGNGAAGGVVNIITKQAGAETHGNLSVYSNFPQHKAEGASERMSFGLNGPLTENLSYRVYGNIAKTDSDDWDINAGHESNRTGKQAGTLPAGREGVRNKDIDGLLSWRLTPEQTLEFEAGFSRQGNIYTGDTQNTNSNNYVKQMLGHETNRMYRETYSVTHRGEWDFGSSLAYLQYEKTRNSRINEGLAGGTEGIFDPNNAGFYTATLRDLTAHGEVNLPLHLGYEQTLTLGSEWTEQKLDDPSSNTQNTEEGGSIPGLAGKNRSSSSSARIFSLFAEDNIELMPGTMLTPGLRWDHHDIVGDNWSPSLNLSHALTERVTLKAGIARAYKAPNLYQLNPDYLLYSRGQGCYGQSTSCYLRGNDGLKAETSVNKELGIEYSHDGLVAGLTYFRNDYKNKIESGLSPVDHASGGKGDYANAAIYQWENVPKAVVEGLEGTLTLPLADGLKWSNNLTYMLQSKNKETGDVLSVTPRYTLNSMLDWQATDDLSLQATVTWYGKQKPKKYDYHGDRVTGSANDQLSPYAIAGLGGTYRLSKNLSLGAGVDNLFDKRLFRAGNAQGVVGIDGAGAATYNEPGRTFYTSLTASF

SEQ ID NO: 20 - protein, 784 aa, Pseudomonas aeruginosa
MSPSRALSPLSRALLLACLGGPVLVSAGSACAAEIRTDARQYYRLPAEPLEQALNHLGRQAGVLIAFSPEQTAARRSQALDGEYTLEEALAALLVGSGLEARARGDGAYTLEALPVEDPANLQALTVVGDWLADASAADVFEHPGARDVVRREQFQAQGAASTREVLERIPGVSAPLNNGTGSHDLALNFGIRGLNPRLASRSTVLMDGIPVPFAPYGQPQLSLAPVSIGNMDAVDVVRGGGAVRYGPQNVGGIVNFVTRAIPEDFATKLDVHSELSPSSSQDGLKTTHNVLIGGTGANGLGGALLYSGTRGGDWREHSDTRIDDLILKGRFQPSDEHTFSAMTQYYDGEADMPGGLGTAAYHDDPYQSTRPYDKFWGRRTLASASYEYTPNASQKLNVTGFFTKTLRSGYLDQGRNLTLSPREYWVRGLETRFSQGFELGESRHEVGIGHRYVNEASHELRYWTRADSGQLPSTGSRNDRDTRGSTEANAFYIDDRIDIGNWTITPGIRYEKIDSEQKNLLKNSKDSGRYNASLPALNVIYHLTPSWNLYANTEGSFGTVQYSQMGKAVRSGDIEPEKARTWELGSRYDDGILRAELGAFLINFDNQYESNQQTDSVTARGKTRHKGIEAAIAYDLADLDPLLSGFDVYASYAYVDASIREDGPNKGNQVPFSSKHKGTLGANYRTGAWSYNLDGSFQTSQYADNANTESESADGSTGRIAGWMVWSARGTYDFGPQLNDLKLGLGVKNLFDRRYYTRSFDDNNKGLYVGQPRTLYVQASVGF

SEQ ID NO: 21 - protein, 851 aa, Pseudomonas aeruginosa
MTLPFTRAAWRPLCSAAVLGAALWAAGASAAERRFDLPAQPLAASLSRLAQQAQVQVLFDESLLRGLRAPALSGSYGVREALERLLVGSELELVEAGGGYVVRRRQVDAYSDNALQLDAQTIVGNGREVDASNVGRSTLTRRDIERQQADNIPSLLQTLPGVTMGGSPKPGGQTTNIWGLGDAEDVPYTLDGAQKSGFERYQQGTVFIEPEMIKRIEVEKGPHSVFTGNGGFGGTVHMETKDAPDLLREGRDVGAMLKYGYHSNDQQKIYSGAVFGRSEDRRVDALLYLNGRDGRDMKLADNLPLSPTDYPINPKRLPNSAQDEKTGLFKLNLHPTEEHDLGFTYLRSKSSRWTPFSASSYPTPPSQWTIDRYGYELGLTRLLAHRDTTDTTWTGKYNYHPLDNPWIDLQLSYSDARTEQLDRREDTAFYQLATGGKRMRTEYQDKVLELRNTSRFDTGALQHELTLGAALHKHKRDILMHMPGKTYETPRYNYGWLQPAFMPAGKQDTQSFYIQDAITYGSLTVTPSMRFDSVRNDGQANLAPIYDNPKLGHDYRAQTYSGWSPRLSVFWTATPNLAFFADYTETWRAPVIDEQYEVQNSSTIGGSSRDLDAERIHAIRGGSVINLPDLLVAGDSLQIRTTLFQNRIKDEIFRTRSVGCRQQSIDNGSIGGSCGDMLPLSNYRNLPGLTIKGFEIESFYDSQRLFGSLSYSWMTGKHDGAYSNPWGPNVWARDIPPPKWVAMLGLKVPEWDAKLGWQGEFVRKTDRLPSDRYSGGMGTGSGDIYWDHAANDSYDTHRLFAEWVPAKLGLKDTRIDFTVDNLFNRSYRQPLGGDLVYSQGRNAKISVTQFF

SEQ ID NO: 22 - protein, 880 aa, Pseudomonas aeruginosa
MHRSLHTDAPLGAALLLALQLAPGSAAAAEEQAPVDPPTVQLQRIEVTGSAIRRVDAETAVPISVLRAEELRQQGVTSTEELIGRLSGNQGVYNSSRSVGSATGGASFADLRGIGANKTLVLLNGRRLANNAIDGSAVDLNTIPFAAIDRVEVLRDGASALYGTDAIGGVINFITRKSLNEGRFDSGYASPTHDGGGNQRNVSASWGFGELEEDRFNVFAVANYDKQERLGAKDRGYTYNYQPGRGLDYSSGTAFPGNWSQGANASNPLAAGGCKGADLIPRNGICRQSLWRYLDLVPETEKTSVFSRATGKLADEHNVSLEYFWSRSDNATQVGPGTLTGLQIDPGTAFYPGNGITPGPGGFVLDPSRPVEVNWRQSVLGPRLQSSQNTGQRLLLGFDGQFAGWDYDIGASYNQNKVVDHIHSGYVDDRAAALGIANGTLNPFGPQTDAGLAYLGSHALSGDFRTSVGRVKGLDARASREIGDWFGAGPAALALGGEFRKEAFHQDIQDFAGNVQSLGVDPAATVSGERNLKAQYAELNVPVLDSLELSAAIRHDKYSDFGSTSNPKYSFRFQPFRQLVLRGAYSEGFRAPSLYELYNPTFTTYTSANYDDPRLCAGGQPSQGGIANRDCAQQFYNATGGNTDLRPETARNVTLGLVYQPLRDLSVGLDFWWIRIANQIAEFPEAAIFADPQAYAGRIVRKADGSIDHVVTGLANLGKVKTSGVDLSLDYRFPASRYGQFGLDLQGTYVSRYDFQQQIGGQYLDNVGDFQGVGVIARWKHVANATWSRDAWQATLSNRYTSGYNDYDRASHGKVGSWNLWDLAGSYRLSHALGLTLGVKNLFDREPPFSNQTYTFQSGYDPRYTDPYGRILFGRLSYSF

SEQ ID NO: 23 - protein, 919 aa, Pseudomonas aeruginosa
MVRLRTLVRAIAAASVLTSGMAHGLGLGEITLKSALNQPLDAEIELLEVRDLGSGEVIPSLASPEEFSKAGVDRLYYLTDLKFTPVVKPNGKSVIRVTSSKPVQEPYLNFLVQVLWPNGRLLREYTVLLDPPLYSPQAAASAPQAPVSAPRATGAPRAPQAPAPVRTTAPAGSDTYRTVSNDTLWEIAQRNRTDRVSVPQAMLAFQELNPGAFVDGNINRLKSGQVLRIPTEQQMLERSPREALSQVQAQNQSWRGSRNPAAGSAGARQLDATQRNAAGSAPSKVDATDNLRLVSGEGKASKGADKGGKGDSKAIADTLAVTKESLDSTRRENEELQSRMQDLQSQLDKLQKLIQLKDAQLAKLQGQLGAEGQGAAQPNAALPDASQPNAAAQAPAQPGTPAAAAPTPAPAGEAPAAPAQPPVAPPPAPAAEKPPAPAVPAPAPVQAAEQPAPSFLDELLANPLWLAVIGGSALLALLVLLMILSRRNAQKEKEEAQAFAADTGEEQEDALDLGKDGFDDLTLDEPEPQVAAVAPQVEKTTAQTSDALGEADIYIAYGRFNQAAELLQNAIYDEPQRTDLRLKLMEVYAEMGDREGFARQENELREIGGAQPQVEQLKSRYPAMVAVAAVAGLAGAKLAQDELDSFSLDDLSLDDSGHAAKPDAAGQDLDDAFDLSLDDLGGDDVQADLKSDSGALDDLTLDSDLDLAASTPADKPVDDLDFGLDFAELAETPSQPKHDDLGDFSLDLDAPEDKLSDDDFLLSLNDEVPAAAPADNEFTLDTEAAEEPALSLPDDFDLSLADEPTEPAAPEKGEDSFAAQLDEVSAQLDELASNLDEPKSATPSFSAEDAAVASALDGDADDDFDFLSGADEAATKLDLARAYIDMGDSEGARDILDEVLAEGNDSQQAEARELLERLA

SEQ ID NO: 24 - protein, 995 aa, Pseudomonas aeruginosa
MTDDHSFRPRPTSLSAALLLGAWIAQPATAAYVEAGRPGDPASWRSAEYQQDWGLERMRADQAYAAGIDGQGVKIGEMDSGFDPSHPDTPASRYQPVTASGTYVDGTPFSVSGAMNGNNDSHGTHVGGTLGASRDGVGMHGVAYAAQVYVANTNQNDSFLFGPTPDPNYFKAAYQALADAGVRAINNSWGSQPKDVSYETLDGLHAAYAQHYGRSTWLDAAAGVSRQGVINVFSAGNSGYANASVRSALPYFQPDLEGHWLAVSGLDQQNGQRYNRCGIAKYWCITTPGRLINSTMPGGGYANKSGTSMAAPHATGALALVMQRYPYLNNEQALQVLLTTATQLDGTPTGAPTDTVGWGVPDLGRAMHGPGQLLGRFEANLPAGLRDEWSNPISDSALLQRQAEDAAEHAAWQRTLKDKGWENGLPAGASQQERTDYAIGMARDQAAAQRQYQGSLVKAGAGSLVLSGDSTYRGPTLVDGGLLSVDGSLLSAVEVNAGGTLGGSGRIGGLLARSGGTVAAGNSIGTLEVAGDLRFESGSTYAVELSESASDRIVASGKASIAGGNVTLAMENSPDLLSQSQVESLVGRRYDILDAAGGIDGRFDAVLPNYLFLGGTLDYAANAIRLDIGRNGTTLASVAQTPNQAAVAGAVETLGAGNPVYESLLLSENAATAQRAFQQLSGEIYPALAGLLLNDSRYLRDSVGERLRQTSDGEAGGEAPEGWFKALGSWGKSADGSHGSEGYRHSVGGFLLGVDSQVASDTRLGLVAGYSNSSLNMDSSLQSSASIDSYHLGAYLGRQLQQWRLSLGAAHAWHRAEVKRDLQYGAVAGKQKAKLDAQSSQLFAEAAYALGWRSLELEPFAGLAYVHVASDDFRERGSAAALEGGDDNLDAAFTTLGLRAKRHFELDAGRRLALSGTLGWRHNLSDTTPQRHLAFASGSQPFSVESVALSRDAALLGVDASLAVNREVSVRLGYNGLLGSREKDHGVGLAVDWRF

SEQ ID NO: 25 - protein, 1057 aa, Pseudomonas aeruginosa
MKRMLINATQPEELRVALVDGQRLFDLDIESGAREQKKANIYKGRITRVEPSLEAAFVDFGAERHGFLPLKEISREYFKKSPEGRINIKEVLSEGQEVIVQVEKEERGNKGAALTTFISLAGRYLVLMPNNPRAGGISRRIEGEERNELREALNGLNAPADMGLIVRTAGLGRSTEELQWDLDYLLQLWSAIKEASGERGAPFLIYQESNVIIRAIRDYLRQDIGEVLIDSIDAQEEALNFIRQVMPQYASKVKLYQDSVPLFNRFQIESQIETAFQREVKLPSGGSIVIDPTEALVSIDINSARATKGGDIEETALQTNLEAAEEIARQLRLRDIGGLIVIDFIDMTPAKNQRAVEERVREALEADRARVQVGRISRFGLLEMSRQRLRPSLGETSGIVCPRCNGQGIIRDVESLSLAILRLIEEEALKDRTAEVRARVPFQVAAFLLNEKRNAITKIELRTRARIFILPDDHLETPHFEVQRLRDDSPELVAGQTSYEMATVEHEEAQPVSSTRTLVRQEAAVKTVAPQQPAPQHTEAPVEPAKPMPEPSLFQGLVKSLVGLFAGKDQPAAKPAETSKPAAERQTRQDERRNGRQQNRRRDGRDGNRRDEERKPREERAERQPREERAERPNREERSERRREERAERPAREERQPREGREERAERTPREERQPREGREGREERSERRREERAERPAREERQPREGREERAERPAREERQPREDRQARDAAALEAEALPNDESLEQDEQDDTDGERPRRRSRGQRRRSNRRERQREVSGELEGSEATDNAAAPLNTVAAAAAAGIAVASEAVEANVEQAPATTSEAASETTASDETDASTSEAVETQGADSEANTGETADIEAPVTVSVVRDEADQSTLLVAQATEEAPFASESVESREDAESAVQPATEAAEEVAAPVPVEVAAPSEPAATEEPTPAIAAVPANATGRALNDPREKRRLQREAERLAREAAAAAEAAAQAAPAVEEIPAVASEEASAQEEPAAPQAEEITQADVPSQADEAQEAVQAEPEASGEGAADTEHAKKTEESETSRPHA

SEQ ID NO: 26 - protein, 1161 aa, Pseudomonas aeruginosa
MKSVLHQIGKTSLAAALSGAVLLSAQTTHAAALSVSQQPLMLIQGVAPNMLVTLDDSGSMAFAYAPDSISGYGNYTFFASNSFNPMYFDPNTQYKLPKKLTLVNGQVQIQDYPAPNFSSAWRNGFTRSGSINLSNSYKVTIEYGRGYDKESTIKADAAYYYDFTGSSSCNRTNQACYTRRYVSTEQRQNFANWYSFYRTRALATQTAANLAFYSLPENARVSWQLLNDSNCNQMGSGSSSGNCFSNYLRDFTGQHRVNFFNWLEKLSVNGGTPLRQAMTRAGEFLKKTGVNGPYAYRPGTQTAPEYSCRGSYHILMTDGLWNNDSANVGNADSTARNLPDGKSYSSQTPYRDGTFDTLADQAFHYWATDARPDIDDNIKPYIPYPDQANPSAEYWNPRNDPATWQHMVTYTLGLGLTTSLTSPRWEGSTFSGGYNDIVAGNLSWPRASNNDSNNVYDLWHAAVNSRGEFFSADSPDQLVAAFQDILNRISGKDLPASRPAISSSLQEDDTGDKLTRFAYQTSFASDKNWAGDLTRYSLTTQDKATVQTKLWSAQSILDAMPNGGAGRKIMMAGSGTSGLKEFTWGSLSADQQRQLNRDPDRNDVADTKGQDRVAFLRGDRRKENSDNFRTRNSILGDIINSSPATVGKAQYLTYLAQPIEPSGNYSTFAEAQKTRAPRVYVGANDGMLHGFDTDGNETFAFIPSAVFEKLHKLTARGYQGGAHQFYVDGSPVVADAFFGGAWHTVLIGSLRAGGKGLFALDVTDPANIKLLWEIGVDQEPDLGYSFPKPTVARLHNGKWAVVTGNGYSSLNDKAALLIIDLETGAITRKLEVTGRTGVPNGLSSPRLADNNSDGVADYAYAGDLQGNLWRFDLIAGKVNQDDPFSRANDGPAVASSFRVSFGGQPLYSAVDSAGAAQAITAAPSLVRHPTRKGYIVIFGTGKYFENADARADTSRAQTLYGIWDQQTKGEAAGSTPRLTRGNLQQQTLDLQADSTFASTARTIRIASQNPVNWLNNDGSTKQSGWYLDFMVNGTLKGEMLIEDMIAIGQVVLLQTITPNDDPCADGASNWTYGLDPYTGGRTSFTVFDLARQGVVDSKSDYSYNKQNVAVSGTEQKGLGGLTLSTNEQGNPEVCSSGECLTVNPGPNTRGRQNWRPIEGKN

SEQ ID NO: 27 - protein, 1211 aa, Pseudomonas aeruginosa
MKILAIRLKNLASLAGEQEIDFTREPLSSAGLFAITGPTGAGKSTVLDALCLALFGSTPRLESTSASSKVPDGRNELSSNDERNLLRRGCASGYAEVDFVGIDGHRYRARWETRRSRDKADGALQKSQQSLQDLETQQMLAANKKSEFREQLEQKLGLNFAQFTRAVLLAQSEFSAFLKASDNDRGALLEKLTDTGLYSQLSKAAYQRASQADEQRKQLEQRLEGSLPLAEQARAGLEAALESHAQARLQEQQALQRLEGQQQWFTEEQRLLQSCEHAQGQLAEARQAWDALATERETLQWLERLAPVRGLIERLKQLEQELRHSEQQQRQRTEQQAAGTERLQGLQARLQEARERQAQADNHLRQAQAPLREAFQLESEARRLERTLAERQELHRQSNQRHAQQSDAARQLDMEQQRHVAEQAQLQAALRDSQALAALGDAWVTHQGQLATFVQRRQRALESQAQLPELEKSLAHAGEPLERLQAQWTALHGSEPDDLAARLVELRRQTDSLERQQALHKEWQQVLDQRAGLARRLGELDQRMVEQEQALLDLKRQGSQCAEEVKAAEQALQVTRELLQRQRLARSASVEQLRAGLVDGEACPVCGSQEHPYHHSEQLLAALGEHDDQEQVRAEQSLERLRQTLVGLREGYSSQRERLNQSRQEQQELTGQLAALDRQLDQWTLPEELRLLQPSAQLEWLAQRLDDLAGQRQQCQRDFDRLIARQRQTQQLQQELRAAETILQQRQQALTEQRQRYEHLQQQVEEDSQQLRPLLSDEHWQRWQADPLRTFQALGESIEQRRQQQARLQQIEQRLQELKQRCDESSWQLKQSDEQRNEARQAEERAQAELAELNGRLGAHLGQHACAQDWQLSLEHAAQAAQSAVETLQAPLDSLREEQLRLAEALEHLQQQRQRQQDEFQRLQADWQAWRERQDNLDDSRLDALLGLSEEQATQWREQLQRLQEEITRQQTLEAERQAQLLQHRRQRPETDREALEDNLRQQRERLAASEQAYLETYSQLQADNQRREQSQALLAELERARAEFRRWGRLNELIGSSSGDKFRRIAQGYNLDLLVQHSNVQLRQLARRYRLQRGGSELGLLVVDTEMGDELRSVYSLSGGETFLISLALALGLASMASSKLRIESLFIDEGFGSLDPESLQLAMDALDNLQAQGRKVAVISHVQEMHERIPVQVRVQREGNGMSSLKVVG

SEQ ID NO: 28 - protein, 2468 aa, Pseudomonas aeruginosa
MSIQAKVTPIDQSISSAAAVEVPENGILKLSQSSNVALDVAPESVAGYSKSGSDLIVQLKTGESVRIANFYAEGQPSSQLFLADKDKLVAVDLPPVAADGPLMAGYIPQESLAGFESLTGAGVLGGMSAGTALLVGAAAIGAGVAISNSSGGGGGGGSSVPPDTTPPKAASGLKIAPDGSSISGQAEAGASVGIDTNGDGKPDLTVIADANGNFTAPLNPPLTNGQTVTVVVTDPAGNASPPAQVTAPDTTAPAPATDVQVAPDGSSVTGKAEPGSTVGVDTDGDGQPDTTVVVGPGGSFEVPLNPPLTNGETVTVIVTDPAGNNSTPVTVEAPDTTAPAPATDVQVAPDGSSVTGNAEPGATVGVDTDGDGQPDTTVVVGPGGSFEVPLNPPLTNGETVTVIVTDPAGNSSTPVTAEAPDFPDAPQVNASNGSVLSGTAEAGVTIVITDGNGNPIGQTSADANGNWSFTPGSQLPDGTVVNVVARDAAGNSSPATSITVDGVAPNAPVVEPSNGSELSGTAEPGSSVTLTDGNGNPIGQTTADANGNWSFTPSTPLPDGTVVNVVARDAAGNSSPPASVTVDAVAPATPTVDPSNGTTLSGTAEPGSSVTLTDGNGNPIGQVTADGSGNWTFTPSTPLPNGTVVNATATDPSGNASSPASVTVDAVAPATPVVNPSNGTTLSGTAEPGATVTLTDGNGNPIGQVTADGSGNWSFTPTTPLPNGTVVNATATDASGNTSAGSSVTVDSVAPATPVINPSNGTTLSGTAEPGSSVTLTDGNGNPIGQVTADGSGNWSFTPSTPLADGTVVNATATDPAGNTSGQGSTTVDGVAPTTPTVNLSNGSSLSGTAEPGSTVILTDGNGNPIAEVTADGSGNWTYTPSTPIANGTVVNVVAQDAAGNSSPGASVTVDSQAPAAPVVNPSNGTTLSGTAEPGATVTLTDGNGNPIGQVTADGSGNWSFTPGTPLANGTVVNATASDPTGNTSAPASTTVDSVAPAAPVVNPSNGAEISGTAEPGATVTLTDGSGNPIGQVTADGSGNWSFTPSTPLADGTVVNATATDPAGNTGGQGSTTVDAIAPATPTVNLSNGSSLSGTAEPGSTVILTDGNGNPIAEVTADGSGNWTYTPSTPIANGTVVNVVAQDASGNSSPPATVTVDSSAPPAPVINPSNGVVISGTAEAGATVTLTDAGGNPIGQVTADGSGNWSFTPGTPLANGTVIVATATDPTGNTGPQAATTVDAVAPPAPVIDPSNGTTISGTAEAGAKVILTDGNGNPIGETTADGSGNWSFTPGTPLANGTVVNAVAQDPAGNTGPQGSTTVDAVAPNTPVVNPSNGNLLNGTAEPGSTVTLTDGNGNPIGQTTADGSGNWSFTPGSQLPNGTVVNVTASDAAGNTSLPATTTVDSSLPSIPQVDPSNGSVISGTADAGNTIIITDGNGNPIGQVTADGSGNWSFTPGIPLPDGTVVNVVARSPSNVDSAPAVITVDGVAPAAPVIDPSNGTEISGTAEAGATVILTDGGGNPIGQATADGSGNWTFTPSTPLANGTVINAVAQDPAGNTSGPASVTVDAIAPPAPVINPSNGVVISGTAEAGATVILTDGNGNPIGQVTADGSGNWSFTPGTPLANGSVINALAQDAAGNNSSPTSATVDSLAPAAPVIDPSNGSVIAGTAEAGATVILTDGNGNPIGQVTADGSGNWSFTPGTPLSNGTVVNAVAQDAAGNTSGPVSTTVDAVAPATPVIDPSNGVELSGTAEPGVRVILTDGNGNPIGQTLADGSGNWSFTPGTPLANGTVVNAVAQDPAGNTSGPASTTVDTVAPATPVINPSNGSVITGTAEVGAKVILTDGNGNPIGETTADGSGNWTFTPGTPLANGTVINAVAEDAAGNASGPASTTVDSVAPSAPLLSISADGALLTGTAEPNSQVRIVVNGDTANPITVTVDGAGNFSLPFAPPLITGELIAGVAVDAAGNVSGPATINAPDLAPPTISVPEAADTWINAAEIGDGIQVDVTVRPTMQVGQVVTVKFAGQNGYEAEVSHTLTAGDIAAGNLTLTLTPPGGMGPFPEGASTVTADINGGTASTPVPFTIDTIPPATPVLSLVGNILTISAEPGTELTVTVDVGGVTATATVTADNSGLASLNLLTDLDIDFSWDQLLNAQVSVVGRDPAGNPSNTASIGVGTSIEQPVTIGNFGLDVSLNPLNPRFGFSGTTEPDSSVVIRVITPALNVELLPIQADSSGNFSLNLLSPTILTQLGLNITDILNLGSQISFNLVSTDSNGNDSAAYGITLTPNGLSLNIGQIDVNGTSGDDVLSGANGSSEHINGGDGSDLIFNVGTGDHVVAGNGNDTIQITATDFVSIDGGAGFDTLVLANGIDLDYNAVGVGTLSNLERIDLGKGDSGSVLTLTAAEVDAITDANNTLQITGENNDTLNVVGAVNTGTTQLINGITYDVYTFGSTTLLIEDNTVQVVV

SEQ ID NO: 29 - protein, 3535 aa, Pseudomonas aeruginosa
MDIRSPLNQCIALSLAGILFLNPIVAAAAGLALDKAAGGNTGLGQAGNGVPIVNIATPNDAGLSNNHFRDYNVGANGLILNNATGKTQGTQLGGIILGNPNLKGQAAQVILNQVTGGNRSTLAGYTEVAGQSARVIVANPHGITCQGCGFINTPRATLTTGKPIMDGQRLERFQVDGGDIVVEGAELNVGNLEQFDLITRSAKLNAKLYAKNLNIVTGRNDVQADSLQATPRAADGSEKPQLAIDSSALGGMYAGAIRLVGTEQGVGVRLAGDMAASGGDIRIDASGKLSLAQASSQGDLKIAAQAVELNGKTYAGGSAEIRSAEELVNRQSLAARERIVLEAAHIDNAGVIEAGVEPDERRNARGDLELRSGTLRNAGSLVASRALEAKASQALDNQGGSLKGATVRVDAGHLDNRGGKLLAEGELRVEASSLDNRQDGLLQSRDRAVVKTRGDLDNRGGQVIGLNDLEVGAATLDNGQQGLLGSQQSTRVSAQALVNRGDGEVSGKRVEARVGSLDNRGGKLIGDDLLVVASGAIDNRLGLFSAANRLDLRARSLDNSGKGTLSSRGGLEVSLGGLLDNRDEGNLLSQGAQRVTVGQLDNRAGGLLSSRSELNVHGASLDNRGGVLVADAGLSATGGAFDNRDGGSASGKAGVRVEVASLRNDQGGKLLSDGRLDLAANAVGNAGGRIAAKGDLQATLGSLAQQGGELVSEKTLKVAADTLDNSQSGLIAANGGIAIEARQVDNRAGEISSTSKVAVNAREQLDNRGGKVIGDSGLRLTVQRLLNQAKGVLAGRDGLSLDGGELFNGDGGRLDSQNSLSVSLGGVLDNQGGALVSEGSLTARAARLDNRGGTFSSAGALALTSQAALDNQGGRLLSDAGVTLQGASLDNSRSGVISAKGAVDIRTGVLDNSRNGGIGSNAGITLVAARLDNGQQGRVSAKGLLDANLKGLDQRGGGVLISETGVTLDLNGGTLVNRDGGLIATPGALLLRQLGAVDNGAGGEISSDRAFTLAAASLDNRGGRLIGAANLTLRIAQALDNSLAGVISGAAGLDIAAARLDNSAKGTLASRAGIDLRVDGALDNHAEGTVSGARLTLASASLDNSGKGLLSGNAGLSVATGALDNAEGGQLISQGVLDVSSADLDNRGGALSGKQSLRLSAANLDNRGGLLTSDGELELTAGRVDSADGGEISARGDLRLTVERLVQRQGRLVGERGVSLDLRGGDLDNQGGLISARGPLSIERLSVLDNRQGGEISSQQGFELLARRIDNGQQGRIISAGKLRLDADALGNAGAGLLSGWQGLTVTGGSLDNSAGGTLSSKDGELAISLGGALDNHGQGALVSKGAQRIDAASLDNAQGIVSGESDVTLSIAGKLDNGQGGLVSAQRALSFERDDTLLNNAGGRINGGSLLLKGASLDNSDGQLISQGRLDAILGGALVNTGAARLASGGDLLLRSASVDNRGGKLVSQGLLEISAGSLDNSASGTLASQAGMSLRLGGGALRNQQDGLIFSQAGALDVQAGSLDNRQGTLQAQGDNRLRIGGALDNQGGRLDSRAGNLDLQSGSLDNGAGGVLNSAKGWLKLVTGLFDNSAGVTQAQSLEIRAGQGVRNQQGHLSALGGDNRIVTADFDNQGGGLYASGLLSLDGQRFLNQGAAAGQGGKVGAGRIDFSLAGALANRFGQLESESELHLRAAAIDNSGGSLRALGRSGSTRLVAGGLNNAYGVLESANQDLDLQLGSLANAGGRILHTGNGTFGLDSGQVIRAGGELTTNGLLDIRASEWTNSSVLQAGRLNLDIGTFRQTAEGKLLAVQSFTGRGGDWSNDGLLASDGSFRLDLSGGYRGNGRATSLGDFALNAASLDLGNAASLAGGANVTLGAGNLLVNRGRITAAGDLVASAASLNNYGTLGGGGNLRLNAPALLNERGLLFSGADMTLRAGDITNLYGDVYSLGRLDIARDDAGNRAASLRNLSGVIESGKDFSLRASLIENRRAVLESKSGLYTAKMEQTACIEGVNAGDCSGKRNAIWTITQRDKTEVTASSAMGQLLAGGDFAIDGGTLNNLSSLIGSGGNLTANLEVLDNQGLETGELETIRVLRTARGGDIGGIDQKSRNFTNLYWYQSANFDPARAGEIPAALNAILSDWSFEYEFPSKGPTPISSGDQSYAAVIQAAGDVTVNASTRIDNGVTRPGYTFVGSGRQVGDSAVGGSGVSVVVPLTSQLPPDLARRQVNPVTLPGFSLPQGDNGLFRLSSRFAEDGNGSAALGAGADRTQGGSGVSVGQQGAGNAAGTWQGQGVRVDGLAGAANVQGQGGSTLGGSLPGVARVQGVPGNATPSASHKYLIETNPALTELKQFLNSDYLLSGLGMNPDDSKKRLGDGLYEQRLIRDAVVARTGQRYIDGLSSDEALFRYLMDNAIAYKDQLHLQLGVGLSAEQMAALTHDIVWLEEVEVNGEKVLAPVVYLAQAEGRLAPNGALIQGRDVKLVSGGDLHNVGTLRARNDLSATADNLDNSGLIEAGKRLDLLAGDSIRNRQGGVIAGRDVSLTALTGDVINERSVTRYDSALDGRTWERSFADSAARVEAANSLNVQAGRDIANLGGVLQSRGDLSLDAGRDVTVAAVEDRQGQTRWSTSRLQSVTQLGAEVSAGRDLNVSAGRDLTAVASTLEARRDIALSAGRDVTLAAAANEEHAYSKTRKVTYQEDKVAQQGTRVDAGGDLAINAGQDLRLIASQASAGDEAYLVAGDKLELLAANDSNYYLYDKKKKGDFGRKETRRDEVTDVKAVGSQISSGGDLTLLSGGDQTYQGAKLESGNDLAIVSGGAVTFEAVKDLHQESHEKSKGDLAWNSAKGKGQTDETLRQTQIVAQGNLAIKAVEGLKIDLKHIDQKTVSQTIDAMVQADPQLAWLKEAEQRGDVDWRMVQEVHDSWKYSNSGMGPATQIAVAIAAAAIGGMAAAGALSGAGVGASSFAMGAGVGAAGSLSGTAAVSLINNKGDLGKVLKDSFSSDSLKQIAIASLTGGLTAEYFDGILQTKTDPLTGKVTVDLSSLSGVGRFAANQAMQNATSTVLSQALGQGGSLNEALKSALYNSFAAAGFNFVGDIGQEYSLKPGDPSMVTMHALMGGLAAQVSGGDFATGAAAAGANEALVAKLDQAFKSLSPENREAMVTMGSQLVGVLAAAVRDPDVTGKALESAAWVAKNSTQYNFLNHQDVADLDNALQKCKSQGNCRQVEEEFKARSDENRRRLNGCVAVGNCAEIRAEIDAGSTALNELVARQETANPGGSDSDIAYGFLMGRNVVDWTTAGQLHLEQTANLWWNGNPQWQKEVGAYLDQTGFNPFGIGVPAMGGAAGKVTAKALMNALKAGELPKGEVAPGKANLPTIGALADAEAGMPYTHPVKLAAKATGTAGKIKIEAGAIPDANEVRAGQGLSGLGYDVTHQTTASAKGIQGQRTADLHVDGLGSIDVYTPKNLDPTKIVRAIEKKSNQAGGVLVQADLPSTDMSSIAARMWGKTNAQSIKTIFFQKPDGSLVRFDRPAGGG

SEQ ID NO: 30 - protein, 5627 aa, Pseudomonas aeruginosa
MDIRSPLNQCIALSLAGILFLNPIVAAAAGLALDKAAGGNTGLGQAGNGVPIVNIATPNGAGLSNNHFRDYNVGANGLILNNATGKTQGTQLGGIILGNPNLKGQAAQVILNQVTGGNRSTLAGYTEVAGQSARVIVANPHGITCQGCGFINTPRATLTTGKPIMDGQRLERFQVDGGDIVVEGAELNVGNLEQFDLITRSAKLNAKLYAKNLNIVTGRNDVQADSLQATPRAADGSEKPQLAIDSSALGGMYAGAIRLVGTEQGVGVKLAGDMAASGGDIRIDASGKLSLAQASSQGDLKIAAQAVELNGKTYAGGSAEIRSAEELVNRQSLAARERIALEAAHIDNAGVIEAGVEPDERRNARGDLELRSGTLRNAGSLVASRALEAKASQALDNQGGSLKGATVRVDGGHLDNRGGKLLAEGELRVEASSLDNRQDGLLQSRDRAVVKTRGDLDNRGGQVVGLNELQVQAAALDNRSAGLLSSKGDMDIEFARLDNSAGGKLVSERRTLLKADRLDNRSGRIVAGQDLDLSSRLIDNRAGDISSTSRVVASAREQLDNRGGKIVGDSGLDITTPRMLNQDKGVLASRDGLRLSATELFNGAGGLLSSQKGIDVSLAGAFDNQAGSLDSRGFLTVKSAWLDNQGGTLSSAGALAVTSQGALNNQGGRLASDAGLSLSSASLDNSQAGAISGKGAVEIRTGNLNNSRKASIGSDAGLTLVAARVDNSQAGRIAAKGVIDADLQGLDQHDRGNLVSDTGITLDLNKGSLVNRAQGLIATPGTLLLRQLGVVDNSGGEISSDRAFTLATSALNNQGGRLLSGGALTLRIAQALDNSLEGIVSGAGGLDIQAFVLDNRSGSIGSKGAIDIGVTRLENDAGTLIAERGLKLVADEANSSKGRIAANGSLHAKVGTLSQKGGELTSQDSLTLDLGILNNNAGRIAGNQGVDITARQVDNSVGEIASQGVVALNLTEQLDNRGGKIVGDSGLGITAPHVLNQDKGVLASRDGLRLSATELFNGAGGLLSSQKGIDVSLAGAFDNQAGSLDSRGFLTVKSAWLDNQGGTLSSAGALAVTSQGALNNQGGRLASDAGLSLSSASLDNSQAGAISGKGAVEIRTGNLNNSRKASIGSDAGLTLVAARVDNSQAGRIAAKGAIDAALQGLDQHDRGSLVSDTGITLDLNKGSLVNRAQGLIATPGTLLLRQLGVVDNSGGEISSDRAFTLATSALNNQGGRLLSGGALTLRIAQALDNSLEGIVSGAGGLDIQAFVLDNRSGSIGSKGAIDIGVTRLENDAGTLIAERGLKLAADEANNSKGRIVAKDELRAKLGALVQNGGELTTQGALALDADKVDNGAGRIAGNRGVVIDARQVDNRAGEIASQGVATLNLTEQLDNRGGKVVADSGLGITAPRVLNQDKGVIASRDGLRLSGTELFNGNAGLLSSQRHIEVTLDGVLDNQGKGALLSDGTLTVSAGRIHNQDATLSSAGALRLSSQEAVDNRGGKLVTDSSLRLTSASLDNSRSGIISANAAAEIHTGVLNNSQKGNLGSNDGLGLIATEVDNSQEGRITAKGMIDANIKGLDQQGKGRLVSNAGIILDLNEGTLANGAQGLIATPGTLLLRQLGMVDNSGGEISSDRAFTLTTSALTNQGGRLRSGGVLTLRIAQALDNSLEGVLSGTGGLDIRALALDNRSGSIGSKGAVDIDVSRLENDDGDLLSEGRLKLTAERANSVRGRIAARGDLHASVTAFNQAGGELSSEGALMLEADSLDNRSGGLVSADGNLTVSARRIDNRAGEIASPGQVTLDVAEQLDNRGGKAIGDSGLRLAAPRVLNQDGGVLASRDGLRLNGAELFNGNGGLLSSQQSIDVILDGVLGNQAGSLSSQGRLSVKSGRLDNQGGAVSSAGTLSLSSQGALNNQGGRVVTDAGAVLRSASLDNSQGGIVSAKGAAEIRTGSLNNSQKGGIGSGAGLALVADLVDNSQNGRITAKGAIDANLKGLDQQGSGRLVSDTAIALDLRGGELVNRAQGLIATPGALLLRQLGVVDNSGGGEISSDRSFTLAATALSNRGGRVISGDSLTLRIAQALDNSLQGVLSASGGLDVAALVFDNHSGIVASKGDTHIGVNRLENEAGRVVSEGALDLTAKQVSSAKGRIAAKGDLQVTVGTLEQQGGELASQGTLTLDADSLDNRNGGLVSADGGVTAEARQIDNRGGEISSVAKVALAVREQLDNRGGKVIGDSELSLTVQRLLNQAKGVLASRDGLHLDGAELLNGDGGLLSSQRLVDVTLSGALDNQGSGALVSEESLTVKADQVNNQAGTFSSAGSLLVTSRGELNNQGGRLVTDAGATLNSTGFDNSRAGLVSAKGAVAIRTGALNNSQKGSIGGNTGVTLVAGLVDNGREGRISTKGTLDANLKGLLQQGGGSLVGERGVTLDLNGGTLDNHDLGLVSTPGALLLRQLGMVDNSVGGEISSDRAFTLAANTLNNQGGRLISSEALTLRIAKTLDNSLKGQVLATDGLAIESQVLDNRAGTIGSKGDARISVTSLDNAEQGSLVSEGRLELVADQVSNGNQGRIAARGVLEAAVGTLLQQGGELVSQGSLDLRADTLDNSQSGLIAANGGIAIEARQVDNRAGEISSTSKVAVNAREQLDNRGGKVIGDSGLRLTVQRLLNQAKGVLAGRDGLSLDGGELFNGDGGRLDSQNSLSVSLGGVLDNQGGALVSEGSLTARAARLDNRGGTFSSAGALALTSQAVLDNQGGRLLSDAGVTLKGASLDNSRSGVISAKGAVDIRTGVLDNSRNGGIGSNAGITLVAARLDNGQQGRVSAKGLLDANLKGLDQRGGGVLVSETGVTLDLNGGTLVNRDGGLIATPGALLLRQLGAVDNGAGGEISSDRAFTLAAASLDNRGGRLIGADSLTLRIAQALDNSLAGVISGAAGLDIAAARLDNSAKGTLASRAGIDLRVDGALDNHAEGTVSGARLTLASASLDNSGKGLLSGNAGLSVATGALDNAEGGQLISQGVLDVSSADLDNRGGALSGKQSLRLSAANLDNRGGLLTSDGELELTAGRVDSADGGEISARGDLRLTVERLVQRQGRLIGERGVSLDLRGGDLDNQGGLISARGPLSIERLNVLDNRQGGEIYSQQGFELLARRIDNGQQGRIISAGKLRLDADALGNAGAGLLSGWQGLTVTGGSLDNSAGGTLSSKDGELAISLGGALDNHGQGALVSKGAQRIDAASLDNAQGIVSGESDVTLSIAGKLDNGQGGLVSAQRALSFERDDTLLNNAGGRINGGSLLLKGASLDNSDGQLISQGRLDAILGGALVNAGAARLASGGDLLLRSASVDNRGGKLVSQGLLEISAGSLDNSASGTLASQADMSLRLGGGALRNQQDGLIFSQAGALEVQAGSLDNRQGTLQAQGDNRLRIGGALDNQAGRLDSRAGNLDLQSGSLDNGAGGVLNSAKGWLKLVTGLFDNSAGVTQAQSLEIRAGQGVRNQQGHLSALGGDNRIVTADFDNQGGGLYASGLLSLDGQRFLNQGAAAGQGGKVGAGRIDFSLAGALANRFGQLESESELHLRAAAIDNSGGSLRALGRSGSTRLVAGDLNNAYGVLESANQDLDLQLGSLANAGGRILHTGNGTFGLDSGQVIRAGGELTTNGLLDIRASEWTNSSVLQAGRLNLDIGTFRQTAEGKLLAVQSFTGRGGDWSNDGLLASNGSLRLELSGGYRGNGRATSLGDFALNAASLDLGNAASLAGGANVTLGAGNLLVNRGRITAAGDLVASAASLNNYGTLGGGGNLRLNAPALLNERGLLFSGADMTLRAGDITNLYGDVYSLGRLDIARDDAGGWANRLENISGNLESTGDMRFSVSSLLNRRETLEIEGDLQNSAIGVRCTGCQLSERWGKTRSSSELVWIREYKSTLGDSSAAASITAGRDLLVVGASLQNIASNISAVRDATLSLSNFENKGYALGEYAVRGVYSPPSKFGEELLMRILAYNAVNDPSYGEGYASTGGRLPNIHYFDKNFNEKVSPLEVIHGNGKNGGPGWHLYFGTLDVEYPDTDRWNKAIGRIPAPNYSSKKTDAIPDLLKGLAPLDELTINKGANSTVGAVVQAGGRVTVNAAESFNNSVLQGFQAVQETQLPHQDIAVSSTTSAVVTLKSQLPADLARQQINPLTLPGFSLPQGQNGLFRLASQGAQVNQASGALKSASDLTQSGHGVSVSAQTGSGASGWSTQARRVGDDRVTSLAGSAYQGRVAEAIDALRASAPISGDGGNTGRFQAGEHQATTGLGGLVEGNASGHSGNGVILADLRGGLPSFSSLPASDHVQGTVPGHDGNGTILANWQGAQATVQASPSTVRVEGVVSSPGGNGSILADLPAEQSSVQALPSAVRAQGSLPRLEERSALLAEPPVGQPALQTLPSVARVEGVPSNATPSNSHKYLIETNPALTELKQFLNSDYLLGGLGINPDDSKKRLGDGLYEQRLVREAIVQRTGQRFIAGLNSDEAMFRYLMDNAIASKDVLGLTPGVTLSAAQVAALTHDIVWLEEVEVNGEKVLAPVVYLAQAEGRLGPNGALIQGRDVNLITGGDLRNAGTLRAQNDLSATAGNIDNSGLIEAGNRLDLLASGSIRNDQGGIIAGREVSLSALTGDVINERTVTQHQSSYRGTGTTEAFADSAARIEAAQKLTVSAGRDVANIGGVIDSKGDLALQGGRDVLVSAAVAERGWTAGSQAYQTQTTQMGAEVVAGRDISVSAGRDISVVGSRIDARRDVTFEAGRDVGLVAAANEEHAYGKTKKVTFQDDKITQQATRVDAGGDLAINAGQDLRLVASQASAGDEAYLVAGDKLELLAANDSSYYLYDKKSKGSFGSKKTRRDEITDVTAVGSQISSGGDLTLLSGGDQTYQGAKLESGNDLAIVSGGAVTFEAVKDLHQESHEKSKGDLAWQSSKGKGQTDETVRQSQIVAQGNLAIKAVEGLKIDLKHIDQKTVSQTIDAMVQADPQLAWLKQMEQRGDVDWRRVQELHDSWKYSNSGLGVGAQLAIAIVVAYFTAGAASAALGSMAGVGAGSGSMMAAAGSTAMVQAGTAVGTAAAGWANAAGTAVAMGMASNGAISTINNRGNLGDVVKDVTSSDALRGYVVAGTTAGLTAGVYDKWTSTQTGTSTALPNTGAVAPAAGLGTWQGVGQFTSNQLLQNGTSVLLDRALGGKGSLGDALQNSLANAFAAYGFKLIGDTTHGVLDDGSLGKIGLHALMGGLAAEAVGGDFRTGALAAGVNEALVDSLAKQYASLPIDDKKGLLIMSSQLIGVLAASTQGDADAKSLQTGAWVAGNATQHNYLSHWQEEKKRQEVDGCKDKQLCKTGIEAKWAIISAQQDVGIVVGVGGGIGLSTAETAVGVYELVKNWRETYAALEQLATSPEFRQQFGDNYLKGLEERAAFLTQAYEDAGWQGSVTAGVEGGRFAAELVGVLTAVKGGAQITAKLPTAAKNLVNAIAESPVSGSMSSQLGAVGDLGRLGGGGKGYVDILSHEAKQHILYGDKPGSGGHLWPGQAGKTVFPQNWSADKIVHEVGDIATSPSTKWYAQTGTGGVYTSKGDPAKWVAYEVRDGVRMRVVYQPATGKVITAFPDNAPIPPYKPIK

SEQ ID NO: 31 - DNA, 201 bp, Pseudomonas aeruginosa
atgagtcaggaaccccacgtacacggcccgaactgcaaccacgaccacgatcatcatcacgatcatggccatggtcatgtccatggtccgcactgcaaccacagccacgagccggtgcgcaatccgctcaaggccgtaggccgcaacgatccctgcccctgcggcagcgagaagaaattcaagaagtgccacggcgcctga

SEQ ID NO: 32 - DNA, 237 bp, Pseudomonas aeruginosa
atgaaaaagaccgtaactcttgccctgctgctcgctgccagccttggcctggccgcttgcgacaagaaagaggaagacaaggcagcggccccggcagctccggctaccgagacccagccgagcgctccggctactccccctgccgagcccagcgccccggcgccgtcgagcgacactccggcaaccccgcagactccggcaccgactccggagcaaccgcaacagaaccagcaataa

SEQ ID NO: 33 - DNA, 315 bp, Pseudomonas aeruginosa
atgaaaaagatttccctcgcttcttccgtcgtcggcgctgctctgctcggcgtagccagtgtcggcgcgcatgccgcgcagaatcccttcgccgtgcaggagctgagcagcggctacagcgtggctgccgccgagaaagccaaggaaggttcctgcggcgaggccaagtgcggtgccgacaagggcaagcgcgaagcctccaaggccggtcatgaaggcagctgcggtgcggatcgcaaggccaaggaaggttcctgcggtggcgagaagaaggccggcgaaggcaactgcggcgccgacaagaagaagtcgtaa

SEQ ID NO: 34 - DNA, 468 bp, Pseudomonas aeruginosa
atgtccgttttcgattcgcgtcaaaagacttccgccagcctgctcggtgccgtactggtggggggaatgctgctcggcggttcggcgttcgccgtcgagccgctgggccaggggctgcaagtggcggcggcgagcgccggcgaaggcaagtgcggagaaggcaagtgtggtagcggcggctccgcgaagaccccggccaaggccggcgccgagggcaagtgcggggagggcaagtgcggcgacgcctcctttgcccgaaccgacaccgatcacgatggcaaggtctcgcgcgccgagttcctcgcggtggccaaggaccgtgccggtgagttcgacagcatcgatagcgaccatgacggcttcatttccgaagccgaggcctacgaacacctgcgcaagacctacgaggccaacggcaagccgatgcccgccgggctgttcagcaagctggagcaaggccagcactga

SEQ ID NO: 35 - DNA, 540 bp, Pseudomonas aeruginosa
atgcgttccctgtccctccttctcctcctctcgctggcgtccacctgcgaggccgctgcggtattccgctgcgaagacgccagcggccatgtcagcttcacccaactcggttgccccgccgggcaggccggcgagaccgtcgtggcggacaacccgccgccgggaggcaggagcgtcacgccgatggccgagacgaagacgaaaaaggcgtccatcggccggaaaagcgtgccgctcgcggtgatcggagaaagagaagatcgctgcggcagacgcctggacgagaaggaacgccgcaaggcgatcgtggagcagcggataatggcgggaatgacccgctccgatgtggagcgggcgctgggcaagccggaccgggtcagcgggaacaatgcggaggtgcgttatcagtacaaggccgacaagcgacggggagcgagaagcgtgagcttcgatcaggagggatgtgtgaagggaagagaaggtaccgggtggagcgagtcgatcccgggagctaaggccgggccgtcctcataccgatga

SEQ ID NO: 36 - DNA, 915 bp, Pseudomonas aeruginosa
atgagccaacccagcgaaaaccgtttgatcacctcggcgcgctacgcgctctgcctgttgaccgccagcggcgtgctgctcagcggctgcgccagcagcggcgtcggctcggtcgcccagaccacccgcgcggaatactacccgtcctgctacgagccggtgtcgcacctgcgcagcaccgataacgcagtgcgcaattcggccatcaccggcgccattaccggcggcctcctgggcggcctggccggcggcctggccagcgacgagaaccgcggccgcaatgccgccctcgctgccgcaggcggcgccctggccggcggcgcggcgggctactacatggagaagcagaagcagatcagcgatgaccgcgcgcgcatcggctcctacggtaccgacgtcgaccgcagcaccgtcgagatcaaccgtagcgtggcctacgccaagtcggcgcaaagctgctaccagagccagttcaaggctctgctcgacggtcgcaagaacaagtcgatcaacgaagccgaagggcgcaagcgcctggccgagatcgtcagcggcctgcaggagaccaacgccttgctggtcgccgccaacggccgtgccggcgagaacatcagcaactacacccaggcctacgagaaagacctgcagcaggtcggcgtaccgcgcgccgaggtgaccaaggtcgccgaggccgagaaccgcgccagcactacgaaaggcggcagcaagcccaagaccggcagcaatcccaaggtgccgaaggaagcggtcgccaccgagcagaccatccgcaaggcccaggacgcgcaaagcgaaggcaacaaggtggcctcccagggccagggcatgatccgggaagtctgcaacagcccggacatgggcgactgggcgccgccgagctgcgccaaggcctga

SEQ ID NO: 37 - DNA, 930 bp, Pseudomonas aeruginosa
atggctggcaagaagaagagcgaaaaagagtccagttggatcggcgagatcgagaaatactcgcggcagatctggctggctggtctgggggcctactcgaaggtcagcaaggacggcagcaagctgttcgagaccttggtgaaagacggcgagaaggctgaaaaagaagcgaagtccgatgtggacgcgcaggtcggtgcggcgaaggcttccgcccgctctgcgaagagcaaggtcgacgaggttcgggaccgtgcgctcggcaagtggagcgagctcgaggaagctttcgacaagcgcctgaacagcgccatctcgcgtctcggcgtgccgagccgcaacgaggtgaaggagctgcacagcaaggtcgatacgctgaccaagcagatcgagaaactcaccggcgtcagcgtcaagccggcggcgaaggcagcggccaagcctgcggcgaaaccggctgccaagcccgcggcgaaaaccgcagcggccaagccggcagctaaaccggcagccaaggccgccgccaagcctgcggcgaaacccgcggcgaaaaaaaccgcggcgaaaaccgcggccgccaagccggcagccaagcccgccgccaaaccgactgcgaaggccgcagcgaaaccggcgaccaagccggcagccaaggccgcggcgaagcctgctgcgaaacctgccgcagccaagcctgccgcgaagccggcagccaagccggccgctgcgaccgccgccaagcccgcggcgaaacctgccgccaagccggctgcgaaaaagcctgcggcgaagaagccggcagccaagcccgccgcggcgaaaccggccgctcccgccgcgtcttcgagcgcgcccgctgcccccgccgccacaccggctgccagcgctccggcagcgaacgctccggcgacgccgagcagccagggctga

SEQ ID NO: 38 - DNA, 1023 bp, Pseudomonas aeruginosa
atgaaagcgactatggtcctgaccccgctggccctggcaatggctgcagtgctgtcggtatcggcctacgccggaaacgaaggtggctggcacccgccgaaacccaacccgcagtcgaacaacaagggcggagccacggccctggtggtggatacgcagcagaactacaacaacaaggtcagcaacttcggcacgctgaacaatgcctcggtgagcggctcgatcaaggatgcctcgggcaacgtcggggtcaacgtcgccgccggcgacaacaaccagcaggccaacgccgccgcgctggccagcgccgacgccagcttcgtgttcggcaccgcgaccgccagcaccagcgtgctgcagagcggctacggcaatacgctgaacaactactccaaccccaacaccgcatcgctgagcaactcggccaacaacgtctcgggcaacctgggcgtgaacgtcgccgccggcaacttcaaccagcagaagaacgacctggccgccgccgtctccaacggccagtacagcactgccggtagcgccgcgtcgcagacctccaccggcaacaccaccgtcaacagcgccaactacgcctatggcggcacctacgtgtcgctgaagctgaacgccgacggcagctacaagggcacctccgaccagatcggcgacgtctacctcgacacctgggaaggccagacccatccgggcggcagcaataccggccacatcgacgtggacagccaggcccagggcgccaaggacctgaaccacgacggcggcgcgttcgccttcaaggaaaagggcgacgtcgacctgaaaggcacggtgtccggcttcatcccggcgatcgtcggcttcaagaccccggtcaccaacaacgccagcctgagcaactcgttgcagaacgtctcgggcaacgtcggggtgaacatcgccgccggtggcggcaaccagcagagcaactccctgtccatcgccgccggttgcagcagctgcccggccggtggcgagagccttggcttctga

SEQ ID NO: 39 - DNA, 1044 bp, Pseudomonas aeruginosa
atgaagcaacagttcgaacgctcgccttccgagagttatttctggcccgtcgtcctggcggtggtcctgcacgttctgatcttcgccatgctgttcgtcagctgggcgtttgctccggagcttcctccctccaagccgatcgtgcaggccacgctctaccagctcaagtcgaagagccaggcgacgacacagaccaaccagaagatcgctggcgaggcgaagaagaccgcctccaagcaatacgaagtcgagcagctcgaacagaagaagctcgagcagcagaaactcgagcaacaaaagctggaacagcagcaggtcgctgctgcgaaagcggcggaacaaaagaaggctgacgaggctcgaaaggccgaggcccagaaagccgccgaggcgaaaaaggccgatgaagccaagaaagctgccgaggccaaggccgccgaacagaagaagcaggctgacatagccaagaagcgcgccgaggacgaggccaagaaaaaggccgctgaggacgccaagaaaaaggcagccgaggacgcgaagaagaaagcggccgaggaggccaagaagaaggctgctgcggaagcggcgaagaagaaagccgccgtcgaggccgccaagaaaaaggccgccgccgctgccgcggcagcccgcaaggctgccgaggacaagaaggcgcgggcattggccgagttgctttcggatacgaccgagcgccagcaggccctggccgacgaggtgggcagcgaggtcaccggcagtctcgacgacctgatcgtcaacctggtgagccagcagtggcggcgtcctccatcggcgcgtaatggaatgagcgtagaagtactgatcgaaatgctgccggacggtaccatcaccaatgccagcgtcagccgttcgagtggcgacaagcctttcgacagttcggcggtggcggcggtgcgcaacgtcggccgtattcccgagatgcagcaattgccgcgggctaccttcgacagcctgtatcgtcagcgccgcatcatctttaaaccggaggatttgagtctgtga

SEQ ID NO: 40 - DNA, 1059 bp, Pseudomonas aeruginosa
atgtcggccaacaagaagcccgtcaccacccccttgcacctgttgcagcaactttcccacagccttgtcgagcacctggaaggtgcgtgcaaacaagcgctggtcgattcggaaaagctcctggccaaacttgaaaagcaacgtggcaaagcccaggaaaagctgcacaaggctcgcaccaagctgcaggatgctgccaaggccggcaagaccaaggcacaggccaaggcgcgcgagaccatcagcgacctggaagaggcgttggataccctgaaggcccggcaggcggacacccgtacctacatcgtcggcctcaagcgtgacgtacaggaaagcctcaagctggcgcagggtgtcggcaaggtgaaggaagctgctggcaaggctctggagagccgcaaggcgaaacccgcgaccaaacctgctgcgaaggcggcagccaagcctgcggtgaaaaccgtagcggcgaagcctgcggccaagccggctgcgaagcctgctgcgaaaccggcggccaagcctgcggcgaaaaccgcggcagcgaagcccgcagccaagccgacggcgaagcctgctgcgaaaccggcggccaagcccgcggcgaaaaccgcagccgcgaagcccgcagccaagccggcggcgaagcctgtggcgaaaccggcggccaagcctgcggcgaaaaccgcagccgcgaagcccgccgccaagccggcagcgaagcctgtcgcgaaaccgacggccaagcccgcggcgaaaaccgcagccgcgaagcccgcagccaagccagctgcgaagcctgcggcgaaaccggcggccaagcctgtggcgaaatccgcggccgcgaagcctgcagccaagccggctgcgaagcctgcggcgaaaccggcggccaagcctgcggcgaaacccgtagccgcgaaacctgccgcaaccaagcccgccaccgctcctgctgcgaagcctgcggcgactcccagcgccccggcagccgcctccagcgctgcttcggcaacgcctgccgcgggcagcaacggcgccgccccgaccagcgcctcctaa

SEQ ID NO: 41 - DNA, 1263 bp, Pseudomonas aeruginosa
atgtggggtcttacgatgaagtttgcgagcctgattctgatgcttctctttgccacggtggcgagggctgaggattactactggaaaattcagtcactgcctgaacgcttttcttcgccctcggcagcttgcgcggcgtgggccaaagccacgggacgccctggggagttcaccttcaccgggtctatgaaagcccgtgaccagacctcgttttggtgcgagttcacgaacaacgaaaccggcaagactgctgccgggtatggtcctgccggacgctatggcgatagctgtcccgaggggacggaatacgataaggcgaccggggtttgtaagtcgcctccgcaagaatgcaaggaaggcgaactgttcccggccaaaggcccggactctcccgtggttacctcgggaggccgtaactatgtcggtgacggcggcgccccgaccgcctgctatcaaagctgtgagtatggcggcaatcccagcccggccagttgctatctggtcaaaggctccaccacgaccggcttctgcaattacatcctcaagggcaccggacagaattgcggtgccgattcctacaccttctcccagaccggcgattcgctgaacccgcccgacactccgaacaccgatccttccgacccgaacgaccccggctgcccgcccggctggtcgtggtcgggaactacctgcgtcaaggccccgaccgatcccacggatccaaccgacccgaccacgccgggcagtgacggcggcggcgatggcaatggcggtggaaacaataacggcggcggcaatgacggcggcaccggcaatggcggcgacggcagcgggggaggggacggcaacggcgggggcgatggtagcggcgacggtgacggcagcggcacgggcggcgatggcaacggcacctgcgacccggcgaaagagaactgctccaccggccccgaaggccccggcggcgaactcaaggagcccacgcccggcacctgggatgacgccatcgccacctgggaaaagaaggtcgaggacgccaagcaagaactcaagaccaaggtgaaggccaacgtcgatcagatgaagggcgccttcgacctcaacctggcggaaggcggcgggcaactgccctgcgagtccatgaccatttggggcaagtcctactccctctgtatctccgactacgccggccaactctccagcctgcgcgtggcgctgctgctgatggccgcgctgatcgccgccctcattctgctgaaggactga

SEQ ID NO: 42 - DNA, 1284 bp, Pseudomonas aeruginosa
atggccgtcgcccctggtgtgttgttgccgccgacgcctgatgtaaagcccaaggccgctgcgccgaagagccagcagaaaacgcctgagcccagtaacgacaagacttccagcttctccgacatgtatgccaaggagaccgcgaagaagcccgccgagcgcgccgacggtcccgcgaagggttcgcgggacaagccacgggacgccggcaaggacgccgccgaagcgcagccgacggatgccgtcaggcagccggccgttgccgaagacggcaagcctttgccggccgacggccaggccaaggccgacggcgaagataaagtcgaaacgccggtcgatccgctgcaattgctcggcctcggcggtgccgtaccgttgctcgacgagaatacccaggcgactttgctgccaccggccgtgccgacggccagcagtgctccggccagccttaccgaagccagcagcgacccgaccctggtcaagctcaacggcgtgccggcggtgaacatggccctggagcagggcgcccaggacgccgcgcagacggcgaaaggcgggccggcgaagagcgccgatccccgccaggcgaacctcggcgatgcccttgccggcctgacctcggattccttgaccaaggccgtcgacggcaaggcgctcgaggcccagttgcagcagaccgccgagccggccgtcgccagcgccgcctccgagagcctgctggagagcaaggcggaaccccgcggtgaacctttcgcggccaagctcaacgggctgacccaggccatggcgcaacaggccctgaccaaccgtccggtgaacggcacggtgcccggccagccggtggcgatgcagcagaacggctggagcgaggcggtggtggaccgggtgatgtggatgtccagccagaacctgaagtcggcggagatccagctcgaccccgccgagctgggacgcctggacgtgcgcatccacatgaccgccgaccagacccaggtgaccttcgccagtcccaacgccggcgttcgcgacgccctggaaagccagatgcaccggctgcgcgacatgttcagccagcagggcatgaaccagctcgacgtgaacgtctccgaccagtcgctggcgcggggctggcagggccagcagcagggcgagggcggatcggcgcgcggacgcggcttggccggcgaggcctcgggcgatgaggaaaccctcgccggagtcagcgagatccgcagccggccgggtgcgtcggcggcgcgcggtctggtcgactactacgcctga

SEQ ID NO: 43 - DNA, 1287 bp, Pseudomonas aeruginosa
atgctccgcctccttcctctcctgctatccctcgcctgtctcgctccggccttcgccgacgagcgcgccgacacccaacgccagctggaacagacgcagaaggacatcggcgagctgaagaagctgctggacggcatccagcaggaaaagagcggcgtgcagaagcagctgaagtccaccgagaccgagatgggcgacctggaaaaacagatcaaggccctgcaggacgagctggacaagagcgaagccgagctgaaacggctggatggggagaaaaaaaaactccaggacgcgcgcattgagcagcagcgcctcctcgccatccaggcccgcgcggcctaccagagtggacgcgaggaatacctgaagctgctgctgaaccaggaacacccggaaaaattcagccgcaccctcacctactacgactacatcaacaaagcccgtctcgaacagctcgccagcttcaacgaaaccctccgccagctggccaacgtcgagcaggacatctctgcgcagaaagccgaacaactgagcaagcaaggcgagctggacagccgccgcgaggcgctggcagcgacccgcaaggagcgccagcaagccctggccaagctgaacagcgactaccgcgaacgcgaccagaagctcaagtcccgccaacaggaccaggccgagctggccaaggtactgcggaccatcgaggaaaccctggcccgccaggcccgcgaagccgccgccgcggcggagcgcgagcgccagcgcgcgctggccgccgaacgcgagcgtgcgcgccagcagcaggccgcccccggacgagtcaccagcccgccgcgcgaacctgcgccgggcccgctggtctcaagcactggcgcggtctacggcggcgcgttcggctcggcccgcggcaagctgccgtggccggtgaatggccgcgtcgtggcgcgcttcggcagccagcgcggcgacgatccgcgggcgaaatgggacggcgtactgatttcggcgagcgccggcagcaccgtccgcgcggtgcacggcggacgcgtggtattcgccgactggttgcgcggagccggcctgttggtcatcctcgaccacggtggcggctacctcagcctttatggccataatcaaagcctgctgaaagacgccggcgacaccgtgaaggccggagacccgatcgccaccgttggaaccagcggcggccagagtagcccggccgtgtacttcgccattcgccatcagggccgcccggcggaccctactacctggtgccgcgcacagggatag

SEQ ID NO: 44 - DNA, 1707 bp, Pseudomonas aeruginosa
atgcaaagactgtcgcgtatcggccgcaacaccctcgccgtctccgtttccaccttgctcctcagcgcctgcaaccagggcgacgatgcgccgaagcctgcggcagtcgcgccgcaaccggccgcaccgagcatggctgcactgagcatcccgctatgcctcaacggccagtgcgcggtgatcgaccaggacgccaagctgctcgtgccgttcgacaacgactacgacaatatcgtcgccagcgcctaccagggcaccctgatggcggcgcgcgaggagcgctggaacctgatccaggcgaaggacggcaaggtgttgcgcgacgatatcggcgaagccctgtcgctgctcacccccaacctctatggcttcgtccgcgatggcaagtacggcgtggtcgacggccagggcaaggaagtccaggcgccgcgtttcgacgacatctaccccaacagtgccaacgaattcatcatctacgagatcgatggcaagcgcggcatcctcgatgccaagggcaagcagctcaccgaggcgctctacgacaccaccctggtcaacggcagcgtcgccgaacacggtggcttgatcagcgccgagcgtggcgaggagaagtggatcatcaacctcgctaccggcgaacagaaggccgtggcctacgagagcctgggcgacctccacgacggcgtgatgagcgccagcgtcatcggcaagggctcccaactggtggatgccaagggcgacgtggtcggtgacggcaagagctacgattacctgggcaccccggccaacggcctggtcgcgttccgcgagaagtacgacagcccctgtggctacctcgactaccagggcaaggtggcgatcgccgcccagttcgccggttgcggcgccttcggcaagcagggcgggctggcccagcagcgcatggaagatggctcgtcgggcaagtacggcctgatcgatcgcagcggcgcctggaaggtgcagccgcagtacgattcggccgacagcgccggcctcaccgcgcttggctacaccgtcgacgtgcccggcctggctgccgtcggcgtgagcaccggcctgttcagcgccgacttcggcatcttcaacctcgacgaaggcagcgagtgggtgaagccgggttatgcgcagatcggcgcgctgggcaacgacctgttcgtcgtggcgaagaagggcgggccgcagaagaccgtcagcttcatgggttcggaaagccaggtgccggtggtgggcctgatggaccgcagcggcaagatgctgctggagccggacgaactgatcagcatccagtctgcttatgacggtcgtttcctggaaggtctcgacggtatggacaacgctgcccacaccgtgttgctcgatcgccagggacgcacgctggttccagcgctctggcagaagctggaggtgaatccgcagcagggttacatcctgggctacgaagtcagcggcactggcgacgaggcgacggaaaccttgcgcgcactgtacgacctgaacggcaagccgcgcttcaccgtggccaccaccgattgcggcgccgaacagttgctcgacggcaatggcaaggcgatctggccgcaggacccgaccccgtattgccagtcggacgacgagcaggacgacgaaggcgagccggagcaggagccggcgcccgtcgaagagagcgaggaaaccagcgagagctga

SEQ ID NO: 45 - DNA, 1740 bp, Pseudomonas aeruginosa
atgcttcgccccgccaggtctctctcgctctgctccgccctggtcatcctgctcgccgcctgtggcgagggcgaaccgctgctcccggccgatgcgcgcctgcctgacggcgcgcgctatcgcggcgagctggtggacgggcgcctggaaggccagggccggctggactacgacaacggcgcctggtacgccggccgcttcgagcatggcctgctgcacggccatggcacctggcagggcgccgacggcagccgctacagcggtggcttcgcggccggcctgttcgacggtcagggacgcctggcgatggccgatggcagcgtctaccagggcggtttccgccagggcctgttcgatggcgaaggcagcctggaacaacagggcactcgctaccgcggcggtttccgcaagggcctgtacagcggccagggcacgctggacggcagcgatggcagccgctaccagggcagcttccgccagggccgcctggaaggcgaaggcagcttcagcgacagccagggcaaccagtacgccggtaccttccgcgacgggcaactgaacggcaaggggcgctggagcgggcccgatggcgaccgctacgtcggccagttcaaggacaaccagttccatggccaggggcgctacgaaagcgccagcggcgatgtctggatcggccgcttcagcgaaggcgcgctgaacggccccggcgagcttctcggcgccgacggcagccgctaccgcggcggtttccagttctggcgcttccatggccagggcctgctcgaacaactggacggcacccgctacgaaggcggcttcgccgccggcgcctatgccggccaaggcaccctggaccgcgccgacggcagccgtgagcagggactctgggccgacggcaagcgcatccgcgacgccgccggcaaggccctgcccgacactctggaagtcggcctgttggcccagggtcgcctgctcgacgaagaactgcgcaagatcccggcctcgacgccggccagcgaactctatgccctgagcctgggcggcgatggccgccagggcgtgttcctgcgcgaggccgattacgccggcgacctgctcggccagcgtttcgccgctcgtggcgtgattcgcctggtcaaccaccgcgaccacttcggcgaccgcccgctggctacccgggaaagcctgtcccgcgccgtgcgcaccctggccgaacgcagcgggccggaagacctggtcttcatctacctgaccagccacggctccagcgaccaccagttggccctggacatgcccggcctgaacctcggcgacctgccggccgcggaactggccgaactgctcgcgccgctgcgccagcgcgacaaggtgctggtggtatcggcctgctacagcgggggcttcatcccgccgctgaaagacgaacgtaccctgatcctgaccgccgcgcgtgccgaccgggtctcgttcggctgttccgacgacgccgacttcacctatttcggccgcgccttgctggccaatgcgctgaaccgcaccgacgatctgtccaaagcgttcgaactggcgaaagaggaagtgcgtcaaagggagaaggaggaaggtttcgaagcttcggaaccgcaagcctggttaccggaacgcgtgctcgcgcactggcggacgctgcgggggcagcaagccgagcgcgcgctcgcgtcccgggaaggaaaaaccggcgagggcgcggcgggcaaatag

SEQ ID NO: 46 - DNA, 1866 bp, Pseudomonas aeruginosa
atgctgcagaacatcagggataattcccagggctggatcgccaagaccatcattggcgtgatcatcgttctcctgtcgctgaccggcttcgacgcgatcatccgggccaccgaccactccaacgtggccgccaaggtcaacggcgacgatatcagtctcaatgaagtccaacaggccgtggacatgcagcgtcgccagctgctgcaacgcctgggcaaggatttcgatccatccatgctggatgacaagctgctcaaggaagcggccctgaaggggctgatcgagcgtaccctgctgctccaggccgccaaggacgacaagttcgccttctccgaccaggcgctggaccagttgatcctgcaaactcccgagttccaggtcgacggcaagttcaacgcggatcgcttcgaccaggtcatccgccagatgaactacagccgcatgcagttccgccagatgctcggccaggaaatgctcatcggccagcttcgcgccggcctggcgggcaccggtttcgtcaccgacaacgaattgcagtccttcgctcgcctcgagaagcagacccgcgacttcgccaccctggcgatcaaggccgacgcctccaagagcagcgtgagcgacgacgaggtgaaggccttctacgaaggccacaagagcgagttcatgactcccgagcaggtggtcgtcgaatacgtggagctgaagaagtcctccttcttcgaccaggtcaaggtgaagcaggaagacctcgaggcgctgtaccagaaggaaatcgccaacctttccgagcagcgcgatgccgcccacatcctgatcgaggtgaacgacaaggtcggcgacgagcaggccaaggcgaagatcgacgagatcaaggctcgcctggccaagggcgaggatttcgccgcgctggccaaggagttctcccaggatatcggctcggccgccaccggcggcgacctgggctacgccggtcgcggcgtgtacgaccccgcgttcgaggaggcgctgtatgcgctgaagcaaggtgaggtatccgccccggtgaagactccgtacggctaccacctgatcaagctgctgggcgtgcaggcgccggaagtaccgagcctggaaagcctcaagccgaagctcgaggacgaactgaagaaacagatggtcgagcagcgcttcgtcgaggctaccaaggacctggaaagctccgcctacgaagccgccgacctgagccagccggcgcaggaaatgggcctgaaggtccagaccagccagccgttcggacgttcggggggcgacggcatcgctgccaaccgccagatcgtgcagaccgcgttcagcgccgaggtgctggaagaagccgccaacagtggcgccatcgagctggatccggacaccgtggtggtgctgcgggtcaaggaacacaacaagccgaaggagcaaccgctggagcaggtcgcggcgaacatccgcgagcgcctggccgccgaaaaggccgccgaggaggcgcagaagcgtggcgaggccctgatcgcagagctgcgtgaaggccgtacctcttccgcagcgggtgagtcgtggaaagtggtcgaggcggcctcccgcggccacgaaggcgtcgatccgaaactgctccaggcggtgttccgcatgcagcgtccggaggccaaggacaagccttcgttctctggcgtgaccctggccaatggcgattacgtggtgatccgcctgaatggcgtcagcgagccggaggaggctatctccgacgacgagaaggccatgtaccgccgcttcctggcttcgcgcagcggacaggcagacttcgccgccttccgccgtcagttgcaggacaaggcggaagtcgagaaatactga

SEQ ID NO: 47 - DNA, 2067 bp, Pseudomonas aeruginosa
atggatatgacgtcgctgatgcccctcctgctgggagtgggcctggtcgttctgctggtcgtgggcctgctggccctgttcaaggccttctacatcaaggtcccgcaaggcaccgcgctgatcgtcaacgacatgtcgtcgacgcccaaggtgcatttcaccggtgcgctggtctatccggtgatccacctgaaggagttcatgcgcatctcgctgatcaccctggaggtcgaccggcgcggcaaggacggcctgatctgccgcgacaacatgcgcgcggacatcaccgttgccttctacctgcgggtcaacgagacccaggacgacgtgctcaaggtggccaaggccatcggcgtcgaccgtgcttccgaccgttcggcggtgaacgagctgttcaatgccaagttctccgaggcgctgaagaccgtcggcaagcagttcgacttcgtccagctgttcgagaatcgccaggacttccgtgaccgcatcatcgaggtgatcggcaacgacctgaacggctacgtcctggaagacgtcgccatcgactacctggagcagaccgcgaagaactcgctggacccgagcaacatccttgatgccgagggcatccgcaagatcaccgagctgaccgccacccagaacgtcatcaccaacgaactggagcgcaacgaagagctggcgatcaagaagaagaacgtcgagacccgcgaggcggccctggccctggagcgccagcaggctgacgccgaggcccggcagaagcgcgagatcgagaccatccgtgcccgcgaggaagcggaaaccgcgcgggtcaaggaagaggagcggctgaaggccgagcaggcgcggatccaggcgcagcaggaaatcgacgtgcgcaccgagaaccaccagcgcgaggtcgaggtggcgcagcagaaccgccagcgcgcggtggtcatcgaggtggagaaggtcacccgcgccaaggacctggagatcgtcgcccgcgagcgtgaggtggagctgcagaagatcgagaaggaaaaggcgctggaagagcagcgcaagaacattgccaatgtgattcgcgagcgcgtcgcggtggaaaagaccgtggcccaagaggaggagcggatcaaggaggtgcgcgaggtttccgaggccgagcgggtcaagcaggtgatactgctgcaggcccaggcggaagccgagcaggagctggtacgccaggtcaagcaggcggaagccgacgaggcccgctccaagcacaaggcggtggaaatcaacaccatggcgcaggccgagctggaggcggcgtcgaagcaggccgaggcgaagaagcgtctggccgagggcatcgaggccgagcgcgcagcgccgggcctggccgatgcgcgggtgctggaagtcaccgccgcggcgaaggaaaaggatggcttggcagcggcgcgggtacgtgccgaacaactgatcgccgaagccaggggcgacgaagagcgcggcctggccgacgcccgggtgctcgaggcgcaggccgcggccaaggagaaggacggcctggccgaagccaaggtgctggccgagaagctcggcgcccaggcgcgcggcgaggagcagctcggcgcggccaaggccaaggccaccaaggaccagggcagcgcggaagcggaagtactgctgcagcgcctgaatgccgaggccgaggggcttggcaagaagttcggcgccctggatgccctcagcgacagcgctcgccagcacgaagagttccgcatgcagctggagaagagcttcgaggaggccatggcggccatcgccgcgaacaaggacatcgccaaggaccaggccgaggtgctcgccaccgcgctgggcaaggcgaacatcgagatcgtcggcggcgagggcgacttcttcaactccttcgccaagtcgctgtcggtgggcaaggccatcgaaggtgtggtcggcaagagcccggtggtgcaggacgtcctcgcccgcctgctcaacggccgtggcgcagccgctgcggtgatgccggaacgcaagagcggccacgagaacgagccggcggcggaagtctga

SEQ ID NO: 48 - DNA, 2229 bp, Pseudomonas aeruginosa
atgtacccccaattccgtcgcggccatctcgccgctgccgtccttttcgcttcatcgagcctgctgggcgggcaggccctggccgaggacgagcgcctggaagaactggacgaacgcgccgaatcggtggtccagctgggtgacgaggtggtgctgggcaccgccgaacaggagctcaagcaggcaccgggggtatccatcatcaccgccgaggacatcaggaagcgcccgccggtgaacgatctctccgagatcatccgcaccatgcccggggtcaacctcaccggcaacagttccagcggccagcgcggcaacaaccggcagatcgacatccgcggcatggggccggagaacaccctgatcctggtcgacggcaaaccggtcagctcgcgcaactcggtgcgctacggctggcgcggcgaacgcgacacccgcggcgacagcaactgggtgccgccggaggaggtcgagcgcatcgaggtcctccgtgggcccgcggcggcacgctacggttccggcgcggcgggcggggtagtcaacatcatcaccaagcgcccgaccgatcgtttgcgtggttccatgacggtgttcaccaacattccggaaagctccaaggatggcgccacgcgccgcgccaacttcagccttagcgggccgctgaccgaagccttgagcttccgcgcgtacggcagcgcgaacaagaccgattcggacgataccgacatcaacctcggacataccgtcaacccgagccgtaccgtggccggacgcgaaggggtacgcaatcgcgatctcagcgggatgctgtcgtggcaggtgacccccgaccaggtcgtcgatttcgaagcgggcttcagccgacagggcaatatctatgccggcgatacccagaacaacaacggcaccgccaatacccagggactcgccgacgacggtgcggagaccaaccgcatgtatcgcgagaactacgccatcacccacaacgggacctggtcgttcggtacttccaggttcgtcgcccagtacgactccacccgcaacaaccgtctggaggaggggctggccggttccgtcgaggggcagatcggcgccgaccgttcgttcagcgccagcaagctggagaactatcgcctcagcggcgaactcaaccttccgttgcatgcgttgttcgagcaggtgctgacggtgggcgcggagtggaacaaggaaaccctcaacgacccgtcctcgctcaagcagggcttcgtgggaagcgatagcttgccggggacccccgcggccggctcgcgaagcccgaaaagcaaggcggagatccgcgcgctgtacgtggaagacaatatcgaactgcgccccggcaccatgctcacccccgggctgcgcctggacgatcacagcgacttcggcctgaactggagcccgagcctgaacgcttcccaaacgctcggcgaatacttcacggtcaaggccggtatcgcacgggccttcaaggcgcccaacctgtaccagagcaacccgaactacctgctctatacccgtggcaacggttgcccgatccagactagcagcggcggctgctacctggtcggcaacgagaacctggacgccgagaccagcgtaaacaaggaactgggcatcgagttccggcgcgatggctgggtcgccgggctcacctacttccgcaacgactacaagaacaagatcgtcgcgccgctggatgtcatgggacagaccgggaccggcaacaacatcctgcaatggagcaacgcgaagaaagcagtggtcgagggcctggaaggcaacctgctggtccccctgcacgaggacctgagctggagcaccaacctgacctatatgctgcaatccaaggacaaggacaccggcaacccgctttcggtgatccccgagtacaccctgaactcgaccctggactggcaggccagcgagcgtctttccacccaactgaccagcaccatctacggccgccaggagccgccgaagcatggcaccagccgcaacacgccggtggtctcgcgaaaagaggtgggtacctatggcatctggggcgtcagcgccggctacaccttcagcgagaacctgagcgtacggggcggggtaagcaacctcttcgacaagcgcctgtaccgccagggcaactccttcgacgccggcgcggcaacctacaacgagccgggtcgcgcctactacgtttcgatgaccacctcgttctga

SEQ ID NO: 49 - DNA, 2241 bp, Pseudomonas aeruginosa
atgtcctcacgcgcccttcccgccgttcccttcctgctgctgtccagttgcctgctcgccaacgccgtacacgccgccggccagggcgacggctccgtcatcgagctgggcgagcagaccgtggtcgccaccgcccaggaggaaaccaagcaggcgccgggggtttccatcatcaccgccgaggacatcgccaagcgaccgccgagcaacgacctgtcgcagatcatccggaccatgccgggggtcaacctgaccggcaacagctccagcggccagcgtggaaacaaccggcagatcgacatccgcggcatgggcccggagaacaccctgatcctggtcgacggcaagccggtcagctcgcgcaactcggtgcgctacggctggcgcggcgagcgcgacagccgcggcgacaccaactgggtgccggccgaccaggtcgagcgcatcgaagtgatccgcggcccggcggcggcgcgctacggcaacggcgcggcgggcggcgtggtgaacatcatcaccaagcaggccggcgcggaaacccacggtaatctcagcgtctacagcaatttcccgcaacacaaggccgaaggcgccagcgaacggatgagcttcggtctcaacgggccgctcacggaaaacctcagctaccgcgtctacggcaacatcgccaagaccgactcggacgactgggacatcaacgccggccacgaatccaaccgtaccggcaagcaggccggcaccctccccgccggtcgcgaaggcgtgcgcaacaaggacatcgacgggctgctcagctggcgcctgacgcccgagcagaccctcgagttcgaggccggcttcagccgccagggcaacatctacaccggcgacacgcagaacaccaacagcaacaactacgtgaagcagatgctcggccacgagaccaaccgcatgtaccgcgagacctactcggtcacccatcgcggcgaatgggacttcggcagctcgctggcctacctgcagtacgagaagacccgcaacagccggatcaacgaaggcctggccggcggcaccgaaggtatcttcgaccccaacaacgccggcttctacaccgccaccctgcgcgacctgaccgcccacggcgaggtcaacctgccgctgcacctgggctacgagcagaccctgaccctcggcagcgagtggaccgagcagaagctcgacgaccccagctccaacacccagaacaccgaggaaggcggctcgatccccggtctcgccggaaagaaccgcagcagcagttcctcggcgcggatcttctcgctgttcgccgaggacaacatcgagctgatgcccggcaccatgctcaccccaggcctgcgctgggaccaccacgacatcgtcggcgacaactggagcccatcgctgaacctgtcccacgcgctcaccgagcgggtcaccctgaaggccggtatcgcccgcgcctacaaggcccccaacctgtaccagctgaaccccgactacctgctctacagccgtggccagggttgctacgggcaaagcaccagttgctacctgcgcggcaacgacggcctcaaggccgagaccagcgtgaacaaggaactgggcatcgagtacagccacgacggcctggtagcggggctgacctacttccgcaacgactacaagaacaagatcgaatccggcctgtcaccggtcgaccacgccagcggcggcaagggcgactacgccaacgcggcgatctaccagtgggagaacgtgcccaaggcggtggtcgagggcctcgaaggcaccctgaccctgcccctggccgacggcctgaagtggagcaacaacctcacctacatgctgcaatcgaagaacaaggaaaccggcgacgtgctctcggtgacgccgcgctacaccctcaactcgatgctcgactggcaggccaccgacgacctctcgctgcaagccacggtcacctggtacggcaagcagaagccgaagaaatacgactatcacggcgaccgtgtcaccggcagcgccaacgaccagctctcgccctacgccatcgccggcctcggcggcacctatcggttgagcaagaacctgagcctcggcgccggcgtcgacaacctgttcgacaagcgcctgttccgcgccggcaatgcccagggcgtggtcggcatcgacggggccggcgcggcgacctacaacgagcccggacggaccttctataccagcctgaccgcgtcgttctga

SEQ ID NO: 50 - DNA, 2355 bp, Pseudomonas aeruginosa
atgtccccgtcacgcgccctgtcgccgctcagccgcgccctgctcctcgcctgcctcggcggtcccgtcctggtttccgccggcagcgcctgcgccgccgagatccgcaccgatgcccgccagtactaccgcctgcctgccgagccgctggagcaggcgctgaaccacctaggccgccaggccggcgtgctgatcgccttcagcccggaacagaccgccgcgcgacgcagccaggcgctggacggcgagtacaccctggaggaagccctggccgccctgctcgtcggctccggcctggaggcgcgcgcccgcggcgacggcgcctacaccctggaagcgctgccggtggaagacccggccaacctgcaggcgctcaccgtggtcggcgactggctggccgacgccagcgccgccgacgtcttcgagcatcccggtgcgcgcgacgtggtccgccgcgagcagttccaggcccaaggcgcggccagcacccgcgaagtgctggagcgcattcccggggtcagcgcgccgctcaacaacggcaccggcagccacgacctggcattgaacttcggcattcgcggcctcaacccgcgcctggcgtcgcgctcgacggtgctgatggacggcatcccggtgcccttcgccccctacggccagccacagttgtcgctggcgccggtgtccatcggcaacatggacgcggtggacgtggtccgcggcggcggcgcggtgcgctacgggccgcagaacgtcggcggcatcgtcaacttcgtgacccgggcgatccccgaggacttcgccaccaagctcgacgtgcacagcgaactcagccccagctccagccaggacggcctgaagaccacccacaacgtgctgatcggcggcaccggcgccaacggcctcggcggcgccctgctctactccggcacccgcggcggcgattggcgcgagcacagcgatacgcggatcgacgacctgatcctcaagggccgcttccagcccagcgacgaacacacgttttcggcgatgacccagtactacgacggcgaggccgacatgcccggcggcctcggcaccgcggcctaccacgacgacccgtaccagtcgacccgtccctacgacaagttctggggccgccgtaccctggccagcgccagctacgaatacacccccaacgccagccagaagctcaacgtcaccggcttcttcaccaagaccctgcgcagcggctacctcgaccagggccgcaacctcaccctgtcgccgcgcgaatactgggtgcgaggcctggaaacccgcttcagccagggcttcgagctgggcgaaagtcgccacgaagtgggcatcggccaccgctacgtcaacgaagccagccacgagctgcgctactggacccgcgccgacagcggccagctacccagcaccggcagccgcaacgaccgcgacacccgcggcagcaccgaagccaacgcgttctacatcgacgatcgcatcgacatcggcaactggaccatcacccccggcatccgctacgagaagatcgattccgaacagaagaacctgctgaagaacagcaaggacagcggccgctacaacgcctcgctgccggcgctcaacgtgatctaccacctcacgccgagctggaacctctacgccaacaccgagggctcgttcggcaccgtgcagtacagccagatgggcaaggcggtgcgcagcggcgacatcgagccggagaaggcccgcacctgggaactcggcagccgctacgacgacggcatcctgcgcgccgaactgggcgccttcctgatcaacttcgacaaccagtacgagagcaaccagcagaccgacagcgtgaccgcccgcggcaagacccggcacaagggcatcgaggcggcgatcgcctacgacctggccgatctcgacccgctgctctccggcttcgacgtctatgccagctacgcctacgtcgacgcgagcattcgcgaagacgggccgaacaagggcaaccaggtgccgttctcctcgaagcacaagggcacccttggcgccaactaccgcaccggcgcctggagctacaacctcgacggcagcttccagaccagccagtacgccgacaacgccaacaccgagagcgaaagcgccgacggcagcaccgggcggatcgccggctggatggtctggagcgcgcgcggcacctacgacttcggcccgcaactgaacgacctcaagctcggcctgggggtgaagaacctgttcgatcgccgctactacacccgctcgttcgacgacaacaacaagggcctctacgtcggccagccgcgcaccctgtacgtacaggcctcggtcggtttctga

SEQ ID NO: 51 - DNA, 2556 bp, Pseudomonas aeruginosa
atgaccttgcctttcacccgcgccgcctggcgcccgctgtgttccgccgccgtgctcggcgccgcgttgtgggccgccggcgccagcgctgccgaacgacgcttcgacctgccggcgcagccgctggccgcctcgctgtcgcgcctggcgcagcaggcgcaggtccaggtgctgttcgacgagtcgctcctgcggggcctgcgcgctccggcgctgagcggcagctacggggtgcgcgaggcgctggagcggttgctggtcggttccgagctggagctggtggaggcgggcggcggctacgtggtgcgccggcgccaggtcgacgcctacagcgacaacgcgctgcaactggacgcgcagaccatcgtcggcaacggtcgcgaagtggacgccagcaacgtcggccgttcgaccctgacccggcgggatatcgaacgccagcaggcggacaacatccccagcctgctgcagaccctgcccggagtgaccatgggcggctcgcccaagccgggcggacagaccaccaacatctggggcctgggcgacgccgaggacgtgccctataccctggacggcgcgcagaagagcggcttcgagcgctaccagcagggcaccgtgttcatcgaaccggaaatgatcaagcgcatcgaggtggagaagggaccgcactcggtgttcaccggcaatggcggcttcggcggcaccgtgcacatggagaccaaggacgcgccggacctgctgcgcgaaggccgcgacgtcggcgccatgctcaagtacggctatcactccaacgaccagcagaagatctactccggcgccgtgttcggtcgcagcgaagaccgccgcgtcgatgccctgctctatctcaacggtcgcgacggccgcgacatgaagctggccgacaacctgccgctgtcgcccaccgactacccgatcaaccccaagcgcctgcccaacagcgcccaggacgagaagaccggcctgttcaagctcaacctgcaccccaccgaggagcacgacctgggtttcacctacctgcgctcgaaaagctcgcgctggacgccgttctccgccagcagctacccgaccccgccgagccagtggaccatcgaccgctacggctacgagctgggcctgacccgcctgctggcccaccgcgataccaccgacaccacctggaccggcaagtacaactaccatccgctggacaacccctggatcgacctgcaactgagctattccgacgcccgcaccgagcaactcgaccgtcgcgaggacaccgccttctaccagctcgccaccggtggcaagcggatgcgtaccgagtaccaggacaaggtcctggaactgcgcaacaccagccgtttcgataccggagcgctacagcacgagctgaccctgggcgcggcgctgcacaagcacaagcgcgacatcctcatgcacatgccgggcaagacctacgagaccccgcgctacaattacggctggctgcaaccggcattcatgccggccggcaagcaggacacgcagagcttctacatccaggacgcgatcacctacggcagcctgaccgtcaccccatcgatgcgcttcgacagcgtgcgcaacgacggccaggccaacctggcgccgatctacgacaatcccaagctcggccatgactatcgcgcccagacctactccggctggtcaccgcggctgtcggtgttctggaccgcgacgccgaacctggcgttcttcgccgactacaccgagacctggcgagcgccggtgatcgacgagcagtacgaagtgcagaacagttcgaccatcggtggcagcagccgcgacctggacgccgagcgcatccatgcgatccgtggcggcagcgtgatcaacctgccggacctgctggtcgccggcgacagcctgcagatccgcaccacgttgttccagaaccgcatcaaggacgagatattccgcacccgcagcgtcggctgccgccagcagtcgatcgacaacggcagtatcggtggtagctgcggcgacatgctgccgctgagcaactaccgcaacttgccgggcctgaccatcaagggcttcgagatcgagagcttctacgacagccagcggctgttcggcagcctgtcctactcgtggatgaccggcaagcacgatggggcctacagcaatccctggggaccgaacgtgtgggcgcgcgacatcccgccgccgaagtgggtggccatgctcggcctgaaggttccggaatgggatgccaagctcggctggcagggcgagttcgtgcgcaagaccgaccgcctgcccagcgatcgctacagcggcgggatgggtaccggttccggcgatatctactgggatcacgcggccaacgacagctacgacactcatcggctgttcgccgagtgggtcccggccaagctgggcctgaaggacacccgcatcgacttcaccgtggacaacctgttcaaccgctcctatcgccagccgctgggcggcgacctggtctacagccagggacgcaacgccaagatcagcgtcacccagttcttctga

SEQ ID NO: 52 - DNA, 2643 bp, Pseudomonas aeruginosa
atgcaccgatcgctccacaccgacgcgccgctgggcgccgccctgctgctggccctgcagctcgctcccggcagcgccgccgcggcggaggaacaggcgcctgtcgacccgcccacggtccagttgcaacgaatcgaggtgaccggcagcgcgatccgccgggtcgatgcggaaaccgcggtgccgatcagcgtcctgcgcgccgaggagctgcgccaacagggcgtgaccagcaccgaggaactgatcggccggctttccggcaaccagggcgtatacaactccagtcgctcggtcggcagcgccaccggcggcgcctcgttcgccgacctgcgcggaatcggcgcgaacaagaccctggtgctgctcaacggccggcgcctggcgaacaatgccatcgacggctccgcggtggatctcaacaccattcccttcgccgccatcgaccgggtcgaggtgctgcgcgacggcgcctccgcgctgtacggcaccgatgccatcggcggggtgatcaacttcatcacccgcaagagcctgaacgaaggccgcttcgacagcggctacgcctcccccacccacgacggcggcggcaaccagcgcaacgtcagcgctagctggggcttcggcgagctggaggaggatcgcttcaatgtcttcgcggtggccaactacgacaagcaggagcgcctcggcgccaaggaccgcggctacacctacaactaccagccgggacgcggcctcgactacagctccggcaccgccttccccggcaactggagccagggcgccaacgccagcaatccgctggccgccggcggttgcaagggcgccgacctgattccgcgcaacggcatctgccggcagagcctgtggcgctacctcgacctggtgccggaaaccgagaagacctcggtgttcagccgcgccaccggcaagctggccgacgagcacaacgtcagcctggagtacttctggtcgcgcagcgacaacgctacccaggtcggcccagggaccctcaccggcctgcagatcgatcccggcaccgccttctatcccggcaacggcatcactcccggacccggcggcttcgtcctcgacccgagccggccggtggaggtcaactggcgacagagcgtgctcgggccgcgcctgcaatcctcgcagaacaccggccagcgcctgctgctcggcttcgacggccagttcgccggctgggactacgatatcggcgcctcgtacaaccagaacaaggtggtcgaccatatccacagcggctacgtcgatgatcgcgccgccgccctcggcatcgccaacgggacgctgaacccgttcgggccgcagaccgacgccggcctcgcctacctcggcagccatgccctgagcggcgacttccgtacctcggtcggccgcgtcaagggcctggacgcccgcgccagccgggagatcggcgactggttcggcgccgggccggcggccctggcgctgggcggcgagttccgcaaggaagcgttccaccaggacatccaggacttcgccggcaacgtgcagagcctcggcgtcgatcccgccgccacggtcagcggcgagcgcaacctgaaggcgcagtacgccgaactcaacgtgccggtgctggacagcctggaactcagcgcggcgatccgccacgacaagtacagcgacttcggcagcaccagcaacccgaaatattcgttccgcttccagccgttccgccagttggtcctgcgcggcgcctacagcgaaggtttccgtgcgccgtcgctgtacgaactgtacaacccgaccttcaccacctataccagcgccaactacgacgacccgcgcctgtgcgccggcggccagccgagccagggcggcatcgccaaccgcgactgcgcccagcagttctacaacgccaccggcggcaataccgacctgcgaccggaaaccgcgcgcaacgttaccctgggcctggtctaccagccgctgcgcgacctttccgtcggcctggacttctggtggatcaggatcgccaaccagatcgccgagtttcccgaagcggcgatcttcgccgacccgcaggcctacgccggacgcatcgtgcgcaaggccgacggctcgatcgatcacgtcgtcaccggactggccaacctcggcaaagtgaagaccagcggcgtcgacctgagcctcgattatcgtttcccggccagccgctacgggcagttcgggctcgacctgcaaggcacctacgtgtcccgctacgacttccagcagcagatcggcggccagtacctggacaacgtcggcgacttccagggcgtcggcgtgatcgcccgctggaagcacgtcgccaacgccacctggagccgcgacgcctggcaggccaccctgagcaaccgctacaccagcggctacaacgactacgaccgcgccagccacggcaaggtcggctcgtggaacctctgggacctggccggcagctaccgcctcagccacgcgctggggctgaccctcggggtgaagaacctgttcgaccgcgaaccgccgttcagcaaccagacctacaccttccagagcggctacgacccgcgctacaccgatccctacgggcgcatcctgttcggccgcctcagctacagcttctga

SEQ ID NO: 53 - DNA, 2760 bp, Pseudomonas aeruginosa
atggttcggcttcgtacactggttcgggcaatcgcggcggcctcggtcctgacttccggcatggcgcatggattgggactgggggaaatcaccctgaagtcggcgttgaaccaaccgttggatgccgagatcgagctgctcgaagttcgtgacctgggttcgggcgaggtgatcccgagcctggcgtcgccggaagagttcagcaaggcgggcgtcgatcgcctgtactacctcaccgacctgaagttcacgccggtggtgaagcccaacggcaagagcgtcattcgcgtgacctcgtcgaagccggtgcaggagccctacctgaacttcctggtccaggtgctctggccgaacggccgcctgctgcgcgagtacaccgtcctgctggatccgccgctgtactccccgcaggccgcggcaagcgctccgcaagcgccggtcagcgcgccgcgcgcgaccggcgccccgcgagccccgcaggctccggctccggtgcgtaccaccgcgccggcaggcagcgacacctatcgcaccgtttccaacgacacgctctgggagatcgcccagcgcaaccgtaccgatcgcgtttccgtaccccaggcgatgctcgcgttccaggagctgaatccgggcgccttcgtcgatggcaacatcaaccggctgaagagcggccaggtcctgcgcattcccaccgaacagcagatgctggagcgctcgccgcgcgaggcgctgtcccaggtgcaggcgcagaaccagagctggcgcggcagccgcaatccggccgcgggcagcgctggcgccaggcagttggatgcgacccagcgcaatgccgccgggtcggcgccatccaaggtcgacgccacggacaatctgcgcctggtgtctggcgagggcaaggccagcaagggtgccgacaagggcggaaagggcgacagcaaggcgatcgccgataccctggcggtgaccaaggaaagcctcgacagcactcgccgcgagaacgaagaactgcagagtcgcatgcaggatctgcagagccagttggacaagctgcagaagttgatccagctgaaggacgcccagttggccaagctgcaagggcagttgggcgccgaaggccagggcgcagcccagccgaacgcagccctgccggatgcgtcccagcccaatgcggccgcgcaggcgccggctcagcccgggactcctgctgcggcagcgccgactcctgctccagccggagaagcacccgccgctccggcgcagcctccggtggcgccgccgcccgcgccagctgccgagaagcctccggcacctgccgttccggcgcccgctccggtacaggcggcagagcagccggcaccgagcttcctcgacgaactgctggccaacccgctgtggttggcggtgatcggcggtagcgcactgctggcgttgctggtgctgctgatgatcctgtcgcggcgcaatgcgcagaaagagaaggaagaagcccaggctttcgccgcggataccggcgaggaacaggaggatgcgctggacctgggaaaggacggcttcgacgacctgaccctcgacgagcctgagccgcaggtcgcagccgtcgctccgcaggtcgagaagaccaccgcgcagacttccgatgcgctgggcgaggccgacatctatatcgcctacgggcgtttcaaccaggccgccgaactgttgcagaacgccatctacgacgagccgcagcgcaccgacctgcgcctcaagctgatggaagtctatgccgagatgggcgatcgcgaaggtttcgctcgccaggaaaacgagctgcgcgaaatcggcggcgcacagccgcaggtcgagcagctcaagtcgcgctatccggcaatggtcgcggtcgccgcggttgccggcctggccggcgccaagctggcgcaggacgagctggatagcttcagccttgacgacctgtcgctcgacgacagcggtcacgcggccaagccggatgcggcaggacaggatctcgacgacgccttcgacctgagcctggacgacctgggcggcgacgacgtgcaggccgacctcaagtccgacagcggggcgctggacgacctgaccctggacagcgatctggacctggcggcctcgaccccggcggacaagcctgtcgacgatctcgacttcggcctggatttcgcggagttggcagagactccgagccaacccaagcatgacgacctgggcgatttctccctggatctcgacgcgccggaagacaagctttcggacgacgacttcctgctttcgctgaacgacgaagtgcccgccgcggcgcctgccgacaacgaattcaccctcgataccgaggctgccgaagagccggcgttgtccctgccggacgacttcgacctgtcgctggccgacgagccgacggagccggccgctccggagaagggcgaggacagtttcgccgcccagttggacgaggtgagtgcgcagttggacgagttggccagcaaccttgacgagccgaagagcgcgacgccgagtttctccgccgaagatgcagcggtcgcctccgccctggacggagacgccgacgatgacttcgacttcctctccggtgccgacgaagcggcgaccaagctggatctggctcgcgcctacatcgacatgggcgatagcgaaggcgcgcgcgatatcctcgacgaagtcctggccgaaggtaatgacagccagcaggcggaagcccgcgagttgctggagcgcctggcctga

SEQ ID NO: 54 - DNA, 2988 bp, Pseudomonas aeruginosa
atgaccgacgaccactccttccgccctcgccccacctcgttgtcagccgccctgctgctgggcgcctggatcgcacagccggccacggccgcctatgtcgaagccggtcggcccggcgatccggccagttggcgctccgccgaataccagcaggactggggcctggaacggatgcgggccgaccaggcctatgccgccggcatcgacggccagggcgtgaagatcggcgagatggactccggtttcgacccgagccatccggatactcccgcctcgcgctaccagccggtgacggccagcggcacctatgtcgacggcacgccgttcagcgtcagcggcgcgatgaacggcaacaacgactcccacggtacccacgtcggcggcaccctcggcgcctcgcgcgacggcgtcggcatgcacggggtggcctacgcggcacaggtgtatgtcgccaacaccaaccagaacgacagcttcctgttcggcccgacgcccgacccgaactatttcaaggccgcctaccaggcgctggccgacgccggggtgcgggcgatcaacaacagttggggcagccagcccaaggacgtcagctacgagaccctcgacggcctgcacgccgcctatgcccagcactacgggcgctccacctggctggacgccgccgccggcgtctcccgccagggcgtgatcaacgtcttcagcgccggcaacagcggctacgccaacgccagcgtgcgctccgccctgccctacttccagccggacctggaaggccactggctggccgtgtccggcctcgaccagcagaacggccagcgctacaaccgctgcggcatcgccaagtactggtgcatcaccacgcccggccgcctgatcaacagcaccatgcccggcggcggctacgccaacaagtccggtacctcgatggccgcgccccacgccaccggcgcgctggccctggtcatgcagcgctatccgtacctgaacaacgagcaggcgctgcaggttctgctgaccaccgccacccagctcgacggcacgccgaccggcgcccccaccgacaccgtcggctggggcgtgccggatctcggtcgggcgatgcatgggcctggacaattgctcggccgcttcgaggccaacctcccggccggcctgcgcgacgaatggagcaacccgatttccgatagcgccctgctccagcgccaggccgaggacgccgccgagcacgcggcctggcagcggacgctgaaggacaagggctgggaaaacggcttgccggccggtgccagccagcaggaacgcaccgactatgccatcggcatggcccgcgaccaggccgccgcccagcgccagtaccagggcagcctggtcaaggccggtgccggcagcctggtcctgagcggcgacagcacctatcgcgggccgaccctggtcgatggcgggctgctcagcgtcgacggttcgctgctgtccgccgtcgaagtcaatgccggcggcaccctcggcggcagcggcaggatcggcggcctgctggcgcgctccggcggcacggtggccgcgggcaactccatcggcaccctggaggtcgccggggacctgcgcttcgaatccggctcgacctacgcggtggagctttcggaaagcgccagcgaccggatcgtcgccagcggcaaggcgagcatcgcgggcggcaacgtcaccctggccatggaaaacagccccgacctgctcagccagtcccaggtcgagagcctggtcggccgccgctacgacatcctcgacgccgccggcggcatcgacgggcgcttcgacgcggtattgccgaactacctgttcctcggcggcaccctggactacgcggccaacgccatccgcctggatatcggacgcaacggcacgaccctcgccagcgtcgcgcagacgcccaaccaggcggcggtcgctggggccgtggaaacgctcggcgccggcaacccggtctacgaaagcctgctcctgtcggaaaacgccgcaaccgcccaacgggccttccagcaattgtccggggaaatctacccggcgctcgccggcctgttgctcaacgacagccgctatctgcgcgacagcgtcggcgaacgcctgcgccagaccagcgacggcgaggccggcggggaggctcccgaaggctggttcaaggcgctcggctcctggggcaagagcgccgatggcagccacggtagcgaaggctaccggcattcggtcggcggcttcctgctcggcgtcgacagccaggtcgccagcgacacgcgcctcggcctggtggccggctacagcaacagctcgctgaacatggacagcagcctgcaatcctccgccagcatcgacagctaccacctcggcgcctacctcggccggcaattgcagcaatggcgcctgagcctcggcgcagcgcacgcctggcaccgcgccgaggtcaagcgcgacctgcaatacggcgccgtggccggcaagcagaaggccaagctcgacgcacagagcagccagttgttcgccgaggccgcctacgcgctgggttggcgcagcctggagctggaacccttcgccgggctggcctacgtgcacgtcgccagcgatgacttccgcgaacgcggtagcgccgcggccctggagggtggcgacgacaacctggacgccgccttcaccaccctgggcctgcgcgcgaaacggcatttcgagctggatgccggacgccgcctggcgctctccggcaccctcggctggcgccacaacctgagcgacaccaccccgcaacgccacctggcgttcgccagcggcagccagccattcagcgtggaaagcgtggccctgtcccgcgacgccgcgctgctcggcgtcgacgccagcctcgcggtgaatcgcgaagtgagcgtgcggctgggctacaacggcctgctgggcagccgcgagaaggaccatggcgtcggactggccgtcgactggcgtttctga

SEQ ID NO: 55 - DNA, 3174 bp, Pseudomonas aeruginosa
atgaaaagaatgctgatcaacgcgactcaacccgaggagttgcgtgttgcactggtcgacggccaacgcctgttcgacctcgacatcgagtcgggcgcccgcgagcagaagaaggccaacatctacaaaggccgcatcactcgcgtcgaacccagcctcgaagccgccttcgtcgacttcggcgccgaacgccacggcttcctccccctcaaagaaatctcccgcgaatacttcaagaaatcccccgaaggccggatcaacatcaaggaagtcctgagcgaaggccaggaagtcatcgtccaggtcgagaaggaagagcgcggcaacaagggcgccgccctgaccaccttcatcagcctggccggccgttacctggtgctgatgccgaacaacccgcgcgccggcggcatctcccgccgtatcgaaggcgaagagcgcaacgagctgcgcgaggccctgaacggcctcaacgcaccggccgacatgggcctgatcgtgcgcaccgccggcctcggccgcagcaccgaggaactgcagtgggacctcgactacctgctgcaactgtggagcgcgatcaaggaagcgtccggcgaacgtggcgcgcccttcctgatctaccaggaaagcaacgtcatcatccgcgccatccgcgactacctgcgccaggacatcggcgaagtgctgatcgacagcatcgacgcccaggaagaagccctgaacttcatccgccaggtgatgccgcagtacgccagcaaggtgaagctgtaccaggacagcgttccgctgttcaatcgcttccagatcgagagccagatcgagaccgctttccagcgcgaagtgaagctgccgtccggcggctccatcgtcatcgacccgaccgaggccctggtttccatcgacatcaactcggcgcgcgccaccaagggcggcgacatcgaggaaaccgccctgcagaccaacctggaagcggccgaggaaatcgcccgccagctgcgcctgcgtgacatcggcggcctgatcgtcatcgacttcatcgacatgaccccggcgaagaaccagcgcgccgtggaagagcgtgtccgcgaagccctcgaggccgaccgcgcgcgcgtccaggtcggtcgcatctcgcgcttcggcctgctggaaatgtcccgccagcgcctgcgtccgtccctcggcgagaccagcggcatcgtctgcccgcgctgcaacggccagggcatcatccgcgacgtcgagtcgctgtcgctggccatcctgcgcctgatcgaggaagaagccctgaaggaccgcaccgcggaagtccgcgcccgcgtgcccttccaggtcgccgccttcctgctcaacgagaagcgcaacgccatcaccaagatcgaactgcgtacccgcgcgcgcatcttcatcctgccggacgatcatctggaaaccccgcatttcgaagtccagcgtctgcgcgatgacagccccgaactggttgccggccagaccagctacgaaatggccaccgtcgagcacgaagaagcccagccggtcagctcgacccgcaccctggtccgccaggaagcagcagtcaagaccgtcgctccccagcagcccgcaccgcaacacaccgaagcaccggtcgagccggccaagccgatgcccgagccgagcctgttccagggcctggtgaagtccctggtcggcctgttcgcaggcaaggatcaacctgccgccaagcctgctgaaaccagcaagccggctgccgagcgccaaacccgccaggacgagcgtcgcaacggccgccagcagaaccgccgccgcgatggccgcgatggcaatcgccgcgacgaagagcgcaaaccgcgcgaggagcgtgcagagcgtcaaccgcgcgaagagcgcgccgaacgcccgaaccgcgaagagcgcagcgaacgtcgccgcgaagagcgcgccgagcgcccggctcgcgaggagcgccagccgcgcgaaggccgtgaagagcgcgccgagcggacaccccgcgaagagcgccagccgcgcgaaggccgcgaaggtcgcgaggaacgcagcgaacgccgccgcgaagagcgcgccgaacgcccggcccgcgaagagcgccaaccccgcgaaggccgtgaagaacgcgccgagcgcccggcccgcgaagagcgccagccgcgcgaggatcgccaggctcgcgacgccgcggccctggaagccgaggcattgccgaacgacgagagcctggagcaggacgagcaggacgataccgatggcgagcgcccgcgccgccgctcccgcggccagcgtcgtcgcagcaaccgccgcgaacgccagcgcgaggtcagcggcgagctggaaggcagcgaggcgaccgataacgccgccgcgccgctgaacaccgtcgcagccgccgccgctgccggtatcgctgtcgccagcgaagccgtagaagcaaacgtggagcaagccccggccactaccagcgaggctgccagcgaaaccacggcaagcgatgagaccgacgcgtcgaccagcgaagccgtcgaaacccagggcgcggacagcgaggccaataccggcgaaaccgccgacatcgaagcgccggtgaccgtcagcgtggtccgggacgaagccgaccagagcaccctgctggtcgcgcaagccactgaagaagctcccttcgccagcgaaagcgtggaaagccgcgaagacgccgagagcgccgtgcaaccggcaacggaagcggccgaagaagttgccgctccggtgcccgtcgaagtagcagcccctagcgagcccgcagccaccgaggagccgaccccggccatcgcggcggtgccggccaacgcgactggccgtgccctcaacgacccacgggaaaaacgtcgcctgcaacgcgaagccgagcgtctggcacgcgaagccgcagcagcagccgaagcggcagctcaggccgctcccgccgtcgaggagatcccggctgtagcgagcgaggaagcgtcggcccaggaggaacctgctgcaccccaggctgaagaaatcacccaggccgacgttccgtcccaggcggacgaagcccaggaagcggtacaggccgagcctgaagcttccggcgaaggcgccgccgacacggagcacgcgaaaaagaccgaggaaagcgaaacctcgcgcccgcatgcctga

SEQ ID NO: 56 - DNA, 3486 bp, Pseudomonas aeruginosa
atgaaatcggtactccaccagatcggcaagacctcgctggcagccgcgctcagcggcgccgtcctgctctccgcccagaccacccacgccgccgccctgtcggtcagccagcagccgctgatgctgatccagggcgtcgccccgaacatgctggtgactctcgacgactcgggcagtatggcgttcgcctatgcgccagacagcatttccggctatggaaactatacgttcttcgcgtcgaacagcttcaacccgatgtacttcgatccgaacacgcaatacaagcttccgaagaaactcacactggtgaacggacaggtacagatccaggattatccggcccccaacttctcctctgcctggcgcaatggcttcactcgcagcgggagtatcaatctgtcgaacagctacaaggtcaccatcgagtacggcaggggatatgataaggagtcgacgataaaagccgacgctgcctactactatgacttcacgggctcatccagttgcaaccgcaccaatcaggcatgctacacccgccgttatgtgagcacagagcaaaggcagaacttcgccaactggtattcgttctaccgcacccgcgcccttgccactcagaccgccgccaacctggcgttctacagcctgcctgaaaacgctcgggtgagctggcaattgctgaacgactcgaactgcaaccagatgggcagcggctccagctccggcaactgtttcagcaactatctacgggacttcaccggtcaacaccgggtgaacttcttcaattggctggaaaaactttcggtcaatggtggtacgccactgcgccaggcgatgacccgggcaggcgagtttctcaagaagaccggcgtcaacggtccctatgcctatcgcccagggacccagaccgcgcccgagtacagttgccggggcagctatcatatcctgatgaccgacggtctctggaacaacgactcggccaacgtaggcaatgccgacagcaccgctcgtaacctccccgacgggaagagctatagcagccagacaccctacagggacggtacgttcgataccctggccgaccaggccttccattactgggccaccgatgcccggccggatatcgacgacaatatcaaaccgtacattccctacccggaccaggccaatccctcggcggaatactggaatccccgcaacgatccggcaacctggcaacacatggtgacctacaccctgggcctgggcctgaccaccagcctcaccagtccgagatgggaaggctccaccttttccggtggctacaacgatatcgtggctggcaacctgagctggccccgcgcgtcgaacaacgactccaacaacgtctacgatctgtggcacgccgcagtgaactcccggggcgagttcttcagcgccgactcgccggaccaactggtcgcggccttccaggacatcctcaaccgaatttcgggcaaggacctgccggcatcccgccccgccatcagctcgtccctgcaggaagacgacactggcgacaagctgacccgcttcgcctaccagaccagcttcgccagcgacaagaactgggctggcgacctgacccgctacagcctgaccacccaggacaaggccaccgtgcagaccaagctgtggagcgcgcagagcatcctcgacgcgatgcccaacggtggagctggccgcaagatcatgatggccggatccggtacctcgggcctcaaggagttcacctggggcagcctcagcgccgaccagcagcggcagttgaaccgcgatccggaccgcaacgatgtcgccgacaccaagggccaggaccgcgtggccttcctgcgcggcgatcgccgcaaggagaacagcgacaacttccgcacccgcaactcgatcctcggcgatatcatcaactcctcgccggcgacggtcggcaaggcccagtacctgacctacctggcccagccgatcgagcccagcggtaactactccacgttcgcagaagcacagaaaacccgtgccccgcgggtatacgtcggcgccaacgacggcatgctgcacggtttcgataccgacggtaacgagaccttcgccttcatcccaagcgcggtcttcgagaagctccacaagttgaccgcccgcggctaccagggcggcgcccaccagttctacgtcgacggttcgccggtggtcgccgacgccttcttcggcggcgcctggcataccgtgctgatcggcagcctgcgcgccggcggcaagggcctgttcgccctcgacgtgaccgatcccgccaacatcaagctgctctgggaaatcggcgtggaccaggagcccgaccttggctacagcttccccaaacccacggtcgcccggctgcacaacggcaagtgggccgtggtcaccggaaacggttattccagcctgaacgacaaggccgcgctgctgatcatcgacctggagaccggggccatcacccgcaaactggaagtcaccggcaggaccggcgtacccaacggcctatccagccctcgcctggcagacaacaacagcgacggcgtagccgactacgcctacgccggcgacctgcaaggcaacctctggcgcttcgacctgatcgccggcaaggtcaaccaggacgatccgttcagccgagccaacgacggcccggcggtggcctcgagcttcagggtgtctttcggtggccagccgctctattcggcagtcgactccgccggcgcggcgcaagcgatcaccgccgcgccctcgctggttcgccatccgacacgcaagggctacatcgtgatcttcggtaccggcaagtatttcgagaacgccgacgcccgggccgataccagccgcgcccagacgctctacggcatctgggaccagcaaaccaagggcgaagccgcgggcagcacaccccgactgacgcgcggcaacctgcagcagcagaccctggacctccaggccgactcgaccttcgcctcgaccgctcgcaccattcgcatcgccagtcagaacccggtcaactggctgaacaatgacggcagcaccaagcagtccggctggtatctggacttcatggtcaacggcaccctgaagggcgagatgctgatcgaggacatgatcgccatcggccaggtggtgctgctgcaaaccatcaccccgaacgatgacccctgtgccgacggcgccagcaactggacctatggcctcgatccctataccggcggtcgcaccagcttcaccgtgttcgacctggcacgccagggcgtcgtggactcgaaatccgactacagctacaacaagcagaacgtcgcggtatccggtaccgagcagaaaggcctgggaggcttgacgctgagcaccaacgaacagggcaatccggaagtctgctcctcgggcgaatgcctgaccgtgaaccccggtccgaacacccgtggccgccagaactggcgccccatcgaaggaaagaactga

SEQ ID NO: 57 - DNA, 3636 bp, Pseudomonas aeruginosa
atgaagattctcgccatccgcctgaagaacctcgcctccctcgctggcgagcaggaaatcgacttcacccgcgaaccgctgtccagcgccggcctgttcgccatcaccggtccgaccggcgccggcaagagcaccgtgctggacgccctgtgcctggccctgttcggcagcacgccgcggctggaaagcacttcggccagcagcaaggttcccgatggccggaacgagctgtccagcaacgacgaacgcaacctgctgcgccgcggttgcgccagcggctacgccgaagtggatttcgtcggcatcgacggccaccgctatcgcgcccgctgggaaacccggcgctcccgggacaaggcggacggcgccttgcaaaagagccagcagagcctccaggacctggagacccagcaaatgctggcagcgaacaagaaaagcgagttccgcgaacagctggagcagaagctcggcctcaatttcgcccagttcactcgcgccgtgctgctggcccagagcgaattcagcgccttcctcaaggccagcgacaacgaccgcggcgcattgctggagaaactcaccgacaccggcctgtacagccaattgagcaaagccgcctatcagcgcgccagccaggccgacgagcagcgcaagcaactcgagcaacgcctggaaggcagcctgcccctggccgagcaggcccgggccgggctcgaggcggcgctggaatcccacgcccaggcgcgtctccaggagcaacaggcactgcaacgtctggaaggccagcaacaatggttcaccgaggagcagcggctgctgcaatcctgcgagcacgcacaaggccaactggccgaggccaggcaggcctgggacgccctggcgacggagcgggaaaccctgcaatggctggagcgcctggctccggttcgcggactgatcgaacgcctgaagcaactcgagcaggaactccggcactccgagcagcagcagcggcagcgcaccgagcagcaagccgcgggcaccgagcgcttgcaaggattgcaggcccgcttgcaggaggcgcgcgagcgccaggcccaggccgacaaccatctgcgtcaggcccaggcgccgttgcgcgaggctttccagctggagagcgaggccaggcgcctggagcgaacgctggccgagcgacaggaactccatcggcaatcgaaccagcgccacgcccagcaaagcgacgccgctcggcaactggatatggagcagcagcgccatgtcgcggaacaggcgcaactgcaggcggcattgcgcgacagccaggctctcgccgcgctcggcgacgcctgggtgacccaccagggccagctcgccaccttcgtgcaacgtcgccagcgcgcgctcgaaagccaggcgcagctccccgagctggaaaaatccctggcccacgccggggaaccgctcgaacgcttgcaggcgcaatggaccgccctccatggcagcgagccggacgacctggcggcacgcctggtcgaattgcgccggcagaccgatagcctggaacgacaacaagcgctccacaaggaatggcaacaggtcctcgaccaacgcgccggtctggctcgacgcctgggcgaactcgaccagcgtatggtcgagcaggagcaggcattgctcgacctgaaacgacaaggcagccaatgcgccgaggaggtgaaggcggcggagcaggccctgcaggtcacccgcgagttgctccagcgccaacgtctggcccgcagcgccagcgtcgagcaactgcgcgccggcctggtggacggcgaggcctgcccggtctgcggcagccaggagcatccctatcaccattccgagcaactgctcgccgccctcggtgaacacgacgaccaggagcaggtccgcgccgagcagtccctcgagcggctgcgacagaccctggtcggtctgcgcgagggctattccagccagcgggaaagactcaaccagagtcgccaggagcagcaggaactgactggccaactggccgcgctcgatcggcaactggaccaatggacgctgccggaagaactgcgactcctgcagccgtccgcgcagttggagtggctggcacaacgcctggacgacctggcagggcagcgccagcagtgccaacgagacttcgaccggctgatcgcccgccagcgccagacccagcaattgcagcaggaactgcgggccgccgagacgatcctgcaacagcgccagcaggcgctgacggaacaacggcagcgctacgaacatttgcagcagcaggtcgaggaggacagccagcaattgcgtccattgctctccgacgagcactggcagcgctggcaggcagatccgctgcggactttccaggcactcggcgagtccatcgagcaacgccggcagcaacaggcgcggcttcagcagatcgaacagcgtctgcaggagctcaagcagcgctgcgatgaatcgagctggcaactgaagcaaagcgacgagcaacgcaacgaagcccgtcaggcagaggaaagggcccaggcggaactcgccgaactgaacggacgcctcggcgctcacctgggccagcacgcctgcgcccaggactggcagctatcgctggagcacgccgcgcaagcggcgcagagcgccgtcgagacgctccaggcgcccctggattcgctgcgcgaggaacaactgcgactcgccgaagccctggaacacctgcagcagcaacggcagcgccaacaggatgagttccagcgccttcaggccgactggcaggcctggcgcgaacgccaggacaacctcgacgacagccgcctcgacgccctgctcggcctttccgaggaacaggcgacgcaatggcgggagcaattgcagcgactgcaagaggagatcacccgccagcagacactggaagcagagcgccaggcgcaactgctccagcatcgccggcagcggccggaaaccgaccgcgaggcgctggaagacaacctgcggcaacagcgcgaacgcctggccgccagcgaacaggcctacctggagacctacagccagttgcaggccgacaaccagcgccgcgagcagagccaggcgctgcttgccgaactggagcgagcccgcgccgagttccgcagatggggccgcctgaacgaactgatcggttcgtccagcggcgacaagttccgccgcatcgcccagggctacaacctcgacctgctggtgcagcacagcaacgtgcagttgcgccagttggcgcggcgctaccgcctgcagcgcggcggcagcgaactgggcctgctggtggtggacaccgagatgggcgacgaactgcgctcggtgtattcgctctccggcggcgagaccttcctgatttccctggccctggcgctcggcctggcctcgatggcatcgagcaagctgcgcatcgagtcgctgttcatcgacgaaggcttcggcagcctcgacccggaatccctgcaactggcgatggatgccctggacaacctgcaggcccagggacgcaaggtggcggtgatttcccacgtccaggaaatgcacgaacggatcccggtccaggtgcgggtccagcgcgagggcaacggcatgagcagcctgaaggtggtcggctga

SEQ ID NO: 58 - DNA, 7407 bp, Pseudomonas aeruginosa
atgtcgatccaggcgaaagttacccctatcgatcagagtatttcttctgcggctgccgtcgaggttccggaaaacgggatactcaaactctcccagagcagtaatgtcgcgctcgatgtcgcaccggagtcggtggcgggatactcgaagagcggttcggacctgatcgtccagctgaagaccggggaaagcgtccggatcgccaacttctatgcggaaggccagccttccagccaactgttcctggccgacaaggacaagctggtggcggtagatctgccgccggtcgctgccgacgggccgctgatggccggctacatcccgcaggaaagcctggccggtttcgagtcgctgaccggcgccggtgtgctcggtggcatgagcgcagggactgcgctgctggtcggtgcggcggccatcggcgccggggtggcgatttccaacagcagcggcggcggtggcggcggcggttcttcggtgcccccggacaccactccgccgaaggcggccagcggcctgaagatagcgcctgacggcagcagcatcagcggccaggccgaggccggcgcgagcgtcggcatcgataccaatggcgacggcaagccggacctcaccgtgatcgccgatgccaacggcaatttcaccgctccgctgaacccgccgctgaccaatggccagacggtcaccgtggtggtcaccgacccggctggcaacgccagcccgccggcccaggtcaccgctccggacactaccgccccggcgccggctaccgacgtgcaggtggcgccggacggcagcagcgtcaccggcaaggccgaacccggctcgacggtgggcgtcgataccgacggcgacggccagccggacaccaccgtggtggtcggccccggcggcagcttcgaggttccgctgaacccgccgctgaccaatggcgagacggtgacggtgatcgttaccgacccggccggcaacaacagcaccccggtgaccgtcgaggcgccggacaccaccgccccggcgccggccaccgacgtgcaggtggcgccggacggcagcagcgtcaccggcaacgcagagccgggcgccaccgtcggtgtcgacaccgatggcgacggccagccggacaccaccgtggtggtcggtcccggcggcagcttcgaggttccgctgaacccgccgctgaccaatggcgagacggtgacggtgatcgttaccgacccggccggcaacagcagcaccccggtcaccgccgaagcccccgacttccccgacgcgccccaggtcaatgccagcaacggcagcgtcctcagtggtacggcggaagcgggcgtgaccatcgtgatcaccgacggcaacggcaatccgatcggccagaccagcgccgatgccaacggcaactggagcttcacccccggtagccaactgccggatggcaccgtggtcaatgtggtggccagggacgccgccggcaacagcagcccggcgacctccatcaccgtcgacggcgtggcgccgaacgcgccggtggtcgagccgagcaacggcagcgaactcagcgggactgccgaaccgggcagcagcgtgaccctgaccgacggcaatggcaatccgatcggccagaccaccgccgatgccaacggcaactggtctttcacgccgtccaccccgttgccggacggtaccgtggtcaacgtggtggccagggatgccgccggcaacagcagtccgccggccagcgttaccgtggatgccgtcgcgccggccacgcccaccgtcgatccgagcaacggtacgaccctcagcggcaccgccgagccgggcagtagcgtgaccctgaccgacggcaacggtaacccgatagggcaggtcaccgccgacggcagcggcaactggaccttcaccccgagcacgccgttgcccaacggcacggtggtcaacgccacggctaccgacccgtccggcaacgccagttcgccggccagcgtcaccgtggacgccgtggcaccggccacgccagtggtcaacccgagcaacggcaccacgctcagcggcaccgccgagccgggcgccaccgtgaccctgaccgatggcaacggcaatcccatcgggcaggtcaccgccgatggcagcggcaactggagcttcactccgaccacgccgttgcccaacggcaccgtggtcaacgccacggccaccgacgcctccggcaacaccagtgcgggcagcagtgtcaccgtggactcggtagccccggccacgccagtgatcaaccccagcaacggcaccacgctcagcggcaccgccgagccgggcagcagcgtgactctgaccgatggcaacggcaacccgattggccaggtcaccgccgacggcagcggcaactggagcttcaccccgtccacgccgctggcggatggaaccgtggtcaacgccacggccaccgatccggcgggcaacaccagcggccagggcagcaccaccgtcgatggcgtggcgccgaccacgccgaccgtcaacctgagcaacggcagcagcctcagcggcactgcggaaccgggcagcacggtgatcctcaccgacggcaacggcaatccgatcgccgaggtcaccgccgacggcagcggcaactggacctacaccccgtccacgccgatcgccaacggcaccgtggtcaacgtggtggcccaggacgccgccggcaatagcagcccgggcgccagcgtcaccgtggactcgcaggccccggcggctccggtggtcaacccgagcaacggcactacgctcagcggcaccgccgagccgggcgctaccgtgaccctgaccgacggcaacggcaacccgattggccaggtcaccgccgacggcagcggcaactggagcttcacaccgggcacgccgctggccaacggcaccgtggtcaacgccacggccagcgacccgaccggcaataccagcgctccggccagcaccaccgtggactcggtggcgccggccgcgccggtggtcaatccgagcaacggcgcggagatcagcggcaccgccgaaccgggcgccaccgtgaccctgaccgatggcagcggcaatccgatcgggcaggtcaccgccgacggcagcggcaactggagcttcaccccgtccacgccgctggcggatggaaccgtggtcaacgccaccgctaccgacccggccggcaataccggcggccagggcagcaccaccgtggacgccatcgcgccggccacgccgaccgtcaacctgagcaatggcagcagcctcagcggcaccgccgagccgggcagcacggtgattctcaccgacggcaacggcaatccgatcgccgaggtcaccgccgacggcagcggcaactggacctacaccccgtccacgccgatcgccaacggtactgtggtcaacgtggtggcccaggacgcctccggtaacagcagcccgccggcgacggtgaccgtcgattccagcgcgccgccggcgccggtgatcaacccgagcaacggcgtcgtcatcagcggcaccgccgaggccggtgccacggtgaccctcaccgatgccggcggcaacccgatagggcaggtcaccgccgacggcagcggcaactggagcttcacgccgggcaccccgctggccaacggcacggtgatcgtcgccacggccaccgacccgaccggcaataccggcccgcaggccgccaccacggtggacgcggtggcgccgccggcgccggtgatcgatccgagcaacggcacgaccatcagcggcaccgcggaggccggggccaaggtgatcctcaccgacggcaacggcaacccgatcggcgaaaccaccgccgacggcagcggcaactggagcttcacgcccggcacgccgctggccaacggcacggtggtcaacgccgtggcccaggaccctgcgggcaataccggcccgcagggcagcactaccgtggacgcggtggcgccgaacacgcctgtggtcaatccgagcaacggcaacctgctcaacggtaccgccgagccgggcagcaccgtgaccttgaccgacggcaacggcaacccgatcggccagaccaccgccgatggcagcggcaactggagcttcacgcccggctcgcaactgcccaacggcaccgtggtcaacgtgaccgcgagcgacgccgccggcaataccagccttcccgctaccacgacggtggattcctcgctgccgtcgatcccgcaggtggatccgagcaacggttcggtgatcagcggcaccgcggacgccggcaacaccatcatcatcaccgatggcaacggcaacccgattggccaggtcaccgccgacggcagcggcaactggtccttcactccaggcatcccgctgccggatggcacggtggtcaacgtggtggcgcgcagcccaagcaatgtcgacagtgcgccggcggtgatcactgtggatggcgtggccccggcggcgccggtgatcgatccgagcaacggcaccgagataagcggtaccgcggaggccggcgcgacggtgatcctcaccgatggcggcggcaacccgatcggccaggccaccgccgacggcagcggcaactggacgttcaccccgagcaccccgctggccaacggcaccgtgatcaacgccgtggcccaggacccggccggcaataccagcggtccggccagcgtcaccgtcgatgccatcgccccgccggcgccggtgatcaatccgagcaatggagtcgtcatcagcggtacggcggaagccggggccacggtgatcctcaccgacggcaacggcaacccgatcggccaggtcaccgccgacggcagcggcaactggagcttcacgcccggcacgccgctggccaacggctcggtgatcaatgcgctggcccaggacgccgccggcaacaacagcagtcccaccagcgccaccgtcgactcgctggcgccagcagccccggtgatcgatccgagcaacggtagcgtgatcgccggtaccgccgaggctggtgccacggtgatcctcaccgacggcaacggcaacccgatcggccaggtcaccgccgatggcagcggcaactggagcttcacgcccggcacgccgctgtccaatggcacggtggtcaatgcggtggcccaggacgctgccggcaacaccagcggcccggtcagcaccacggtggacgcggtggccccggccaccccggtgatcgacccgagcaacggtgtcgaactcagcggcaccgccgaacccggcgtccgggtgatcctcaccgatggcaatggcaatccgatcggccagacccttgccgacggcagcggcaactggagcttcacgccgggcacgccgctggccaacggcacggtggtcaatgccgtggcccaggacccggccggcaataccagcggcccggccagcaccacggtggacacggtggctccggccacgccggtgatcaatcccagcaacggcagcgtgatcaccggcaccgccgaggtcggcgccaaggtgatcctcaccgatggcaacggcaacccgatcggcgagaccaccgccgacggcagtggtaactggaccttcacccccggcacgccgctggccaacggtacggtgatcaacgccgtcgccgaggacgccgcgggcaacgccagcggtccggccagcaccacggtggactcggtggcgccgtccgctccgctgctgagcatcagcgccgacggcgcgctgctgaccggcaccgccgagccgaacagccaggtgcgcatcgtggtcaacggcgacaccgccaacccgatcacggtcaccgtcgacggcgccggcaacttcagcctgccgttcgcgccgccgctgatcaccggcgagctgatcgccggggtcgccgtcgacgccgccggcaacgtcagcgggccggccaccatcaacgccccggacctggcgccgccgaccatcagcgtgccggaagccgccgatacctggatcaatgccgcggagatcggcgacggtatccaggtcgatgtgacggtccgtccgaccatgcaggtcggccaggtggtcacggtcaagttcgccgggcagaacggctacgaggccgaggtcagccataccctcaccgccggcgacatcgccgccggcaacctgaccctgaccctgacgcctcccggcggcatgggcccgttcccggagggtgcctcgaccgtcaccgccgacatcaacggcggcaccgcgtcgaccccggtgccgttcaccatcgacaccattccgccggcgaccccggtgctgtccctggtcggcaacatcctgaccatctcggcggagccagggaccgagttgacggtgaccgtcgacgtcggcggggtgaccgccaccgccacggtgaccgccgacaacagcgggctggcgtcgctgaacctgctcaccgacctggacatcgacttcagttgggaccagttgctcaatgcccaggtgtcggtggtcggacgcgacccggccggcaacccgagcaacacggcgagcatcggcgtcggcaccagcatcgagcaaccggtgaccatcggcaacttcggcctcgacgtcagcctcaacccgctgaacccgcgtttcggtttcagcggaaccaccgagcctgactccagcgtggtgatccgggtcatcaccccggcgttgaacgtcgaattgctgccgatccaggcggattcgtccggaaacttctcgctgaacctgctgagcccgaccatcctcacccagttggggctgaacatcaccgacatcctcaacctcggctcgcagatctcgttcaacctggtgtccaccgactccaatggcaacgacagcgccgcctacgggatcaccctgacccccaacggactgtcgctcaatatcggccagatcgatgtcaacggtacttccggcgacgacgtgctgtccggcgccaacggcagttcggagcacatcaacggcggcgacggcagcgacctgatcttcaacgtgggcaccggcgatcacgtggtggccggcaacggcaacgacaccatccagatcaccgcgaccgatttcgtcagcatcgatggcggcgccgggttcgacaccctggtcctggccaacggcatcgacctcgactacaacgccgtcggcgtcggcacgctcagcaacctcgagcgcatcgacctcggcaagggcgattcgggtagcgtgctgaccctgaccgcggcggaggtggatgccatcaccgatgccaacaacacgttgcagatcaccggcgagaacaacgacaccctgaacgtggtgggcgcggtgaataccggtaccacgcaactgatcaacggcattacctacgacgtctacaccttcggcagtaccaccctgctgatcgaggacaacacggtacaggtcgtggtctga

SEQ ID NO: 59 - DNA, 10608 bp, Pseudomonas aeruginosa
atggacatccgcagcccgctgaaccagtgcatcgccctgtccctggccggcatcttgttcctcaacccgatcgtcgccgcggcggcggggctggcgctggacaaggccgccggcggcaacaccggcctgggccaggcgggcaacggcgtgcccatcgtcaatatcgccacgcccaacgacgccgggctgtcgaacaaccatttccgcgactacaacgtcggcgccaacgggctgatcctcaacaacgctaccggcaagacccagggtacccagctcggcgggatcatcctcggcaaccccaacctcaagggccaggcggcgcaggtgatcctcaaccaggtcaccggcggcaaccgcagcaccctggccggctacaccgaggtggccgggcagtcggcgcgggtgatcgtcgccaacccgcacggcatcacctgccagggctgcggcttcatcaacacgccgcgcgcgaccctcaccaccggcaagccgatcatggacggccagcgcctggagcgcttccaggtggacggcggcgacatcgtcgtcgaaggcgccgaactgaacgtcggcaacctcgaacagttcgacctgatcacccgcagcgccaagctcaacgccaagctctacgcgaagaacctcaacatcgtcaccggccgcaacgacgtccaggccgacagcctgcaggccacgccgcgcgccgccgatggcagcgagaagccgcagctggcgatcgacagctcggcgctgggcgggatgtacgccggggcgatccgcctggtcggcaccgagcagggcgtgggggtgcggctggccggcgacatggccgccagcggcggcgacatccgcatcgacgccagcggcaagctgagtctggcccaggcctccagccagggcgacctgaagatcgcggcccaggccgtggagctgaatggcaagacctacgccggcggcagcgccgagatccgcagcgcggaggaactggtcaaccggcagagcctggcggcgcgcgaacgcatcgtgctggaggcggcgcatatcgacaacgccggggtgatcgaagccggcgtcgagccagacgagcgacgcaacgcgcgcggcgacctcgagctgcgcagcggcaccctgcgcaacgccggcagcctggtggccagccgcgcgctggaagcgaaggcgagccaggcgctggacaaccagggcggcagcctgaagggggcgaccgtccgggtcgacgccgggcacctggacaaccgtggcggcaagctgctcgccgagggcgaactgcgggtcgaggcgagcagcctggacaaccgccaggacggcctgttgcagagccgggaccgcgccgtggtcaagacccgtggcgatctcgacaaccgtggcggccaggtgatcggcctgaacgatctggaggtcggcgcggcgacgctcgacaacggccagcaaggcctgctcggcagccagcagtccacccgcgtcagcgcccaggcgctggtcaaccggggggacggcgaagtctccggcaagcgcgtcgaggctcgcgtcggtagcctcgacaatcgcggcggcaagctgatcggcgacgacctgctggtggtcgccagcggtgccatcgacaaccgcctcggcttgttctccgcagccaaccgcctcgacctgcgggcgcgcagcctggacaacagcggcaagggcacgctgagcagccggggcggcctggaggtcagcctcggcggcctgctggacaaccgcgatgaaggcaacctgctcagccagggcgcgcagcgcgtgacggtggggcaactggacaaccgcgccggcggcctgctgtcgagccgcagcgagttgaacgtccacggcgccagcctggacaaccgtggcggcgtgctggtggccgacgccggcctgagcgccacgggaggcgccttcgacaaccgcgacggcggcagcgccagcggcaaggctggcgtgcgcgtggaggtcgccagcctgcgcaacgaccagggtggcaagctgctcagcgatggccgcctggacctcgcagcgaacgccgtcggcaacgccggagggcgtatcgccgccaagggcgacctgcaggcgacgcttggcagcctggcccagcaaggtggcgaactggtcagcgaaaagaccctgaaggtcgcggccgacacgctcgacaacagccagtccgggctgatcgccgcgaatggcggcatcgctatcgaggcgcggcaggtcgacaaccgcgccggcgagatttccagcacctcgaaggtcgccgtgaacgcccgcgagcaactggacaaccgcggcggcaaggtcatcggcgacagcggcctgcgcctcaccgtgcagcgcctgctgaaccaggccaagggggtgctggccgggcgcgacggcctgagcctggacggcggcgaactgttcaacggcgacggcggtcggctcgacagccagaacagcctgagcgtgagcctcggcggcgtgctggacaaccagggcggcgcgctggtcagcgaaggcagcctgacggcgcgcgccgcgcgcctggacaaccgtggcgggaccttctccagcgccggtgcgctggcgctgaccagccaggccgcgctggacaaccagggcggcaggctgctcagcgatgccggcgtgacgctgcagggcgccagcctcgacaacagccgttccggcgtgatcagcgccaagggcgcggtggatatccgcaccggcgtactggacaacagccgcaacggcggcatcggcagcaacgccggcatcaccctggtggccgcccggctggacaacggccagcagggccgggtcagcgccaagggcctgctcgacgccaacctgaaaggcctcgaccagcgcggaggcggcgtcctgatcagcgaaaccggcgtcaccctcgacctcaatggcggcacgctggtcaaccgcgacggcggcctgatcgccacgcccggcgcgctgctgctgcgccagctcggcgcggtggacaacggcgccggcggggaaatctccagcgaccgcgccttcaccctcgccgccgccagcctggacaaccgcggcgggcgcctgatcggcgccgccaacctgaccctgcgcatcgcccaggccctggacaacagcctggccggggtgatctccggcgccgccggcctggacatcgcggccgctcgcctggacaacagcgccaagggcaccctggccagccgcgccggcatcgacctgcgcgtcgatggcgcgctggacaaccacgccgaaggcaccgtctccggcgcccgcctgacgctcgccagcgcctcgctggacaacagcggcaagggcctgctctccggcaacgccggcctgagcgtcgccactggcgcgctggacaacgccgagggtggccagttgatcagccagggcgtcctggacgtcagcagcgccgacctcgacaaccgtggcggcgccctcagtggcaagcagtcgctgcgcctgagcgccgccaacctggacaaccgtggcggcctgctcaccagcgacggcgaactggaactgacggcagggcgcgtcgattccgccgacggcggcgaaatctccgcccggggcgacctgcgcctgacggtcgagcgcctggtgcaacgccagggccggctggtcggcgagcgcggcgtcagtctcgacctgcggggcggcgacctggacaaccagggcggcctgatcagtgcccgcggcccgctgagcatcgagcggctgagcgtcctcgacaaccgccagggcggcgagatttccagccagcagggcttcgagctgctggccaggcgcatcgacaacggccagcaggggcgcatcatcagcgccgggaaactgcgcctagacgccgacgcgctgggcaacgccggcgccggcctgctctccggatggcagggcctgacggtgacaggcgggagcctggacaacagcgccggcggcaccctttcgagcaaggacggcgagctggccatcagcctcggcggcgcgctggacaaccacggccagggcgcgctggtcagcaagggcgcgcaacggatcgacgccgccagcctggataacgcccagggcattgtctccggcgaaagcgacgtgaccctgagcatcgccgggaagctggacaacggccagggcggcctggtctcggcgcagcgcgcgctgagcttcgagcgcgacgatacgctgctgaacaacgccggcggccggatcaacggcggcagcctgctgctcaagggcgccagcctggataacagcgacggccagttgatcagccagggccggctcgacgccatcctcggcggcgccctggtcaacaccggcgcggcgcgcctggccagcggcggcgacctgctgctgcgcagcgccagcgtcgacaaccgcggcggcaagctggtcagccaggggctgctggagatcagcgccggcagcctcgacaacagcgcctccggcaccctcgccagccaggccggcatgagcctgcgcctgggcggcggcgccctgcgcaaccagcaggacggcctgatcttcagccaggccggcgccctcgatgtgcaggccggcagcctggacaaccgccagggcacgctccaggcccagggcgacaaccggctgcgtatcggcggcgcgctggacaaccagggcggccgcctggacagccgggccggcaacctcgacctgcagagcggcagcctcgacaacggcgccggcggcgtgctcaacagcgccaagggttggctgaagctggtcaccgggctgttcgacaacagcgccggcgtcacccaggcgcagtcgctggagattcgcgccgggcaaggcgtgcgcaaccagcagggccacctctcggcgctgggcggcgacaaccgcatcgtcaccgccgacttcgacaaccagggcggcggcctctacgccagcggcctgctcagcctcgacggccagcgcttcctcaaccagggcgcggcggcgggccagggcggcaaggtcggcgccgggcgcatcgacttcagcctggccggcgcgctggccaaccgcttcggccagttggaaagcgaaagcgagctgcacctgcgcgccgccgcgatcgacaacagcggcggcagcctgcgcgccctcggccgcagcggcagcacgcggttggtcgctggcggcctgaacaacgcctacggcgtgctggaaagcgccaaccaggacctcgacctgcaactgggcagcctggccaacgccggtgggcgcatcctccacaccggcaatggcaccttcggcctggattccgggcaggtgatccgcgccggcggcgaactgaccaccaatggcctgctggacatccgcgccagcgaatggaccaacagcagcgtgctgcaagccggacgcctgaacctggacatcggcaccttccgccagacggccgagggcaagctgttggcggtgcagtccttcactggccgcggcggcgactggagcaacgacggcctgctggccagcgacggcagcttccgcctcgacctgagcggcggctaccgtggcaacggccgcgccaccagcctcggcgacttcgccctgaacgccgccagcctcgacctcggcaacgccgccagcctcgccggcggtgccaatgtcacgctcggcgccggcaacctgctggtcaaccgtgggcggatcaccgccgccggcgacctcgtggccagcgccgcgagcctgaacaactacggcaccctgggcggcggcggcaacctgcgattgaacgcgcccgccctgctcaacgagcgcgggttgctgttcagtggcgccgacatgaccctgcgcgccggcgacatcaccaacctctacggggatgtgtacagcctcggcaggctggatatcgcccgcgacgatgcgggcaaccgtgccgccagcctgcgcaacctttccggggtgatcgagagcggcaaggacttcagcctgcgtgccagcctgatcgagaaccgtcgcgccgtgctggaaagcaagtcgggcctgtacaccgcgaagatggagcagaccgcctgcatcgaaggcgtcaacgcgggcgactgcagcggcaagcgcaacgccatctggaccatcacccagcgcgacaagaccgaggtcaccgccagcagcgccatggggcaactgctggccggaggcgacttcgccatcgacggcggcaccctgaacaacctttccagtctgatcggcagcggcggcaacctcaccgccaacctcgaagtcctcgacaaccagggcctggaaaccggcgagctggaaaccatccgcgtgctgcgtaccgctcgcggcggcgatatcggcggcatcgaccagaagtcgcgcaacttcaccaacctctactggtaccagagcgccaatttcgacccggcgcgcgcgggcgagatccccgccgcgctcaacgcgatcctcagcgactggtccttcgagtacgaattcccgagcaaggggccgaccccgatcagcagtggcgaccagtcctacgcagcggtgatccaggccgccggcgacgtcacggtcaatgccagcacgcgcatcgacaacggcgtcacccgccccggctacaccttcgtcggcagcggccgccaggtgggcgacagcgcggtgggcggcagcggggtttcggtggtcgtgccgctgacctcgcaactgccgcccgacctggcgcggcgccaggtcaacccggttaccctgcccggcttcagcctgccccagggtgacaacggcctgttccgtctcagctcgcgctttgccgaggacggcaatggcagcgccgcgctcggtgccggcgccgaccgcacccagggcggtagcggcgtctcggtcggccagcaaggcgccggcaacgccgccggtacctggcagggccagggcgtgcgagtcgacggcctggctggcgcggccaacgtccagggtcagggcggcagcacgctcggcggtagcctgccgggcgtcgcccgggtccagggcgtgcccggcaacgccacgccgagcgccagccacaagtacctgatcgagaccaacccggcgctcaccgaactgaagcagttcctcaactcggactacctgctcagcggcctgggcatgaacccggacgatagcaagaagcgtctcggcgacggtctctacgagcagcggctgatccgcgacgcggtggtggcgcgcaccggccagcgctacatcgacgggctgagcagcgacgaggcgctgttccgctacctgatggacaacgccatcgcttacaaggaccaactgcacctgcaactgggtgtgggcctgagcgcggagcagatggcggcgctgacccacgacatcgtctggctggaagaggtcgaggtgaacggcgagaaggtcctcgcgccggtggtctacctggcccaggcggagggtcggctggcacccaacggtgcgctgatccagggccgcgacgtgaagctggtgagcggcggcgacctgcataacgtcggcaccctgcgcgcgcggaacgacctctcggcgacggccgacaacctcgacaacagcggcctgatcgaggccggcaagcgcctcgacctgctcgccggcgactcgatccgcaaccgccagggcggggtcatcgccgggcgtgacgtgagcctcaccgcgctgaccggcgacgtaatcaacgaacgcagcgtgacccgctacgacagcgcgctcgacggccgcacctgggaacgcagcttcgccgacagcgccgcgcgggtggaggcggcgaacagcctgaacgtccaggccggacgcgacatcgccaacctcggcggggtgctgcagagccgcggcgacctcagcctcgacgccggacgcgacgtcaccgtcgccgccgtcgaggaccgccagggccagacccgctggagcacgtcgcggctccagagcgtgacccagctcggcgccgaagtcagcgccgggcgggacctgaacgtcagcgccggccgcgacttgacggcggtggccagcaccctcgaagcgcgccgcgacatcgccctctccgccgggcgcgacgtgaccctggcggcggcggcgaacgaggagcatgcctacagcaagaccaggaaggtcacctaccaggaagacaaggtcgcccagcaaggcacccgcgtggacgccggcggcgacctggcgatcaatgccggacaggacctgcgcctgatcgcgagccaggccagcgccggcgacgaggcctacctggtggccggcgacaagctggaactgctggccgccaacgacagcaactactacctgtacgacaagaagaagaaaggcgacttcggccgcaaggaaacccggcgcgacgaagtcaccgacgtcaaggcggtgggcagccagatcagcagcggcggcgacctcaccctgctcagcggcggcgaccagacctaccagggcgcgaagctggaatcgggcaacgacctggccatcgtcagcggcggcgcggtgaccttcgaggcggtgaaggacctgcaccaggaaagccacgagaagagcaagggcgacctggcgtggaacagcgccaaggggaaagggcagaccgatgaaacgcttcggcagacccagatcgtggcccaggggaatctggcgatcaaggccgtggaagggctgaagatcgacctcaagcatatcgaccagaagaccgtaagccagaccatcgacgcgatggtgcaggcggatccgcaactggcgtggctgaaggaggccgagcagcgcggggatgtggactggcgcatggtgcaggaggtgcacgatagctggaagtacagcaactcgggcatggggccggcgacgcagatcgctgtcgccatcgcggcggcagccatcggtggcatggcggcagcgggagcgctcagtggtgcaggagtgggtgccagtagcttcgccatgggcgcaggagttggtgcggcaggaagcctgtcgggcacggcagcggtcagcctgatcaacaacaagggcgatctcgggaaggtgctgaaagacagcttcagtagtgacagtctgaagcagattgctattgcgagcctgaccggggggctgacggctgagtacttcgacgggattcttcagaccaagactgatccgcttactggaaaggtcacggtagacctcagcagcctatctggtgttggtcgcttcgctgccaatcaggcgatgcagaacgctacatccactgtactgagccaggccttgggccagggcgggagcctgaacgaggcgctgaagagcgcgctctacaacagtttcgcggcggcaggtttcaacttcgtcggcgatatcggccaggaatacagcctgaagccaggcgatccttcgatggtgaccatgcacgccctgatgggtggcctggcggcgcaggtcagcggtggcgatttcgccacgggcgccgcggcggctggcgccaatgaagcgctggtggccaagctagaccaggccttcaagagcttgagccctgagaaccgtgaagccatggtcactatggggtcgcaattggttggtgttctggctgcggcggtacgcgatcctgatgtgacaggcaaagctctggaaagcgctgcttgggtagcgaagaactcgacgcaatacaacttcctcaaccatcaggatgtggccgatctggataatgccttgcagaaatgcaagtcccagggaaattgccgtcaggtagaggaagagttcaaggcgcgtagcgacgagaaccggcggaggttgaatggctgcgtggctgtgggtaattgcgcggagattcgtgcggagatcgatgcggggtctacggctctcaacgagctggtggcccggcaggaaacagctaatccgggaggaagtgacagcgatatagcctacggtttcctgatgggccgaaatgttgtcgactggacgacggctggtcagttgcacctggagcagaccgccaacctctggtggaacggtaatccacagtggcagaaggaagtcggtgcatacctagaccagacggggttcaatccgttcggaatcggcgttccggcaatgggcggtgccgctggcaaggtaacggccaaggcgctcatgaatgcgctgaaggcgggagagttgcccaaaggagaggtggccccaggaaaggctaatctgcctaccattggggcgttggcggatgctgaggcgggaatgccttatacccatccagttaagctcgccgcaaaagcgactgggacagcagggaagattaagattgaagccggcgcaatacctgacgcaaatgaagtacgtgcaggacaagggttatctggtcttgggtacgatgttacgcaccaaaccactgcgtcagctaaaggtattcaagggcagcgaactgcggacttgcatgttgatggactcggttccattgatgtgtatacgccgaagaatcttgatccgacaaagatagttcgagcgatagagaagaagtcgaatcaagccggcggagtcttggtgcaggcggacttgccaagcactgacatgtcgtccattgctgctcgtatgtgggggaagactaacgcgcagagtataaaaactatatttttccagaaaccagacggatcattggtccgatttgatcgacctgctggaggaggctga

SEQ ID NO: 60 - DNA, 16884 bp, Pseudomonas aeruginosa
atggacatccgcagcccgctgaaccagtgcatcgccctgtccctggccggcatcctgttcctcaacccgatcgtcgccgcggcggcggggctggcgctggacaaggccgccggcggcaacaccggcctgggccaggcgggcaacggcgtgcccatcgtcaatatcgccacgcccaacggcgccgggctgtcgaacaaccatttccgcgactacaacgtcggcgccaacgggctgatcctcaacaacgccaccggcaagacccagggtacccagctcggcgggatcatcctcggcaaccccaacctcaagggccaggcggcgcaggtgatcctcaaccaggtcaccggcggcaaccgcagcaccctggccggctacaccgaggtggccgggcagtcggcgcgggtgatcgtcgccaacccgcacggcatcacctgccagggctgcggcttcatcaacacgccgcgcgcgaccctcaccaccggcaagccgatcatggacggccagcgcctggagcgcttccaggtggacggcggcgacatcgtcgtcgaaggcgccgaactgaacgtcggcaacctcgaacagttcgacctgatcacccgcagcgccaagctcaacgccaagctctacgcgaagaacctcaacatcgtcaccggccgcaacgacgtccaggccgacagcctgcaggccacgccgcgcgccgccgatggcagcgagaagccacaactggcgatcgacagctcggcgctgggcgggatgtacgccggggcgatccgcctggtcggcaccgagcagggcgtgggggtgaagctggccggcgacatggccgccagcggcggcgacatccgcatcgacgccagcggcaagctgagcctggcccaggcctccagccagggcgacctgaagatcgcggcccaggccgtggagctgaacggcaagacctacgccggcggcagcgccgagattcgcagcgcggaggaactggtcaaccggcagagcctggcggcgcgcgaacgcatcgcgctggaggcggcgcatatcgacaacgccggggtgatcgaagccggcgtcgagccagacgagcgacgcaacgcgcgtggcgacctcgagctgcgcagcggcaccctgcgcaacgccggcagcctggtggccagccgcgcgctggaagcgaaggcgagccaggcgctggacaaccagggcggcagcctgaagggggcgaccgtccgggtcgacggcggacacctggacaaccgtggcggcaagctgctcgccgagggcgaactgcgggtcgaggcgagcagcctggacaaccgccaggacggcctgttgcagagccgggaccgcgccgtggtcaagacccgtggcgatctcgacaaccgtggcggccaggtcgtcggtctgaacgaactgcaggtccaggctgccgcactggacaatcgcagtgccggtctcctttccagcaagggagacatggacatcgagttcgctcgtctggacaacagtgcgggcggcaagctggtcagcgagcgccgtacgctcctgaaggcggatcggctcgataatcgcagcggtcgcattgtcgccggccaggatctcgacttgagctctcggttgatcgacaaccgagcgggcgatatctccagcacgtcgagggtggtggcgagcgctcgcgaacagttggacaaccgcggtggcaagatcgtcggtgacagtggcctggacatcacaacgccacgcatgctcaaccaggacaagggggtactcgccagccgcgatgggctgcgcctgagtgctacggagttgttcaacggcgcggggggcctgctgtccagccagaagggtatcgacgtctccctggccggtgcgttcgataaccaggccggcagcctggacagccggggcttcctgacggtgaagtcagcctggctcgacaaccagggcggtacgctatccagcgcaggggcattggcagtgaccagccagggcgccctgaacaatcagggcggcagactggcgagcgacgccggacttagcttgagcagcgccagcctcgacaacagccaggccggtgcgatcagtggcaagggggccgtggagattcgtaccggcaacctgaacaacagccggaaagccagtatcggcagcgatgcgggactcaccctggtcgccgctcgggtagacaacagccaggcgggccggatcgccgccaagggtgtgatcgatgcggatctccaagggctggaccagcatgacaggggcaacctggtcagcgataccggcatcacgctcgatctgaacaagggaagcctggtcaatcgcgctcaaggcctgatcgccacgcctggcaccttgctcctgcgccaactcggcgtggtggacaacagcggtggggaaatctccagcgaccgcgcgttcactcttgccacctccgcgttgaacaaccaggggggacgcctgctcagcggcggagccctgaccttgcgtatcgcgcaggccctggacaacagcctcgaggggattgtctccggtgctggaggtctggatatccaggcattcgtcctggacaaccgtagtggctccatcggcagcaagggcgccatcgatatcggtgtgacccgcctggaaaacgacgctggcacactgatcgctgaacgcggcctgaagctggtagccgatgaggcgaacagttccaaggggcgtatcgccgccaatggtagcctgcatgccaaggttggcacgctgagccagaagggaggagaactgaccagtcaggactcgctgactctcgacctgggcatcctaaacaataacgctggccgtatcgctggcaaccagggcgtggacatcacggcccggcaggtggacaacagcgtcggcgagattgccagccagggcgtggtggcgctgaacctcactgagcagctggacaaccgtggcggcaagatcgtcggtgacagtggtctgggcatcaccgcgccgcacgtgctcaaccaggacaagggggtactcgccagccgcgatgggctgcgcctgagtgctacggagttgttcaacggcgcggggggcctgctgtccagccagaagggtatcgacgtctccctggccggtgcgttcgataaccaggccggcagcctggacagccggggcttcctgacggtgaagtcagcctggctcgacaaccagggcggtacgctatccagcgcaggggcattggcagtgaccagccagggcgccctgaacaatcagggcggcagactggcgagcgacgccggacttagcttgagcagcgccagcctcgacaacagccaggccggtgcgatcagtggcaagggggccgtggagattcgtaccggcaacctgaacaacagccggaaagccagtatcggcagcgatgcgggactcaccctggtcgccgctcgggtagacaacagccaggcgggccggatcgctgccaagggtgcgatcgatgcggctctccaagggttggaccagcatgacaggggcagcctggtcagcgataccggcatcacgctcgatctgaacaagggaagcctggtcaatcgcgctcaaggcctgatcgccacgcctggcaccttgcttctgcgccaactcggcgtggtggacaacagcggtggggaaatctccagcgaccgcgcgttcactcttgccacctccgcgttgaacaaccagggtggacgcctgctcagcggtggagccctgaccttgcgtatcgcgcaggccctggacaacagcctcgaggggattgtctccggcgccggaggtctggatatccaggcattcgtcctggacaaccgtagtggctccatcggcagcaagggcgccatcgatatcggtgtgacccgcctggaaaacgacgctggcacgctgatcgccgaacgcggcctgaagctggcggccgatgaggcgaacaactccaaggggcgtatcgtcgccaaggatgaactgcgtgccaaactcggtgcgctggtgcagaacgggggagagctgacgactcagggcgcgctggccctcgacgccgacaaagtcgacaacggcgctggtcgcatcgccggcaaccgaggtgtggtcatcgatgcccggcaggtggacaaccgtgccggcgagattgccagccagggcgtggcgacgctgaatctcactgagcaactggacaaccgtggcggcaaagtcgttgctgacagtggtctgggcatcaccgcgccacgcgtgctcaaccaggacaagggagtaatcgccagccgcgatgggctgcgcctgagtggtaccgaattgttcaatggcaatgccggactgctcagcagtcagagacatatagaggtcactctggacggcgtgctggacaatcagggcaagggcgcgctgctcagcgacggtaccctgacggtgagcgccgggcgcatacacaaccaggacgccactctgtccagcgccggtgcgctgagactgagcagccaggaggcggtggacaaccgtggcggcaagttggtgacggactccagcctgcgcctgaccagcgccagcctggacaacagccgatcagggatcatcagtgccaacgctgcggcggagatccataccggggttctgaacaacagccagaaaggcaatcttggcagtaatgacgggctcggcctgattgctactgaggtggataacagccaggaaggtcggatcactgccaaaggcatgatcgacgcaaatatcaagggactcgatcagcagggcaaagggcggctggtcagtaatgccggcatcatactcgacctgaacgagggaaccctggccaatggcgctcagggcctgatcgccacgcctggaaccttgctcctgcgccaactcggcatggtggacaacagcggcggggaaatttccagcgaccgagccttcacactcaccacctccgcgctgaccaaccagggtggccgcctgcgcagcggcggtgtactgacgttgcgcatcgcccaggctctggacaacagcctcgaaggtgttctctccggcaccggaggcctggatatccgggcgcttgccctggacaaccgcagtggctccatcggcagcaagggcgccgtcgatatcgacgtgtcccgtttggaaaacgatgacggcgacctgcttagcgaaggtcgtctgaaactgactgccgagcgagcgaacagtgtcaggggacggatcgcggccaggggtgacctgcacgccagcgtgacagcctttaaccaggcgggtggcgaattgagcagcgagggtgcgctgatgctcgaggccgatagcctcgacaaccgcagcggcggtctggtcagtgctgatggcaacctgaccgtttccgcccggaggatcgacaaccgtgcgggcgaaatcgccagcccgggccaggtgacactggacgtcgccgagcagttggacaaccgaggcggcaaggccatcggcgatagcggacttcgcctcgccgcgccacgggtactcaaccaggacggcggggtactcgccagtcgtgatgggctgcgcctgaatggcgccgaactgttcaatggcaacggcggcctgctcagcagccagcaaagcatcgacgtcattctggacggcgtattgggcaatcaggcaggcagcttgagcagccagggacgcctgagcgtgaagagcggtcggctggacaaccagggcggtgcagtctccagcgccgggaccttgtcgctttccagccagggtgcgttgaacaaccaggggggcagggtggtcaccgacgccggtgccgtcctgcgcagcgccagcctcgacaatagccagggcggcatcgtcagcgccaagggggccgcggagatccgtactggcagcctcaacaatagccagaagggcggcataggcagcggtgccgggctcgcgctggtcgcggacctggtggacaacagccagaacggccggatcactgccaagggtgcgatcgatgccaacctgaaggggctggatcagcagggcagcggcaggctggtcagcgatacggccatcgcgctcgatctgcgcgggggagaactggtcaaccgtgctcagggcctgatcgccacgcctggagccttgctgctgcggcaactgggtgtcgtggacaacagtggcggtggcgagatctccagcgatcgaagctttaccctcgccgcgaccgcgctgagcaaccggggtggccgcgtgatcagcggcgactccctgaccctgcgcatcgcccaggcactggacaacagcctccaaggcgttctttccgcaagcggagggctggatgtcgctgcactcgtcttcgacaaccatagcggcatcgttgctagcaagggcgatacacacatcggggtgaaccgcctggagaacgaggcaggccgcgtggtcagcgaaggcgccctggatctgaccgccaagcaggtgagcagcgccaaggggcgcattgccgcgaagggcgatctgcaggtcacggttggcaccctggagcagcagggtggagaactggccagtcaggggacgctgactctcgacgccgatagcctggataaccgcaatggcggcctggtgagcgccgatggcggggtcaccgccgaggcacgccagatcgataaccgcggtggggaaatatccagcgtggccaaggtggctctggctgtccgggaacaactggacaaccgggggggcaaggtgatcggcgacagtgagctgagcctaaccgtgcagcgcctgctgaaccaggccaagggtgtgctcgccagtcgcgatggattgcacctggacggcgcggaactgctcaatggcgatggcggcctgctcagcagccaacgcctggtggatgtaacgctcagtggtgcattggacaaccaggggagcggtgcactggtcagcgaagagtcgctgacagtgaaggccgaccaggtcaataaccaggcggggactttctccagtgcgggtagcctgctcgttaccagccggggcgagttgaacaaccagggtggcaggttggtgaccgatgctggagccaccctgaacagcactggcttcgacaacagccgtgcgggcctggtcagtgcgaaaggggctgtggccattcgtaccggagccctgaacaacagtcagaagggatccattggcggcaatacgggcgtcaccctggtcgccgggttggtcgacaacggccgggaaggacggatcagcaccaagggtacgctcgacgccaacctgaaagggttgcttcagcaggggggaggctcgctggtcggcgagcgcggtgtcaccctcgacctcaacggtggcaccctggacaaccacgacctcggtctggtttcaacgcctggcgcgctcctgctgcgccaactcggcatggtggacaacagcgtcggcggagagatatccagcgaccgtgcttttaccctcgccgccaacacactgaacaatcagggcgggcggctgatcagcagcgaagctttgaccctgcgcatcgccaagacactggacaacagtctcaaggggcaggtcctggcgaccgacggactggccatcgagtctcaggtcttggacaaccgtgcgggaaccatcggcagcaagggtgatgcccgtatcagcgtgaccagcctggacaacgccgaacaaggcagcctggtgagtgaaggccgcctggagcttgtagccgaccaggtgagcaacggcaaccaaggccgtatcgccgccagaggcgtgctggaggcggcggtcggtacgctgctccagcaaggcggcgaactggtcagccaggggagcctggaccttcgcgccgacacgctcgacaacagccagtccgggctgatcgccgcgaatggcggcatcgctatcgaggcgcggcaggtcgacaaccgcgccggcgagatttccagcacctcgaaggtcgccgtgaacgcccgcgagcaactggacaaccgcggcggcaaggtcatcggcgacagcggcctgcgcctcaccgtgcagcgcctgctgaaccaggccaagggggtgctggccgggcgcgacggcctgagcctggacggcggcgaactgttcaacggcgacggcggtcggctcgacagccagaacagcctgagcgtgagcctcggcggcgtgctggacaaccagggcggcgcgctggtcagcgaaggcagcctgacggcgcgcgccgcgcgcctggacaaccgtggcgggaccttctccagcgccggtgcgctggcgctgaccagccaggccgtgctggacaaccagggcggcaggctgctcagcgatgccggtgtgacgctgaagggcgccagcctcgacaacagccgttccggcgtgatcagcgccaagggagcggtggatatccgcaccggcgtactggacaacagccgcaacggcggcatcggcagcaacgccggcatcaccctggtggccgcccggctggacaacggccagcagggccgggtcagcgccaagggcctgctcgacgccaacctgaaaggcctcgaccagcgcggaggcggcgttctggtcagcgaaaccggcgtcaccctcgacctcaatggcggcacgctggtcaaccgcgacggcggcttgatcgccacgcccggcgcgctgctgctgcgccagctcggcgcggtggacaacggcgccggcggggaaatctccagcgaccgcgccttcaccctcgccgccgccagcctggacaaccgcggcgggcgcctgatcggcgccgacagcctgaccctgcgcatcgcccaggccctggacaacagcctggccggggtgatctccggcgccgccggcctggacatcgcggccgctcgcctggacaacagcgccaagggcaccctggccagtcgcgccggcatcgacctgcgcgtcgacggcgcgctggacaaccacgccgaaggcaccgtctccggcgcccgcctgacgctcgccagcgcctcgctggacaacagcggcaagggcctgctctccggcaacgccggcctgagcgtcgccactggcgcgctggacaacgccgagggtggccagttgatcagccagggcgtcctggacgtcagcagcgccgacctcgacaaccgtggcggcgccctcagtggcaagcagtcgctgcgcctgagcgccgccaacctggacaaccgtggcggcctgctcaccagcgacggcgaactggaactgacggcagggcgcgtcgattccgccgacggcggcgaaatctccgcccggggcgacctgcgcctgacggtcgagcgcctggtgcaacgccagggccggctgattggcgagcgcggcgtcagtctcgacctgcggggcggcgacctggacaaccagggcggcctgatcagtgcccgcggcccgctgagcatcgagcggctgaacgtcctcgacaaccgccagggcggcgagatttacagccagcagggcttcgagctgctggccaggcgcatcgacaacggccagcaggggcgcatcatcagcgccgggaaactgcgcctggacgccgacgcgctgggcaacgccggcgccggcctgctctccggatggcagggcctgacggtgacaggcgggagcctggacaacagcgccggcggcaccctttcgagcaaggacggcgagctggccatcagcctcggcggcgcgctggacaaccacggccagggcgcgctggtcagcaagggcgcgcaacggatcgacgccgccagcctggataacgcccagggcatcgtctccggcgaaagcgacgtgaccctgagcatcgccgggaagctggacaacggccagggcggcctggtctcggcgcagcgcgcgctgagcttcgagcgcgacgatacgctgctgaacaacgccggcggccggatcaacggcggcagcctgctgctcaagggcgccagcctggataacagcgacggccagttgatcagccagggccggctcgacgccatcctcggcggcgccctggtcaacgccggcgcggcgcgcctggccagcggcggcgacctgctgctgcgcagcgccagcgtcgacaaccgcggcggcaagctggtcagccaggggctgctggagatcagcgccggcagcctcgacaacagcgcctccggcaccctcgccagccaggccgacatgagcctgcgcctgggcggcggcgccctgcgcaaccagcaggacggcctgatcttcagccaggccggcgccctcgaggtgcaggccggcagcctggacaaccgccagggcacgctccaggcccagggcgacaaccggctgcgtatcggtggcgcgctggacaaccaggccggccgcctggacagccgggccggcaacctcgacctgcagagcggcagcctcgacaacggcgccggcggcgtgctcaacagcgccaagggttggctgaagctggtcaccgggctgttcgacaacagcgccggcgtcacccaggcgcagtcgctggagattcgcgccgggcaaggcgtgcgcaaccagcagggccatctctcggcgctgggcggcgacaaccgcatcgtcaccgccgacttcgacaaccagggcggcggcctctacgccagcggcctgctcagcctcgacggccagcgcttcctcaaccagggcgcggcggcgggccagggcggcaaggtcggcgccgggcgcatcgacttcagcctggccggcgcgctggccaaccgcttcggccagttggaaagcgagagcgagctgcacctgcgcgccgccgcgatcgacaacagcggcggcagcctgcgcgccctcggccgcagcggcagcacgcggctggtcgctggcgacctgaacaacgcctacggcgtgctggaaagcgccaaccaggacctcgacctgcaactgggcagcctggccaacgccggcgggcgcatcctccacactggcaacggcaccttcggcctggattccgggcaggtgatccgcgccggcggcgaactgaccaccaatggcctgctggacatccgtgccagcgaatggaccaacagcagcgtgctgcaagccggacgcctgaacctggacatcggcaccttccgccagacggccgagggcaagctgctggcggtgcagtccttcactggccgcggcggcgactggagcaacgacggcctgctggccagcaacggcagcttgcgactcgagctgagcggcggctaccgtggcaacggccgcgccaccagcctcggcgacttcgccctgaacgccgccagcctcgacctcggcaatgccgccagcctcgccggcggcgccaatgtcacgcttggcgccggcaacctgctggtcaaccgtgggcggatcaccgctgccggcgacctcgtggccagcgccgcgagcctgaacaactacggcaccctgggcggcggcggcaacctgcgattgaacgcgcccgccctgctcaacgagcgcgggttgctgttcagtggcgccgacatgaccctgcgcgccggcgacatcaccaacctctacggggatgtgtacagcctcggcaggctggatatcgcccgcgacgatgcggggggctgggcaaatcgcttggagaacatttccgggaatttagagagcacaggtgatatgcgtttctccgtgagttcacttctcaatagaagggaaactctagagattgaaggtgacttgcagaatagcgctattggcgtccgctgtacggggtgtcagctttctgagaggtggggaaaaactaggtcttcgagcgagcttgtctggatcagggaatataagtctacattgggagattcttctgccgctgcttcaattacggctggtcgagatctgcttgttgtaggtgcaagcctgcagaatattgcttctaatataagtgctgtaagagacgccacgctatctctgagtaatttcgaaaacaaaggttatgcgttaggggaatatgcggtcaggggcgtttattcgccgccgagtaaatttggcgaagaattgcttatgcgcatattggcgtataacgctgtcaacgatcccagttatggggagggatatgcgagcacaggggggagacttccgaatattcattatttcgacaagaattttaatgaaaaagtctctccgctggaggtcattcatggaaacgggaaaaatggtgggccgggttggcacctgtacttcggtaccttagatgttgagtatccggacacagatcgctggaataaggctattggacgaataccggcgccgaattattcatcgaaaaaaacggatgctattccagatctacttaagggattggctcctctcgatgagttgacgattaacaaaggggcgaactcaacggttggtgctgtcgtgcaagctggcggtcgtgtaacggtgaatgctgcggagagtttcaataattctgtcctacagggatttcaggccgttcaggaaacccagttacctcatcaggacatagctgtttcaagcacgacgagcgccgtagtgactctgaagagtcaactgccagcggatttggcaaggcaacagatcaatcctctcaccctgccgggcttcagcctgcctcaaggccagaatgggctcttccgcctggcgtcccaaggagcccaggtgaaccaggcaagtggtgctctgaaatccgccagcgatctcacccagagcggccatggcgtatctgtatccgcacagacaggcagtggcgcaagtggctggagtacccaggcgcgtcgtgtcggcgatgatcgggtcacctcgcttgccggttccgcctatcaaggccgggtagctgaggctatcgatgcgctacgggcttccgcgccaatctcgggcgacgggggaaacactggccgtttccaggccggtgagcaccaggcgaccacgggactgggtggactcgtcgagggcaatgcatcgggtcacagcggcaatggcgtcatcctcgccgatctgcgcggtggtctaccctcgttctcaagccttcccgcgtctgatcatgttcaaggcacagtgcccggtcacgatgggaatggaactattctcgccaattggcagggtgcgcaggcgacggtccaggcctcgccttcgacagtgcgtgtagagggggtagtctccagtccaggtggcaatggcagcatccttgccgatctgccggctgaacagtcgtcggtgcaggcactgccttcggccgttagggctcagggcagcctgcctcgcctcgaagagcggagcgcccttcttgccgagcctccggttgggcagccggcgttgcaaaccctgccgtcggttgcgcgcgttgagggcgtgcccagcaatgccacaccgagcaacagccacaagtatctgatcgagaccaacccggcgctcaccgagctgaagcagttcctcaactcggactacctgctcggtggtctgggtatcaatccggacgatagcaagaagcgcctgggtgacggtctatacgagcagcgcctggtacgcgaagcgatcgtccagcgtacggggcagcgcttcatcgccggattgaacagcgacgaagcgatgttccgctatctgatggacaacgccatcgccagcaaggacgtattgggactgacccctggcgtcaccctcagcgccgcccaggtggcggcgctgacccacgatatcgtttggctggaagaagtcgaggtgaatggcgaaaaggtcctcgcccccgtggtctacctggcccaggccgaggggcggttgggcccgaacggcgcgctgatccaggggcgcgacgtgaacctgatcaccggcggggacctgaggaacgccggtaccctgcgcgcgcagaacgacctcagcgcgacagccggcaacatcgacaacagcggcctgatcgaggccggcaaccgcctcgacctgctggccagcggctccatccgcaatgaccagggcggcatcattgccgggcgcgaggtaagcctctctgcccttaccggagacgtcatcaatgaacggacggtgacccagcaccagtcctcctacaggggaaccggtaccactgaggcatttgccgatagcgccgcgcgtatcgaggctgcgcagaagctgaccgtttcggcaggacgcgatgtagccaatattggcggtgtcatcgacagcaagggcgacctcgccttgcaaggcggcagggatgtcctggtttcggctgcggtagcggagcggggctggacggcaggaagccaggcataccagacccagacgacccagatgggcgccgaggtcgtggcggggcgcgatatcagcgtcagcgccggacgcgatatcagcgtcgtgggcagccgcatcgacgctcgtcgcgacgtgacattcgaggcgggtcgcgatgtgggcctggtcgcggctgccaacgaagagcatgcctatggcaagaccaagaaggtcactttccaggacgacaagatcacccagcaggccactcgcgtggacgctggcggcgacctggcgatcaatgccggacaggacctgcggctggtcgcgagccaggccagcgccggcgacgaagcctacctggtggccggcgacaagctggagctgctggccgcgaacgacagcagttactacctctacgacaagaagagcaaaggcagcttcggtagcaagaagacccggcgcgacgaaatcaccgatgtgacggcagtgggcagccaaatatccagcggcggcgacctcaccctgctcagtggcggcgaccagacttaccagggcgcgaagctggaatcgggcaacgacctggccatcgtcagcggcggcgcggtgaccttcgaggcggtaaaggacctgcaccaggaaagccacgagaagagcaagggcgacctggcgtggcagtcgtcgaagggcaagggccagaccgacgaaaccgtgcgccagagccagatcgtggcccaggggaatctggcgatcaaggccgtggaagggctgaagatcgacctcaagcacatcgaccagaagaccgtgagccagaccatcgacgcgatggtgcaggcggatccgcaactggcctggctgaagcagatggagcagcgcggcgatgtggattggcggcgcgtgcaggaactgcatgacagctggaagtacagcaactccgggctgggcgtcggcgcgcagttggcgatagcgatcgttgtggcctacttcacggcgggtgcggcgagtgcggcattgggatcgatggcgggagtgggggcgggctcaggaagcatgatggctgctgccggtagcactgcaatggtccaggccggtacagcagtaggaacagctgccgccggctgggcgaatgcagctggaactgccgtggctatgggcatggccagcaatggagcgatcagcaccatcaacaaccggggaaacctgggggatgtcgtcaaggacgtgacctccagcgatgcgctgaggggctatgtagtcgctggcacgactgcggggctgactgccggcgtctacgacaaatggacctcgacccagaccggcacctcgaccgctctaccgaacaccggggccgtggcgcccgccgcagggttgggcacctggcaaggcgtgggccagttcacctcgaaccagttgctgcagaatggtacttcggtgctgttggaccgggcgctgggcggcaagggcagcctgggcgatgcgttgcaaaacagcctggcaaatgcctttgcggcctacggcttcaagctgattggcgacaccacccatggcgtgctggacgacggcagcctcggcaagatcggcttgcacgccctgatgggaggtctggccgccgaagcggtcggtggcgatttccgtaccggagccctggctgcgggagtcaacgaggcgctggtggatagcctcgccaagcaatacgccagcctgcccatcgatgacaagaagggcctgctgatcatgagttcgcagttgatcggcgtgctggcggcttcgacgcagggcgatgcggacgccaagagcttgcagacgggggcctgggtggcggggaatgccacccaacacaactacctcagtcattggcaggaggagaagaagcggcaggaggtcgatggctgcaaagacaaacagctctgcaaaaccggaatagaagccaaatgggcaattatttcggcccagcaggatgtcggtatcgtcgtaggtgttggaggaggcatcggtctttcgacagctgaaaccgcagtgggtgtttatgagctggtcaagaactggagggaaacctatgcagctctggagcagttggccacttcgccagagttccggcagcaatttggcgataactacctgaaggggctggaggagcgcgccgcattcttgacccaggcatacgaggatgccggctggcaaggttcggtcacagctggtgtcgagggcggtaggttcgctgcggaacttgttggcgttctgacggcagtgaaaggtggcgcgcagataaccgccaagctgccaacagcagccaagaacctggtcaacgcgattgcggagtcacctgtttccggtagtatgagttcgcagcttggggcagtgggggatttgggtcggctgggtgggggaggtaaaggttatgtcgatattctttcccacgaagctaaacagcatattttgtatggcgacaaacctgggagtggtggccatttgtggccggggcaggcagggaagacagttttccctcaaaactggtcggcagataagatagttcacgaggttggtgatattgcgacgtcccctagtaccaaatggtatgcccaaacaggaactggtggggtttatacaagcaagggtgatcccgctaaatgggttgcttatgaggttcgtgatggagttcgtatgcgcgttgtttatcagcccgctacaggaaaggtgatcacagccttccccgacaacgcacctatcccaccttataagcccattaaatag

SEQ ID NO: 61 - RNA, 201 nt, Pseudomonas aeruginosa
augagucaggaaccccacguacacggcccgaacugcaaccacgaccacgaucaucaucacgaucauggccauggucauguccaugguccgcacugcaaccacagccacgagccggugcgcaauccgcucaaggccguaggccgcaacgaucccugccccugcggcagcgagaagaaauucaagaagugccacggcgccuga

SEQ ID NO: 62 - RNA, 237 nt, Pseudomonas aeruginosa
augaaaaagaccguaacucuugcccugcugcucgcugccagccuuggccuggccgcuugcgacaagaaagaggaagacaaggcagcggccccggcagcuccggcuaccgagacccagccgagcgcuccggcuacucccccugccgagcccagcgccccggcgccgucgagcgacacuccggcaaccccgcagacuccggcaccgacuccggagcaaccgcaacagaaccagcaauaa

SEQ ID NO: 63 - RNA, 315 nt, Pseudomonas aeruginosa
augaaaaagauuucccucgcuucuuccgucgucggcgcugcucugcucggcguagccagugucggcgcgcaugccgcgcagaaucccuucgccgugcaggagcugagcagcggcuacagcguggcugccgccgagaaagccaaggaagguuccugcggcgaggccaagugcggugccgacaagggcaagcgcgaagccuccaaggccggucaugaaggcagcugcggugcggaucgcaaggccaaggaagguuccugcgguggcgagaagaaggccggcgaaggcaacugcggcgccgacaagaagaagucguaa

SEQ ID NO: 64 - RNA, 468 nt, Pseudomonas aeruginosa
auguccguuuucgauucgcgucaaaagacuuccgccagccugcucggugccguacugguggggggaaugcugcucggcgguucggcguucgccgucgagccgcugggccaggggcugcaaguggcggcggcgagcgccggcgaaggcaagugcggagaaggcaagugugguagcggcggcuccgcgaagaccccggccaaggccggcgccgagggcaagugcggggagggcaagugcggcgacgccuccuuugcccgaaccgacaccgaucacgauggcaaggucucgcgcgccgaguuccucgcgguggccaaggaccgugccggugaguucgacagcaucgauagcgaccaugacggcuucauuuccgaagccgaggccuacgaacaccugcgcaagaccuacgaggccaacggcaagccgaugcccgccgggcuguucagcaagcuggagcaaggccagcacuga

SEQ ID NO: 65 - RNA, 540 nt, Pseudomonas aeruginosa
augcguucccugucccuccuucuccuccucucgcuggcguccaccugcgaggccgcugcgguauuccgcugcgaagacgccagcggccaugucagcuucacccaacucgguugccccgccgggcaggccggcgagaccgucguggcggacaacccgccgccgggaggcaggagcgucacgccgauggccgagacgaagacgaaaaaggcguccaucggccggaaaagcgugccgcucgcggugaucggagaaagagaagaucgcugcggcagacgccuggacgagaaggaacgccgcaaggcgaucguggagcagcggauaauggcgggaaugacccgcuccgauguggagcgggcgcugggcaagccggaccgggucagcgggaacaaugcggaggugcguuaucaguacaaggccgacaagcgacggggagcgagaagcgugagcuucgaucaggagggaugugugaagggaagagaagguaccggguggagcgagucgaucccgggagcuaaggccgggccguccucauaccgauga

SEQ ID NO: 66 - RNA, 915 nt, Pseudomonas aeruginosa
augagccaacccagcgaaaaccguuugaucaccucggcgcgcuacgcgcucugccuguugaccgccagcggcgugcugcucagcggcugcgccagcagcggcgucggcucggucgcccagaccacccgcgcggaauacuacccguccugcuacgagccggugucgcaccugcgcagcaccgauaacgcagugcgcaauucggccaucaccggcgccauuaccggcggccuccugggcggccuggccggcggccuggccagcgacgagaaccgcggccgcaaugccgcccucgcugccgcaggcggcgcccuggccggcggcgcggcgggcuacuacauggagaagcagaagcagaucagcgaugaccgcgcgcgcaucggcuccuacgguaccgacgucgaccgcagcaccgucgagaucaaccguagcguggccuacgccaagucggcgcaaagcugcuaccagagccaguucaaggcucugcucgacggucgcaagaacaagucgaucaacgaagccgaagggcgcaagcgccuggccgagaucgucagcggccugcaggagaccaacgccuugcuggucgccgccaacggccgugccggcgagaacaucagcaacuacacccaggccuacgagaaagaccugcagcaggucggcguaccgcgcgccgaggugaccaaggucgccgaggccgagaaccgcgccagcacuacgaaaggcggcagcaagcccaagaccggcagcaaucccaaggugccgaaggaagcggucgccaccgagcagaccauccgcaaggcccaggacgcgcaaagcgaaggcaacaagguggccucccagggccagggcaugauccgggaagucugcaacagcccggacaugggcgacugggcgccgccgagcugcgccaaggccuga

SEQ ID NO: 67 - RNA, 930 nt, Pseudomonas aeruginosa
auggcuggcaagaagaagagcgaaaaagaguccaguuggaucggcgagaucgagaaauacucgcggcagaucuggcuggcuggucugggggccuacucgaaggucagcaaggacggcagcaagcuguucgagaccuuggugaaagacggcgagaaggcugaaaaagaagcgaaguccgauguggacgcgcaggucggugcggcgaaggcuuccgcccgcucugcgaagagcaaggucgacgagguucgggaccgugcgcucggcaaguggagcgagcucgaggaagcuuucgacaagcgccugaacagcgccaucucgcgucucggcgugccgagccgcaacgaggugaaggagcugcacagcaaggucgauacgcugaccaagcagaucgagaaacucaccggcgucagcgucaagccggcggcgaaggcagcggccaagccugcggcgaaaccggcugccaagcccgcggcgaaaaccgcagcggccaagccggcagcuaaaccggcagccaaggccgccgccaagccugcggcgaaacccgcggcgaaaaaaaccgcggcgaaaaccgcggccgccaagccggcagccaagcccgccgccaaaccgacugcgaaggccgcagcgaaaccggcgaccaagccggcagccaaggccgcggcgaagccugcugcgaaaccugccgcagccaagccugccgcgaagccggcagccaagccggccgcugcgaccgccgccaagcccgcggcgaaaccugccgccaagccggcugcgaaaaagccugcggcgaagaagccggcagccaagcccgccgcggcgaaaccggccgcucccgccgcgucuucgagcgcgcccgcugcccccgccgccacaccggcugccagcgcuccggcagcgaacgcuccggcgacgccgagcagccagggcuga

SEQ ID NO: 68 - RNA, 1023 nt, Pseudomonas aeruginosa
augaaagcgacuaugguccugaccccgcuggcccuggcaauggcugcagugcugucgguaucggccuacgccggaaacgaagguggcuggcacccgccgaaacccaacccgcagucgaacaacaagggcggagccacggcccuggugguggauacgcagcagaacuacaacaacaaggucagcaacuucggcacgcugaacaaugccucggugagcggcucgaucaaggaugccucgggcaacgucggggucaacgucgccgccggcgacaacaaccagcaggccaacgccgccgcgcuggccagcgccgacgccagcuucguguucggcaccgcgaccgccagcaccagcgugcugcagagcggcuacggcaauacgcugaacaacuacuccaaccccaacaccgcaucgcugagcaacucggccaacaacgucucgggcaaccugggcgugaacgucgccgccggcaacuucaaccagcagaagaacgaccuggccgccgccgucuccaacggccaguacagcacugccgguagcgccgcgucgcagaccuccaccggcaacaccaccgucaacagcgccaacuacgccuauggcggcaccuacgugucgcugaagcugaacgccgacggcagcuacaagggcaccuccgaccagaucggcgacgucuaccucgacaccugggaaggccagacccauccgggcggcagcaauaccggccacaucgacguggacagccaggcccagggcgccaaggaccugaaccacgacggcggcgcguucgccuucaaggaaaagggcgacgucgaccugaaaggcacgguguccggcuucaucccggcgaucgucggcuucaagaccccggucaccaacaacgccagccugagcaacucguugcagaacgucucgggcaacgucggggugaacaucgccgccgguggcggcaaccagcagagcaacucccuguccaucgccgccgguugcagcagcugcccggccgguggcgagagccuuggcuucuga

SEQ ID NO: 69 - RNA, 1044 nt, Pseudomonas aeruginosa
augaagcaacaguucgaacgcucgccuuccgagaguuauuucuggcccgucguccuggcggugguccugcacguucugaucuucgccaugcuguucgucagcugggcguuugcuccggagcuuccucccuccaagccgaucgugcaggccacgcucuaccagcucaagucgaagagccaggcgacgacacagaccaaccagaagaucgcuggcgaggcgaagaagaccgccuccaagcaauacgaagucgagcagcucgaacagaagaagcucgagcagcagaaacucgagcaacaaaagcuggaacagcagcaggucgcugcugcgaaagcggcggaacaaaagaaggcugacgaggcucgaaaggccgaggcccagaaagccgccgaggcgaaaaaggccgaugaagccaagaaagcugccgaggccaaggccgccgaacagaagaagcaggcugacauagccaagaagcgcgccgaggacgaggccaagaaaaaggccgcugaggacgccaagaaaaaggcagccgaggacgcgaagaagaaagcggccgaggaggccaagaagaaggcugcugcggaagcggcgaagaagaaagccgccgucgaggccgccaagaaaaaggccgccgccgcugccgcggcagcccgcaaggcugccgaggacaagaaggcgcgggcauuggccgaguugcuuucggauacgaccgagcgccagcaggcccuggccgacgaggugggcagcgaggucaccggcagucucgacgaccugaucgucaaccuggugagccagcaguggcggcguccuccaucggcgcguaauggaaugagcguagaaguacugaucgaaaugcugccggacgguaccaucaccaaugccagcgucagccguucgaguggcgacaagccuuucgacaguucggcgguggcggcggugcgcaacgucggccguauucccgagaugcagcaauugccgcgggcuaccuucgacagccuguaucgucagcgccgcaucaucuuuaaaccggaggauuugagucuguga

SEQ ID NO: 70 - RNA, 1059 nt, Pseudomonas aeruginosa
augucggccaacaagaagcccgucaccacccccuugcaccuguugcagcaacuuucccacagccuugucgagcaccuggaaggugcgugcaaacaagcgcuggucgauucggaaaagcuccuggccaaacuugaaaagcaacguggcaaagcccaggaaaagcugcacaaggcucgcaccaagcugcaggaugcugccaaggccggcaagaccaaggcacaggccaaggcgcgcgagaccaucagcgaccuggaagaggcguuggauacccugaaggcccggcaggcggacacccguaccuacaucgucggccucaagcgugacguacaggaaagccucaagcuggcgcagggugucggcaaggugaaggaagcugcuggcaaggcucuggagagccgcaaggcgaaacccgcgaccaaaccugcugcgaaggcggcagccaagccugcggugaaaaccguagcggcgaagccugcggccaagccggcugcgaagccugcugcgaaaccggcggccaagccugcggcgaaaaccgcggcagcgaagcccgcagccaagccgacggcgaagccugcugcgaaaccggcggccaagcccgcggcgaaaaccgcagccgcgaagcccgcagccaagccggcggcgaagccuguggcgaaaccggcggccaagccugcggcgaaaaccgcagccgcgaagcccgccgccaagccggcagcgaagccugucgcgaaaccgacggccaagcccgcggcgaaaaccgcagccgcgaagcccgcagccaagccagcugcgaagccugcggcgaaaccggcggccaagccuguggcgaaauccgcggccgcgaagccugcagccaagccggcugcgaagccugcggcgaaaccggcggccaagccugcggcgaaacccguagccgcgaaaccugccgcaaccaagcccgccaccgcuccugcugcgaagccugcggcgacucccagcgccccggcagccgccuccagcgcugcuucggcaacgccugccgcgggcagcaacggcgccgccccgaccagcgccuccuaa

SEQ ID NO: 71 - RNA, 1263 nt, Pseudomonas aeruginosa
auguggggucuuacgaugaaguuugcgagccugauucugaugcuucucuuugccacgguggcgagggcugaggauuacuacuggaaaauucagucacugccugaacgcuuuucuucgcccucggcagcuugcgcggcgugggccaaagccacgggacgcccuggggaguucaccuucaccgggucuaugaaagcccgugaccagaccucguuuuggugcgaguucacgaacaacgaaaccggcaagacugcugccggguaugguccugccggacgcuauggcgauagcugucccgaggggacggaauacgauaaggcgaccgggguuuguaagucgccuccgcaagaaugcaaggaaggcgaacuguucccggccaaaggcccggacucucccgugguuaccucgggaggccguaacuaugucggugacggcggcgccccgaccgccugcuaucaaagcugugaguauggcggcaaucccagcccggccaguugcuaucuggucaaaggcuccaccacgaccggcuucugcaauuacauccucaagggcaccggacagaauugcggugccgauuccuacaccuucucccagaccggcgauucgcugaacccgcccgacacuccgaacaccgauccuuccgacccgaacgaccccggcugcccgcccggcuggucguggucgggaacuaccugcgucaaggccccgaccgaucccacggauccaaccgacccgaccacgccgggcagugacggcggcggcgauggcaauggcgguggaaacaauaacggcggcggcaaugacggcggcaccggcaauggcggcgacggcagcgggggaggggacggcaacggcgggggcgaugguagcggcgacggugacggcagcggcacgggcggcgauggcaacggcaccugcgacccggcgaaagagaacugcuccaccggccccgaaggccccggcggcgaacucaaggagcccacgcccggcaccugggaugacgccaucgccaccugggaaaagaaggucgaggacgccaagcaagaacucaagaccaaggugaaggccaacgucgaucagaugaagggcgccuucgaccucaaccuggcggaaggcggcgggcaacugcccugcgaguccaugaccauuuggggcaaguccuacucccucuguaucuccgacuacgccggccaacucuccagccugcgcguggcgcugcugcugauggccgcgcugaucgccgcccucauucugcugaaggacuga

SEQ ID NO: 72 - RNA, 1284 nt, Pseudomonas aeruginosa
auggccgucgccccugguguguuguugccgccgacgccugauguaaagcccaaggccgcugcgccgaagagccagcagaaaacgccugagcccaguaacgacaagacuuccagcuucuccgacauguaugccaaggagaccgcgaagaagcccgccgagcgcgccgacggucccgcgaaggguucgcgggacaagccacgggacgccggcaaggacgccgccgaagcgcagccgacggaugccgucaggcagccggccguugccgaagacggcaagccuuugccggccgacggccaggccaaggccgacggcgaagauaaagucgaaacgccggucgauccgcugcaauugcucggccucggcggugccguaccguugcucgacgagaauacccaggcgacuuugcugccaccggccgugccgacggccagcagugcuccggccagccuuaccgaagccagcagcgacccgacccuggucaagcucaacggcgugccggcggugaacauggcccuggagcagggcgcccaggacgccgcgcagacggcgaaaggcgggccggcgaagagcgccgauccccgccaggcgaaccucggcgaugcccuugccggccugaccucggauuccuugaccaaggccgucgacggcaaggcgcucgaggcccaguugcagcagaccgccgagccggccgucgccagcgccgccuccgagagccugcuggagagcaaggcggaaccccgcggugaaccuuucgcggccaagcucaacgggcugacccaggccauggcgcaacaggcccugaccaaccguccggugaacggcacggugcccggccagccgguggcgaugcagcagaacggcuggagcgaggcggugguggaccgggugauguggauguccagccagaaccugaagucggcggagauccagcucgaccccgccgagcugggacgccuggacgugcgcauccacaugaccgccgaccagacccaggugaccuucgccagucccaacgccggcguucgcgacgcccuggaaagccagaugcaccggcugcgcgacauguucagccagcagggcaugaaccagcucgacgugaacgucuccgaccagucgcuggcgcggggcuggcagggccagcagcagggcgagggcggaucggcgcgcggacgcggcuuggccggcgaggccucgggcgaugaggaaacccucgccggagucagcgagauccgcagccggccgggugcgucggcggcgcgcggucuggucgacuacuacgccuga

SEQ ID NO: 73 - RNA, 1287 nt, Pseudomonas aeruginosa
augcuccgccuccuuccucuccugcuaucccucgccugucucgcuccggccuucgccgacgagcgcgccgacacccaacgccagcuggaacagacgcagaaggacaucggcgagcugaagaagcugcuggacggcauccagcaggaaaagagcggcgugcagaagcagcugaaguccaccgagaccgagaugggcgaccuggaaaaacagaucaaggcccugcaggacgagcuggacaagagcgaagccgagcugaaacggcuggauggggagaaaaaaaaacuccaggacgcgcgcauugagcagcagcgccuccucgccauccaggcccgcgcggccuaccagaguggacgcgaggaauaccugaagcugcugcugaaccaggaacacccggaaaaauucagccgcacccucaccuacuacgacuacaucaacaaagcccgucucgaacagcucgccagcuucaacgaaacccuccgccagcuggccaacgucgagcaggacaucucugcgcagaaagccgaacaacugagcaagcaaggcgagcuggacagccgccgcgaggcgcuggcagcgacccgcaaggagcgccagcaagcccuggccaagcugaacagcgacuaccgcgaacgcgaccagaagcucaagucccgccaacaggaccaggccgagcuggccaagguacugcggaccaucgaggaaacccuggcccgccaggcccgcgaagccgccgccgcggcggagcgcgagcgccagcgcgcgcuggccgccgaacgcgagcgugcgcgccagcagcaggccgcccccggacgagucaccagcccgccgcgcgaaccugcgccgggcccgcuggucucaagcacuggcgcggucuacggcggcgcguucggcucggcccgcggcaagcugccguggccggugaauggccgcgucguggcgcgcuucggcagccagcgcggcgacgauccgcgggcgaaaugggacggcguacugauuucggcgagcgccggcagcaccguccgcgcggugcacggcggacgcgugguauucgccgacugguugcgcggagccggccuguuggucauccucgaccacgguggcggcuaccucagccuuuauggccauaaucaaagccugcugaaagacgccggcgacaccgugaaggccggagacccgaucgccaccguuggaaccagcggcggccagaguagcccggccguguacuucgccauucgccaucagggccgcccggcggacccuacuaccuggugccgcgcacagggauag

SEQ ID NO: 74 - RNA, 1707 nt, Pseudomonas aeruginosa
augcaaagacugucgcguaucggccgcaacacccucgccgucuccguuuccaccuugcuccucagcgccugcaaccagggcgacgaugcgccgaagccugcggcagucgcgccgcaaccggccgcaccgagcauggcugcacugagcaucccgcuaugccucaacggccagugcgcggugaucgaccaggacgccaagcugcucgugccguucgacaacgacuacgacaauaucgucgccagcgccuaccagggcacccugauggcggcgcgcgaggagcgcuggaaccugauccaggcgaaggacggcaagguguugcgcgacgauaucggcgaagcccugucgcugcucacccccaaccucuauggcuucguccgcgauggcaaguacggcguggucgacggccagggcaaggaaguccaggcgccgcguuucgacgacaucuaccccaacagugccaacgaauucaucaucuacgagaucgauggcaagcgcggcauccucgaugccaagggcaagcagcucaccgaggcgcucuacgacaccacccuggucaacggcagcgucgccgaacacgguggcuugaucagcgccgagcguggcgaggagaaguggaucaucaaccucgcuaccggcgaacagaaggccguggccuacgagagccugggcgaccuccacgacggcgugaugagcgccagcgucaucggcaagggcucccaacugguggaugccaagggcgacguggucggugacggcaagagcuacgauuaccugggcaccccggccaacggccuggucgcguuccgcgagaaguacgacagccccuguggcuaccucgacuaccagggcaagguggcgaucgccgcccaguucgccgguugcggcgccuucggcaagcagggcgggcuggcccagcagcgcauggaagauggcucgucgggcaaguacggccugaucgaucgcagcggcgccuggaaggugcagccgcaguacgauucggccgacagcgccggccucaccgcgcuuggcuacaccgucgacgugcccggccuggcugccgucggcgugagcaccggccuguucagcgccgacuucggcaucuucaaccucgacgaaggcagcgagugggugaagccggguuaugcgcagaucggcgcgcugggcaacgaccuguucgucguggcgaagaagggcgggccgcagaagaccgucagcuucauggguucggaaagccaggugccgguggugggccugauggaccgcagcggcaagaugcugcuggagccggacgaacugaucagcauccagucugcuuaugacggucguuuccuggaaggucucgacgguauggacaacgcugcccacaccguguugcucgaucgccagggacgcacgcugguuccagcgcucuggcagaagcuggaggugaauccgcagcaggguuacauccugggcuacgaagucagcggcacuggcgacgaggcgacggaaaccuugcgcgcacuguacgaccugaacggcaagccgcgcuucaccguggccaccaccgauugcggcgccgaacaguugcucgacggcaauggcaaggcgaucuggccgcaggacccgaccccguauugccagucggacgacgagcaggacgacgaaggcgagccggagcaggagccggcgcccgucgaagagagcgaggaaaccagcgagagcuga

SEQ ID NO: 75 - RNA, 1740 nt, Pseudomonas aeruginosa
augcuucgccccgccaggucucucucgcucugcuccgcccuggucauccugcucgccgccuguggcgagggcgaaccgcugcucccggccgaugcgcgccugccugacggcgcgcgcuaucgcggcgagcugguggacgggcgccuggaaggccagggccggcuggacuacgacaacggcgccugguacgccggccgcuucgagcauggccugcugcacggccauggcaccuggcagggcgccgacggcagccgcuacagcgguggcuucgcggccggccuguucgacggucagggacgccuggcgauggccgauggcagcgucuaccagggcgguuuccgccagggccuguucgauggcgaaggcagccuggaacaacagggcacucgcuaccgcggcgguuuccgcaagggccuguacagcggccagggcacgcuggacggcagcgauggcagccgcuaccagggcagcuuccgccagggccgccuggaaggcgaaggcagcuucagcgacagccagggcaaccaguacgccgguaccuuccgcgacgggcaacugaacggcaaggggcgcuggagcgggcccgauggcgaccgcuacgucggccaguucaaggacaaccaguuccauggccaggggcgcuacgaaagcgccagcggcgaugucuggaucggccgcuucagcgaaggcgcgcugaacggccccggcgagcuucucggcgccgacggcagccgcuaccgcggcgguuuccaguucuggcgcuuccauggccagggccugcucgaacaacuggacggcacccgcuacgaaggcggcuucgccgccggcgccuaugccggccaaggcacccuggaccgcgccgacggcagccgugagcagggacucugggccgacggcaagcgcauccgcgacgccgccggcaaggcccugcccgacacucuggaagucggccuguuggcccagggucgccugcucgacgaagaacugcgcaagaucccggccucgacgccggccagcgaacucuaugcccugagccugggcggcgauggccgccagggcguguuccugcgcgaggccgauuacgccggcgaccugcucggccagcguuucgccgcucguggcgugauucgccuggucaaccaccgcgaccacuucggcgaccgcccgcuggcuacccgggaaagccugucccgcgccgugcgcacccuggccgaacgcagcgggccggaagaccuggucuucaucuaccugaccagccacggcuccagcgaccaccaguuggcccuggacaugcccggccugaaccucggcgaccugccggccgcggaacuggccgaacugcucgcgccgcugcgccagcgcgacaaggugcuggugguaucggccugcuacagcgggggcuucaucccgccgcugaaagacgaacguacccugauccugaccgccgcgcgugccgaccgggucucguucggcuguuccgacgacgccgacuucaccuauuucggccgcgccuugcuggccaaugcgcugaaccgcaccgacgaucuguccaaagcguucgaacuggcgaaagaggaagugcgucaaagggagaaggaggaagguuucgaagcuucggaaccgcaagccugguuaccggaacgcgugcucgcgcacuggcggacgcugcgggggcagcaagccgagcgcgcgcucgcgucccgggaaggaaaaaccggcgagggcgcggcgggcaaauag

SEQ ID NO: 76 - RNA, 1866 nt, Pseudomonas aeruginosa
augcugcagaacaucagggauaauucccagggcuggaucgccaagaccaucauuggcgugaucaucguucuccugucgcugaccggcuucgacgcgaucauccgggccaccgaccacuccaacguggccgccaaggucaacggcgacgauaucagucucaaugaaguccaacaggccguggacaugcagcgucgccagcugcugcaacgccugggcaaggauuucgauccauccaugcuggaugacaagcugcucaaggaagcggcccugaaggggcugaucgagcguacccugcugcuccaggccgccaaggacgacaaguucgccuucuccgaccaggcgcuggaccaguugauccugcaaacucccgaguuccaggucgacggcaaguucaacgcggaucgcuucgaccaggucauccgccagaugaacuacagccgcaugcaguuccgccagaugcucggccaggaaaugcucaucggccagcuucgcgccggccuggcgggcaccgguuucgucaccgacaacgaauugcaguccuucgcucgccucgagaagcagacccgcgacuucgccacccuggcgaucaaggccgacgccuccaagagcagcgugagcgacgacgaggugaaggccuucuacgaaggccacaagagcgaguucaugacucccgagcagguggucgucgaauacguggagcugaagaaguccuccuucuucgaccaggucaaggugaagcaggaagaccucgaggcgcuguaccagaaggaaaucgccaaccuuuccgagcagcgcgaugccgcccacauccugaucgaggugaacgacaaggucggcgacgagcaggccaaggcgaagaucgacgagaucaaggcucgccuggccaagggcgaggauuucgccgcgcuggccaaggaguucucccaggauaucggcucggccgccaccggcggcgaccugggcuacgccggucgcggcguguacgaccccgcguucgaggaggcgcuguaugcgcugaagcaaggugagguauccgccccggugaagacuccguacggcuaccaccugaucaagcugcugggcgugcaggcgccggaaguaccgagccuggaaagccucaagccgaagcucgaggacgaacugaagaaacagauggucgagcagcgcuucgucgaggcuaccaaggaccuggaaagcuccgccuacgaagccgccgaccugagccagccggcgcaggaaaugggccugaagguccagaccagccagccguucggacguucggggggcgacggcaucgcugccaaccgccagaucgugcagaccgcguucagcgccgaggugcuggaagaagccgccaacaguggcgccaucgagcuggauccggacaccgugguggugcugcgggucaaggaacacaacaagccgaaggagcaaccgcuggagcaggucgcggcgaacauccgcgagcgccuggccgccgaaaaggccgccgaggaggcgcagaagcguggcgaggcccugaucgcagagcugcgugaaggccguaccucuuccgcagcgggugagucguggaaaguggucgaggcggccucccgcggccacgaaggcgucgauccgaaacugcuccaggcgguguuccgcaugcagcguccggaggccaaggacaagccuucguucucuggcgugacccuggccaauggcgauuacguggugauccgccugaauggcgucagcgagccggaggaggcuaucuccgacgacgagaaggccauguaccgccgcuuccuggcuucgcgcagcggacaggcagacuucgccgccuuccgccgucaguugcaggacaaggcggaagucgagaaauacuga

SEQ ID NO: 77 - RNA, 2067 nt, Pseudomonas aeruginosa
auggauaugacgucgcugaugccccuccugcugggagugggccuggucguucugcuggucgugggccugcuggcccuguucaaggccuucuacaucaaggucccgcaaggcaccgcgcugaucgucaacgacaugucgucgacgcccaaggugcauuucaccggugcgcuggucuauccggugauccaccugaaggaguucaugcgcaucucgcugaucacccuggaggucgaccggcgcggcaaggacggccugaucugccgcgacaacaugcgcgcggacaucaccguugccuucuaccugcgggucaacgagacccaggacgacgugcucaagguggccaaggccaucggcgucgaccgugcuuccgaccguucggcggugaacgagcuguucaaugccaaguucuccgaggcgcugaagaccgucggcaagcaguucgacuucguccagcuguucgagaaucgccaggacuuccgugaccgcaucaucgaggugaucggcaacgaccugaacggcuacguccuggaagacgucgccaucgacuaccuggagcagaccgcgaagaacucgcuggacccgagcaacauccuugaugccgagggcauccgcaagaucaccgagcugaccgccacccagaacgucaucaccaacgaacuggagcgcaacgaagagcuggcgaucaagaagaagaacgucgagacccgcgaggcggcccuggcccuggagcgccagcaggcugacgccgaggcccggcagaagcgcgagaucgagaccauccgugcccgcgaggaagcggaaaccgcgcgggucaaggaagaggagcggcugaaggccgagcaggcgcggauccaggcgcagcaggaaaucgacgugcgcaccgagaaccaccagcgcgaggucgagguggcgcagcagaaccgccagcgcgcgguggucaucgagguggagaaggucacccgcgccaaggaccuggagaucgucgcccgcgagcgugagguggagcugcagaagaucgagaaggaaaaggcgcuggaagagcagcgcaagaacauugccaaugugauucgcgagcgcgucgcgguggaaaagaccguggcccaagaggaggagcggaucaaggaggugcgcgagguuuccgaggccgagcgggucaagcaggugauacugcugcaggcccaggcggaagccgagcaggagcugguacgccaggucaagcaggcggaagccgacgaggcccgcuccaagcacaaggcgguggaaaucaacaccauggcgcaggccgagcuggaggcggcgucgaagcaggccgaggcgaagaagcgucuggccgagggcaucgaggccgagcgcgcagcgccgggccuggccgaugcgcgggugcuggaagucaccgccgcggcgaaggaaaaggauggcuuggcagcggcgcggguacgugccgaacaacugaucgccgaagccaggggcgacgaagagcgcggccuggccgacgcccgggugcucgaggcgcaggccgcggccaaggagaaggacggccuggccgaagccaaggugcuggccgagaagcucggcgcccaggcgcgcggcgaggagcagcucggcgcggccaaggccaaggccaccaaggaccagggcagcgcggaagcggaaguacugcugcagcgccugaaugccgaggccgaggggcuuggcaagaaguucggcgcccuggaugcccucagcgacagcgcucgccagcacgaagaguuccgcaugcagcuggagaagagcuucgaggaggccauggcggccaucgccgcgaacaaggacaucgccaaggaccaggccgaggugcucgccaccgcgcugggcaaggcgaacaucgagaucgucggcggcgagggcgacuucuucaacuccuucgccaagucgcugucggugggcaaggccaucgaagguguggucggcaagagcccgguggugcaggacguccucgcccgccugcucaacggccguggcgcagccgcugcggugaugccggaacgcaagagcggccacgagaacgagccggcggcggaagucuga

SEQ ID NO: 78 - RNA, 2229 nt, Pseudomonas aeruginosa
auguacccccaauuccgucgcggccaucucgccgcugccguccuuuucgcuucaucgagccugcugggcgggcaggcccuggccgaggacgagcgccuggaagaacuggacgaacgcgccgaaucggugguccagcugggugacgagguggugcugggcaccgccgaacaggagcucaagcaggcaccggggguauccaucaucaccgccgaggacaucaggaagcgcccgccggugaacgaucucuccgagaucauccgcaccaugcccggggucaaccucaccggcaacaguuccagcggccagcgcggcaacaaccggcagaucgacauccgcggcauggggccggagaacacccugauccuggucgacggcaaaccggucagcucgcgcaacucggugcgcuacggcuggcgcggcgaacgcgacacccgcggcgacagcaacugggugccgccggaggaggucgagcgcaucgagguccuccgugggcccgcggcggcacgcuacgguuccggcgcggcgggcgggguagucaacaucaucaccaagcgcccgaccgaucguuugcgugguuccaugacgguguucaccaacauuccggaaagcuccaaggauggcgccacgcgccgcgccaacuucagccuuagcgggccgcugaccgaagccuugagcuuccgcgcguacggcagcgcgaacaagaccgauucggacgauaccgacaucaaccucggacauaccgucaacccgagccguaccguggccggacgcgaagggguacgcaaucgcgaucucagcgggaugcugucguggcaggugacccccgaccaggucgucgauuucgaagcgggcuucagccgacagggcaauaucuaugccggcgauacccagaacaacaacggcaccgccaauacccagggacucgccgacgacggugcggagaccaaccgcauguaucgcgagaacuacgccaucacccacaacgggaccuggucguucgguacuuccagguucgucgcccaguacgacuccacccgcaacaaccgucuggaggaggggcuggccgguuccgucgaggggcagaucggcgccgaccguucguucagcgccagcaagcuggagaacuaucgccucagcggcgaacucaaccuuccguugcaugcguuguucgagcaggugcugacggugggcgcggaguggaacaaggaaacccucaacgacccguccucgcucaagcagggcuucgugggaagcgauagcuugccggggacccccgcggccggcucgcgaagcccgaaaagcaaggcggagauccgcgcgcuguacguggaagacaauaucgaacugcgccccggcaccaugcucacccccgggcugcgccuggacgaucacagcgacuucggccugaacuggagcccgagccugaacgcuucccaaacgcucggcgaauacuucacggucaaggccgguaucgcacgggccuucaaggcgcccaaccuguaccagagcaacccgaacuaccugcucuauacccguggcaacgguugcccgauccagacuagcagcggcggcugcuaccuggucggcaacgagaaccuggacgccgagaccagcguaaacaaggaacugggcaucgaguuccggcgcgauggcugggucgccgggcucaccuacuuccgcaacgacuacaagaacaagaucgucgcgccgcuggaugucaugggacagaccgggaccggcaacaacauccugcaauggagcaacgcgaagaaagcaguggucgagggccuggaaggcaaccugcuggucccccugcacgaggaccugagcuggagcaccaaccugaccuauaugcugcaauccaaggacaaggacaccggcaacccgcuuucggugauccccgaguacacccugaacucgacccuggacuggcaggccagcgagcgucuuuccacccaacugaccagcaccaucuacggccgccaggagccgccgaagcauggcaccagccgcaacacgccgguggucucgcgaaaagagguggguaccuauggcaucuggggcgucagcgccggcuacaccuucagcgagaaccugagcguacggggcgggguaagcaaccucuucgacaagcgccuguaccgccagggcaacuccuucgacgccggcgcggcaaccuacaacgagccgggucgcgccuacuacguuucgaugaccaccucguucuga

SEQ ID NO: 79 - RNA, 2241 nt, Pseudomonas aeruginosa
auguccucacgcgcccuucccgccguucccuuccugcugcuguccaguugccugcucgccaacgccguacacgccgccggccagggcgacggcuccgucaucgagcugggcgagcagaccguggucgccaccgcccaggaggaaaccaagcaggcgccggggguuuccaucaucaccgccgaggacaucgccaagcgaccgccgagcaacgaccugucgcagaucauccggaccaugccgggggucaaccugaccggcaacagcuccagcggccagcguggaaacaaccggcagaucgacauccgcggcaugggcccggagaacacccugauccuggucgacggcaagccggucagcucgcgcaacucggugcgcuacggcuggcgcggcgagcgcgacagccgcggcgacaccaacugggugccggccgaccaggucgagcgcaucgaagugauccgcggcccggcggcggcgcgcuacggcaacggcgcggcgggcggcguggugaacaucaucaccaagcaggccggcgcggaaacccacgguaaucucagcgucuacagcaauuucccgcaacacaaggccgaaggcgccagcgaacggaugagcuucggucucaacgggccgcucacggaaaaccucagcuaccgcgucuacggcaacaucgccaagaccgacucggacgacugggacaucaacgccggccacgaauccaaccguaccggcaagcaggccggcacccuccccgccggucgcgaaggcgugcgcaacaaggacaucgacgggcugcucagcuggcgccugacgcccgagcagacccucgaguucgaggccggcuucagccgccagggcaacaucuacaccggcgacacgcagaacaccaacagcaacaacuacgugaagcagaugcucggccacgagaccaaccgcauguaccgcgagaccuacucggucacccaucgcggcgaaugggacuucggcagcucgcuggccuaccugcaguacgagaagacccgcaacagccggaucaacgaaggccuggccggcggcaccgaagguaucuucgaccccaacaacgccggcuucuacaccgccacccugcgcgaccugaccgcccacggcgaggucaaccugccgcugcaccugggcuacgagcagacccugacccucggcagcgaguggaccgagcagaagcucgacgaccccagcuccaacacccagaacaccgaggaaggcggcucgauccccggucucgccggaaagaaccgcagcagcaguuccucggcgcggaucuucucgcuguucgccgaggacaacaucgagcugaugcccggcaccaugcucaccccaggccugcgcugggaccaccacgacaucgucggcgacaacuggagcccaucgcugaaccugucccacgcgcucaccgagcgggucacccugaaggccgguaucgcccgcgccuacaaggcccccaaccuguaccagcugaaccccgacuaccugcucuacagccguggccaggguugcuacgggcaaagcaccaguugcuaccugcgcggcaacgacggccucaaggccgagaccagcgugaacaaggaacugggcaucgaguacagccacgacggccugguagcggggcugaccuacuuccgcaacgacuacaagaacaagaucgaauccggccugucaccggucgaccacgccagcggcggcaagggcgacuacgccaacgcggcgaucuaccagugggagaacgugcccaaggcgguggucgagggccucgaaggcacccugacccugccccuggccgacggccugaaguggagcaacaaccucaccuacaugcugcaaucgaagaacaaggaaaccggcgacgugcucucggugacgccgcgcuacacccucaacucgaugcucgacuggcaggccaccgacgaccucucgcugcaagccacggucaccugguacggcaagcagaagccgaagaaauacgacuaucacggcgaccgugucaccggcagcgccaacgaccagcucucgcccuacgccaucgccggccucggcggcaccuaucgguugagcaagaaccugagccucggcgccggcgucgacaaccuguucgacaagcgccuguuccgcgccggcaaugcccagggcguggucggcaucgacggggccggcgcggcgaccuacaacgagcccggacggaccuucuauaccagccugaccgcgucguucuga

SEQ ID NO: 80 - RNA, 2355 nt, Pseudomonas aeruginosa
auguccccgucacgcgcccugucgccgcucagccgcgcccugcuccucgccugccucggcggucccguccugguuuccgccggcagcgccugcgccgccgagauccgcaccgaugcccgccaguacuaccgccugccugccgagccgcuggagcaggcgcugaaccaccuaggccgccaggccggcgugcugaucgccuucagcccggaacagaccgccgcgcgacgcagccaggcgcuggacggcgaguacacccuggaggaagcccuggccgcccugcucgucggcuccggccuggaggcgcgcgcccgcggcgacggcgccuacacccuggaagcgcugccgguggaagacccggccaaccugcaggcgcucaccguggucggcgacuggcuggccgacgccagcgccgccgacgucuucgagcaucccggugcgcgcgacgugguccgccgcgagcaguuccaggcccaaggcgcggccagcacccgcgaagugcuggagcgcauucccggggucagcgcgccgcucaacaacggcaccggcagccacgaccuggcauugaacuucggcauucgcggccucaacccgcgccuggcgucgcgcucgacggugcugauggacggcaucccggugcccuucgcccccuacggccagccacaguugucgcuggcgccgguguccaucggcaacauggacgcgguggacgugguccgcggcggcggcgcggugcgcuacgggccgcagaacgucggcggcaucgucaacuucgugacccgggcgauccccgaggacuucgccaccaagcucgacgugcacagcgaacucagccccagcuccagccaggacggccugaagaccacccacaacgugcugaucggcggcaccggcgccaacggccucggcggcgcccugcucuacuccggcacccgcggcggcgauuggcgcgagcacagcgauacgcggaucgacgaccugauccucaagggccgcuuccagcccagcgacgaacacacguuuucggcgaugacccaguacuacgacggcgaggccgacaugcccggcggccucggcaccgcggccuaccacgacgacccguaccagucgacccgucccuacgacaaguucuggggccgccguacccuggccagcgccagcuacgaauacacccccaacgccagccagaagcucaacgucaccggcuucuucaccaagacccugcgcagcggcuaccucgaccagggccgcaaccucacccugucgccgcgcgaauacugggugcgaggccuggaaacccgcuucagccagggcuucgagcugggcgaaagucgccacgaagugggcaucggccaccgcuacgucaacgaagccagccacgagcugcgcuacuggacccgcgccgacagcggccagcuacccagcaccggcagccgcaacgaccgcgacacccgcggcagcaccgaagccaacgcguucuacaucgacgaucgcaucgacaucggcaacuggaccaucacccccggcauccgcuacgagaagaucgauuccgaacagaagaaccugcugaagaacagcaaggacagcggccgcuacaacgccucgcugccggcgcucaacgugaucuaccaccucacgccgagcuggaaccucuacgccaacaccgagggcucguucggcaccgugcaguacagccagaugggcaaggcggugcgcagcggcgacaucgagccggagaaggcccgcaccugggaacucggcagccgcuacgacgacggcauccugcgcgccgaacugggcgccuuccugaucaacuucgacaaccaguacgagagcaaccagcagaccgacagcgugaccgcccgcggcaagacccggcacaagggcaucgaggcggcgaucgccuacgaccuggccgaucucgacccgcugcucuccggcuucgacgucuaugccagcuacgccuacgucgacgcgagcauucgcgaagacgggccgaacaagggcaaccaggugccguucuccucgaagcacaagggcacccuuggcgccaacuaccgcaccggcgccuggagcuacaaccucgacggcagcuuccagaccagccaguacgccgacaacgccaacaccgagagcgaaagcgccgacggcagcaccgggcggaucgccggcuggauggucuggagcgcgcgcggcaccuacgacuucggcccgcaacugaacgaccucaagcucggccugggggugaagaaccuguucgaucgccgcuacuacacccgcucguucgacgacaacaacaagggccucuacgucggccagccgcgcacccuguacguacaggccucggucgguuucuga

SEQ ID NO: 81 - RNA, 2556 nt, Pseudomonas aeruginosa
augaccuugccuuucacccgcgccgccuggcgcccgcuguguuccgccgccgugcucggcgccgcguugugggccgccggcgccagcgcugccgaacgacgcuucgaccugccggcgcagccgcuggccgccucgcugucgcgccuggcgcagcaggcgcagguccaggugcuguucgacgagucgcuccugcggggccugcgcgcuccggcgcugagcggcagcuacggggugcgcgaggcgcuggagcgguugcuggucgguuccgagcuggagcugguggaggcgggcggcggcuacguggugcgccggcgccaggucgacgccuacagcgacaacgcgcugcaacuggacgcgcagaccaucgucggcaacggucgcgaaguggacgccagcaacgucggccguucgacccugacccggcgggauaucgaacgccagcaggcggacaacauccccagccugcugcagacccugcccggagugaccaugggcggcucgcccaagccgggcggacagaccaccaacaucuggggccugggcgacgccgaggacgugcccuauacccuggacggcgcgcagaagagcggcuucgagcgcuaccagcagggcaccguguucaucgaaccggaaaugaucaagcgcaucgagguggagaagggaccgcacucgguguucaccggcaauggcggcuucggcggcaccgugcacauggagaccaaggacgcgccggaccugcugcgcgaaggccgcgacgucggcgccaugcucaaguacggcuaucacuccaacgaccagcagaagaucuacuccggcgccguguucggucgcagcgaagaccgccgcgucgaugcccugcucuaucucaacggucgcgacggccgcgacaugaagcuggccgacaaccugccgcugucgcccaccgacuacccgaucaaccccaagcgccugcccaacagcgcccaggacgagaagaccggccuguucaagcucaaccugcaccccaccgaggagcacgaccuggguuucaccuaccugcgcucgaaaagcucgcgcuggacgccguucuccgccagcagcuacccgaccccgccgagccaguggaccaucgaccgcuacggcuacgagcugggccugacccgccugcuggcccaccgcgauaccaccgacaccaccuggaccggcaaguacaacuaccauccgcuggacaaccccuggaucgaccugcaacugagcuauuccgacgcccgcaccgagcaacucgaccgucgcgaggacaccgccuucuaccagcucgccaccgguggcaagcggaugcguaccgaguaccaggacaagguccuggaacugcgcaacaccagccguuucgauaccggagcgcuacagcacgagcugacccugggcgcggcgcugcacaagcacaagcgcgacauccucaugcacaugccgggcaagaccuacgagaccccgcgcuacaauuacggcuggcugcaaccggcauucaugccggccggcaagcaggacacgcagagcuucuacauccaggacgcgaucaccuacggcagccugaccgucaccccaucgaugcgcuucgacagcgugcgcaacgacggccaggccaaccuggcgccgaucuacgacaaucccaagcucggccaugacuaucgcgcccagaccuacuccggcuggucaccgcggcugucgguguucuggaccgcgacgccgaaccuggcguucuucgccgacuacaccgagaccuggcgagcgccggugaucgacgagcaguacgaagugcagaacaguucgaccaucgguggcagcagccgcgaccuggacgccgagcgcauccaugcgauccguggcggcagcgugaucaaccugccggaccugcuggucgccggcgacagccugcagauccgcaccacguuguuccagaaccgcaucaaggacgagauauuccgcacccgcagcgucggcugccgccagcagucgaucgacaacggcaguaucggugguagcugcggcgacaugcugccgcugagcaacuaccgcaacuugccgggccugaccaucaagggcuucgagaucgagagcuucuacgacagccagcggcuguucggcagccuguccuacucguggaugaccggcaagcacgauggggccuacagcaaucccuggggaccgaacgugugggcgcgcgacaucccgccgccgaaguggguggccaugcucggccugaagguuccggaaugggaugccaagcucggcuggcagggcgaguucgugcgcaagaccgaccgccugcccagcgaucgcuacagcggcgggauggguaccgguuccggcgauaucuacugggaucacgcggccaacgacagcuacgacacucaucggcuguucgccgagugggucccggccaagcugggccugaaggacacccgcaucgacuucaccguggacaaccuguucaaccgcuccuaucgccagccgcugggcggcgaccuggucuacagccagggacgcaacgccaagaucagcgucacccaguucuucuga

SEQ ID NO: 82 - RNA, 2643 nt, Pseudomonas aeruginosa
augcaccgaucgcuccacaccgacgcgccgcugggcgccgcccugcugcuggcccugcagcucgcucccggcagcgccgccgcggcggaggaacaggcgccugucgacccgcccacgguccaguugcaacgaaucgaggugaccggcagcgcgauccgccgggucgaugcggaaaccgcggugccgaucagcguccugcgcgccgaggagcugcgccaacagggcgugaccagcaccgaggaacugaucggccggcuuuccggcaaccagggcguauacaacuccagucgcucggucggcagcgccaccggcggcgccucguucgccgaccugcgcggaaucggcgcgaacaagacccuggugcugcucaacggccggcgccuggcgaacaaugccaucgacggcuccgcgguggaucucaacaccauucccuucgccgccaucgaccgggucgaggugcugcgcgacggcgccuccgcgcuguacggcaccgaugccaucggcggggugaucaacuucaucacccgcaagagccugaacgaaggccgcuucgacagcggcuacgccucccccacccacgacggcggcggcaaccagcgcaacgucagcgcuagcuggggcuucggcgagcuggaggaggaucgcuucaaugucuucgcgguggccaacuacgacaagcaggagcgccucggcgccaaggaccgcggcuacaccuacaacuaccagccgggacgcggccucgacuacagcuccggcaccgccuuccccggcaacuggagccagggcgccaacgccagcaauccgcuggccgccggcgguugcaagggcgccgaccugauuccgcgcaacggcaucugccggcagagccuguggcgcuaccucgaccuggugccggaaaccgagaagaccucgguguucagccgcgccaccggcaagcuggccgacgagcacaacgucagccuggaguacuucuggucgcgcagcgacaacgcuacccaggucggcccagggacccucaccggccugcagaucgaucccggcaccgccuucuaucccggcaacggcaucacucccggacccggcggcuucguccucgacccgagccggccgguggaggucaacuggcgacagagcgugcucgggccgcgccugcaauccucgcagaacaccggccagcgccugcugcucggcuucgacggccaguucgccggcugggacuacgauaucggcgccucguacaaccagaacaagguggucgaccauauccacagcggcuacgucgaugaucgcgccgccgcccucggcaucgccaacgggacgcugaacccguucgggccgcagaccgacgccggccucgccuaccucggcagccaugcccugagcggcgacuuccguaccucggucggccgcgucaagggccuggacgcccgcgccagccgggagaucggcgacugguucggcgccgggccggcggcccuggcgcugggcggcgaguuccgcaaggaagcguuccaccaggacauccaggacuucgccggcaacgugcagagccucggcgucgaucccgccgccacggucagcggcgagcgcaaccugaaggcgcaguacgccgaacucaacgugccggugcuggacagccuggaacucagcgcggcgauccgccacgacaaguacagcgacuucggcagcaccagcaacccgaaauauucguuccgcuuccagccguuccgccaguugguccugcgcggcgccuacagcgaagguuuccgugcgccgucgcuguacgaacuguacaacccgaccuucaccaccuauaccagcgccaacuacgacgacccgcgccugugcgccggcggccagccgagccagggcggcaucgccaaccgcgacugcgcccagcaguucuacaacgccaccggcggcaauaccgaccugcgaccggaaaccgcgcgcaacguuacccugggccuggucuaccagccgcugcgcgaccuuuccgucggccuggacuucugguggaucaggaucgccaaccagaucgccgaguuucccgaagcggcgaucuucgccgacccgcaggccuacgccggacgcaucgugcgcaaggccgacggcucgaucgaucacgucgucaccggacuggccaaccucggcaaagugaagaccagcggcgucgaccugagccucgauuaucguuucccggccagccgcuacgggcaguucgggcucgaccugcaaggcaccuacgugucccgcuacgacuuccagcagcagaucggcggccaguaccuggacaacgucggcgacuuccagggcgucggcgugaucgcccgcuggaagcacgucgccaacgccaccuggagccgcgacgccuggcaggccacccugagcaaccgcuacaccagcggcuacaacgacuacgaccgcgccagccacggcaaggucggcucguggaaccucugggaccuggccggcagcuaccgccucagccacgcgcuggggcugacccucggggugaagaaccuguucgaccgcgaaccgccguucagcaaccagaccuacaccuuccagagcggcuacgacccgcgcuacaccgaucccuacgggcgcauccuguucggccgccucagcuacagcuucuga

SEQ ID NO: 83 - RNA, 2760 nt, Pseudomonas aeruginosa
augguucggcuucguacacugguucgggcaaucgcggcggccucgguccugacuuccggcauggcgcauggauugggacugggggaaaucacccugaagucggcguugaaccaaccguuggaugccgagaucgagcugcucgaaguucgugaccuggguucgggcgaggugaucccgagccuggcgucgccggaagaguucagcaaggcgggcgucgaucgccuguacuaccucaccgaccugaaguucacgccgguggugaagcccaacggcaagagcgucauucgcgugaccucgucgaagccggugcaggagcccuaccugaacuuccugguccaggugcucuggccgaacggccgccugcugcgcgaguacaccguccugcuggauccgccgcuguacuccccgcaggccgcggcaagcgcuccgcaagcgccggucagcgcgccgcgcgcgaccggcgccccgcgagccccgcaggcuccggcuccggugcguaccaccgcgccggcaggcagcgacaccuaucgcaccguuuccaacgacacgcucugggagaucgcccagcgcaaccguaccgaucgcguuuccguaccccaggcgaugcucgcguuccaggagcugaauccgggcgccuucgucgauggcaacaucaaccggcugaagagcggccagguccugcgcauucccaccgaacagcagaugcuggagcgcucgccgcgcgaggcgcugucccaggugcaggcgcagaaccagagcuggcgcggcagccgcaauccggccgcgggcagcgcuggcgccaggcaguuggaugcgacccagcgcaaugccgccgggucggcgccauccaaggucgacgccacggacaaucugcgccuggugucuggcgagggcaaggccagcaagggugccgacaagggcggaaagggcgacagcaaggcgaucgccgauacccuggcggugaccaaggaaagccucgacagcacucgccgcgagaacgaagaacugcagagucgcaugcaggaucugcagagccaguuggacaagcugcagaaguugauccagcugaaggacgcccaguuggccaagcugcaagggcaguugggcgccgaaggccagggcgcagcccagccgaacgcagcccugccggaugcgucccagcccaaugcggccgcgcaggcgccggcucagcccgggacuccugcugcggcagcgccgacuccugcuccagccggagaagcacccgccgcuccggcgcagccuccgguggcgccgccgcccgcgccagcugccgagaagccuccggcaccugccguuccggcgcccgcuccgguacaggcggcagagcagccggcaccgagcuuccucgacgaacugcuggccaacccgcugugguuggcggugaucggcgguagcgcacugcuggcguugcuggugcugcugaugauccugucgcggcgcaaugcgcagaaagagaaggaagaagcccaggcuuucgccgcggauaccggcgaggaacaggaggaugcgcuggaccugggaaaggacggcuucgacgaccugacccucgacgagccugagccgcaggucgcagccgucgcuccgcaggucgagaagaccaccgcgcagacuuccgaugcgcugggcgaggccgacaucuauaucgccuacgggcguuucaaccaggccgccgaacuguugcagaacgccaucuacgacgagccgcagcgcaccgaccugcgccucaagcugauggaagucuaugccgagaugggcgaucgcgaagguuucgcucgccaggaaaacgagcugcgcgaaaucggcggcgcacagccgcaggucgagcagcucaagucgcgcuauccggcaauggucgcggucgccgcgguugccggccuggccggcgccaagcuggcgcaggacgagcuggauagcuucagccuugacgaccugucgcucgacgacagcggucacgcggccaagccggaugcggcaggacaggaucucgacgacgccuucgaccugagccuggacgaccugggcggcgacgacgugcaggccgaccucaaguccgacagcggggcgcuggacgaccugacccuggacagcgaucuggaccuggcggccucgaccccggcggacaagccugucgacgaucucgacuucggccuggauuucgcggaguuggcagagacuccgagccaacccaagcaugacgaccugggcgauuucucccuggaucucgacgcgccggaagacaagcuuucggacgacgacuuccugcuuucgcugaacgacgaagugcccgccgcggcgccugccgacaacgaauucacccucgauaccgaggcugccgaagagccggcguugucccugccggacgacuucgaccugucgcuggccgacgagccgacggagccggccgcuccggagaagggcgaggacaguuucgccgcccaguuggacgaggugagugcgcaguuggacgaguuggccagcaaccuugacgagccgaagagcgcgacgccgaguuucuccgccgaagaugcagcggucgccuccgcccuggacggagacgccgacgaugacuucgacuuccucuccggugccgacgaagcggcgaccaagcuggaucuggcucgcgccuacaucgacaugggcgauagcgaaggcgcgcgcgauauccucgacgaaguccuggccgaagguaaugacagccagcaggcggaagcccgcgaguugcuggagcgccuggccuga

SEQ ID NO: 84 - RNA, 2988 nt, Pseudomonas aeruginosa
augaccgacgaccacuccuuccgcccucgccccaccucguugucagccgcccugcugcugggcgccuggaucgcacagccggccacggccgccuaugucgaagccggucggcccggcgauccggccaguuggcgcuccgccgaauaccagcaggacuggggccuggaacggaugcgggccgaccaggccuaugccgccggcaucgacggccagggcgugaagaucggcgagauggacuccgguuucgacccgagccauccggauacucccgccucgcgcuaccagccggugacggccagcggcaccuaugucgacggcacgccguucagcgucagcggcgcgaugaacggcaacaacgacucccacgguacccacgucggcggcacccucggcgccucgcgcgacggcgucggcaugcacgggguggccuacgcggcacagguguaugucgccaacaccaaccagaacgacagcuuccuguucggcccgacgcccgacccgaacuauuucaaggccgccuaccaggcgcuggccgacgccggggugcgggcgaucaacaacaguuggggcagccagcccaaggacgucagcuacgagacccucgacggccugcacgccgccuaugcccagcacuacgggcgcuccaccuggcuggacgccgccgccggcgucucccgccagggcgugaucaacgucuucagcgccggcaacagcggcuacgccaacgccagcgugcgcuccgcccugcccuacuuccagccggaccuggaaggccacuggcuggccguguccggccucgaccagcagaacggccagcgcuacaaccgcugcggcaucgccaaguacuggugcaucaccacgcccggccgccugaucaacagcaccaugcccggcggcggcuacgccaacaaguccgguaccucgauggccgcgccccacgccaccggcgcgcuggcccuggucaugcagcgcuauccguaccugaacaacgagcaggcgcugcagguucugcugaccaccgccacccagcucgacggcacgccgaccggcgcccccaccgacaccgucggcuggggcgugccggaucucggucgggcgaugcaugggccuggacaauugcucggccgcuucgaggccaaccucccggccggccugcgcgacgaauggagcaacccgauuuccgauagcgcccugcuccagcgccaggccgaggacgccgccgagcacgcggccuggcagcggacgcugaaggacaagggcugggaaaacggcuugccggccggugccagccagcaggaacgcaccgacuaugccaucggcauggcccgcgaccaggccgccgcccagcgccaguaccagggcagccuggucaaggccggugccggcagccugguccugagcggcgacagcaccuaucgcgggccgacccuggucgauggcgggcugcucagcgucgacgguucgcugcuguccgccgucgaagucaaugccggcggcacccucggcggcagcggcaggaucggcggccugcuggcgcgcuccggcggcacgguggccgcgggcaacuccaucggcacccuggaggucgccggggaccugcgcuucgaauccggcucgaccuacgcgguggagcuuucggaaagcgccagcgaccggaucgucgccagcggcaaggcgagcaucgcgggcggcaacgucacccuggccauggaaaacagccccgaccugcucagccagucccaggucgagagccuggucggccgccgcuacgacauccucgacgccgccggcggcaucgacgggcgcuucgacgcgguauugccgaacuaccuguuccucggcggcacccuggacuacgcggccaacgccauccgccuggauaucggacgcaacggcacgacccucgccagcgucgcgcagacgcccaaccaggcggcggucgcuggggccguggaaacgcucggcgccggcaacccggucuacgaaagccugcuccugucggaaaacgccgcaaccgcccaacgggccuuccagcaauuguccggggaaaucuacccggcgcucgccggccuguugcucaacgacagccgcuaucugcgcgacagcgucggcgaacgccugcgccagaccagcgacggcgaggccggcggggaggcucccgaaggcugguucaaggcgcucggcuccuggggcaagagcgccgauggcagccacgguagcgaaggcuaccggcauucggucggcggcuuccugcucggcgucgacagccaggucgccagcgacacgcgccucggccugguggccggcuacagcaacagcucgcugaacauggacagcagccugcaauccuccgccagcaucgacagcuaccaccucggcgccuaccucggccggcaauugcagcaauggcgccugagccucggcgcagcgcacgccuggcaccgcgccgaggucaagcgcgaccugcaauacggcgccguggccggcaagcagaaggccaagcucgacgcacagagcagccaguuguucgccgaggccgccuacgcgcuggguuggcgcagccuggagcuggaacccuucgccgggcuggccuacgugcacgucgccagcgaugacuuccgcgaacgcgguagcgccgcggcccuggaggguggcgacgacaaccuggacgccgccuucaccacccugggccugcgcgcgaaacggcauuucgagcuggaugccggacgccgccuggcgcucuccggcacccucggcuggcgccacaaccugagcgacaccaccccgcaacgccaccuggcguucgccagcggcagccagccauucagcguggaaagcguggcccugucccgcgacgccgcgcugcucggcgucgacgccagccucgcggugaaucgcgaagugagcgugcggcugggcuacaacggccugcugggcagccgcgagaaggaccauggcgucggacuggccgucgacuggcguuucuga

SEQ ID NO: 85 - RNA, 3174 nt, Pseudomonas aeruginosa
augaaaagaaugcugaucaacgcgacucaacccgaggaguugcguguugcacuggucgacggccaacgccuguucgaccucgacaucgagucgggcgcccgcgagcagaagaaggccaacaucuacaaaggccgcaucacucgcgucgaacccagccucgaagccgccuucgucgacuucggcgccgaacgccacggcuuccucccccucaaagaaaucucccgcgaauacuucaagaaaucccccgaaggccggaucaacaucaaggaaguccugagcgaaggccaggaagucaucguccaggucgagaaggaagagcgcggcaacaagggcgccgcccugaccaccuucaucagccuggccggccguuaccuggugcugaugccgaacaacccgcgcgccggcggcaucucccgccguaucgaaggcgaagagcgcaacgagcugcgcgaggcccugaacggccucaacgcaccggccgacaugggccugaucgugcgcaccgccggccucggccgcagcaccgaggaacugcagugggaccucgacuaccugcugcaacuguggagcgcgaucaaggaagcguccggcgaacguggcgcgcccuuccugaucuaccaggaaagcaacgucaucauccgcgccauccgcgacuaccugcgccaggacaucggcgaagugcugaucgacagcaucgacgcccaggaagaagcccugaacuucauccgccaggugaugccgcaguacgccagcaaggugaagcuguaccaggacagcguuccgcuguucaaucgcuuccagaucgagagccagaucgagaccgcuuuccagcgcgaagugaagcugccguccggcggcuccaucgucaucgacccgaccgaggcccugguuuccaucgacaucaacucggcgcgcgccaccaagggcggcgacaucgaggaaaccgcccugcagaccaaccuggaagcggccgaggaaaucgcccgccagcugcgccugcgugacaucggcggccugaucgucaucgacuucaucgacaugaccccggcgaagaaccagcgcgccguggaagagcguguccgcgaagcccucgaggccgaccgcgcgcgcguccaggucggucgcaucucgcgcuucggccugcuggaaaugucccgccagcgccugcguccgucccucggcgagaccagcggcaucgucugcccgcgcugcaacggccagggcaucauccgcgacgucgagucgcugucgcuggccauccugcgccugaucgaggaagaagcccugaaggaccgcaccgcggaaguccgcgcccgcgugcccuuccaggucgccgccuuccugcucaacgagaagcgcaacgccaucaccaagaucgaacugcguacccgcgcgcgcaucuucauccugccggacgaucaucuggaaaccccgcauuucgaaguccagcgucugcgcgaugacagccccgaacugguugccggccagaccagcuacgaaauggccaccgucgagcacgaagaagcccagccggucagcucgacccgcacccugguccgccaggaagcagcagucaagaccgucgcuccccagcagcccgcaccgcaacacaccgaagcaccggucgagccggccaagccgaugcccgagccgagccuguuccagggccuggugaagucccuggucggccuguucgcaggcaaggaucaaccugccgccaagccugcugaaaccagcaagccggcugccgagcgccaaacccgccaggacgagcgucgcaacggccgccagcagaaccgccgccgcgauggccgcgauggcaaucgccgcgacgaagagcgcaaaccgcgcgaggagcgugcagagcgucaaccgcgcgaagagcgcgccgaacgcccgaaccgcgaagagcgcagcgaacgucgccgcgaagagcgcgccgagcgcccggcucgcgaggagcgccagccgcgcgaaggccgugaagagcgcgccgagcggacaccccgcgaagagcgccagccgcgcgaaggccgcgaaggucgcgaggaacgcagcgaacgccgccgcgaagagcgcgccgaacgcccggcccgcgaagagcgccaaccccgcgaaggccgugaagaacgcgccgagcgcccggcccgcgaagagcgccagccgcgcgaggaucgccaggcucgcgacgccgcggcccuggaagccgaggcauugccgaacgacgagagccuggagcaggacgagcaggacgauaccgauggcgagcgcccgcgccgccgcucccgcggccagcgucgucgcagcaaccgccgcgaacgccagcgcgaggucagcggcgagcuggaaggcagcgaggcgaccgauaacgccgccgcgccgcugaacaccgucgcagccgccgccgcugccgguaucgcugucgccagcgaagccguagaagcaaacguggagcaagccccggccacuaccagcgaggcugccagcgaaaccacggcaagcgaugagaccgacgcgucgaccagcgaagccgucgaaacccagggcgcggacagcgaggccaauaccggcgaaaccgccgacaucgaagcgccggugaccgucagcgugguccgggacgaagccgaccagagcacccugcuggucgcgcaagccacugaagaagcucccuucgccagcgaaagcguggaaagccgcgaagacgccgagagcgccgugcaaccggcaacggaagcggccgaagaaguugccgcuccggugcccgucgaaguagcagccccuagcgagcccgcagccaccgaggagccgaccccggccaucgcggcggugccggccaacgcgacuggccgugcccucaacgacccacgggaaaaacgucgccugcaacgcgaagccgagcgucuggcacgcgaagccgcagcagcagccgaagcggcagcucaggccgcucccgccgucgaggagaucccggcuguagcgagcgaggaagcgucggcccaggaggaaccugcugcaccccaggcugaagaaaucacccaggccgacguuccgucccaggcggacgaagcccaggaagcgguacaggccgagccugaagcuuccggcgaaggcgccgccgacacggagcacgcgaaaaagaccgaggaaagcgaaaccucgcgcccgcaugccuga

SEQ ID NO: 86 - RNA, 3486 nt, Pseudomonas aeruginosa
augaaaucgguacuccaccagaucggcaagaccucgcuggcagccgcgcucagcggcgccguccugcucuccgcccagaccacccacgccgccgcccugucggucagccagcagccgcugaugcugauccagggcgucgccccgaacaugcuggugacucucgacgacucgggcaguauggcguucgccuaugcgccagacagcauuuccggcuauggaaacuauacguucuucgcgucgaacagcuucaacccgauguacuucgauccgaacacgcaauacaagcuuccgaagaaacucacacuggugaacggacagguacagauccaggauuauccggcccccaacuucuccucugccuggcgcaauggcuucacucgcagcgggaguaucaaucugucgaacagcuacaaggucaccaucgaguacggcaggggauaugauaaggagucgacgauaaaagccgacgcugccuacuacuaugacuucacgggcucauccaguugcaaccgcaccaaucaggcaugcuacacccgccguuaugugagcacagagcaaaggcagaacuucgccaacugguauucguucuaccgcacccgcgcccuugccacucagaccgccgccaaccuggcguucuacagccugccugaaaacgcucgggugagcuggcaauugcugaacgacucgaacugcaaccagaugggcagcggcuccagcuccggcaacuguuucagcaacuaucuacgggacuucaccggucaacaccgggugaacuucuucaauuggcuggaaaaacuuucggucaauggugguacgccacugcgccaggcgaugacccgggcaggcgaguuucucaagaagaccggcgucaacggucccuaugccuaucgcccagggacccagaccgcgcccgaguacaguugccggggcagcuaucauauccugaugaccgacggucucuggaacaacgacucggccaacguaggcaaugccgacagcaccgcucguaaccuccccgacgggaagagcuauagcagccagacacccuacagggacgguacguucgauacccuggccgaccaggccuuccauuacugggccaccgaugcccggccggauaucgacgacaauaucaaaccguacauucccuacccggaccaggccaaucccucggcggaauacuggaauccccgcaacgauccggcaaccuggcaacacauggugaccuacacccugggccugggccugaccaccagccucaccaguccgagaugggaaggcuccaccuuuuccgguggcuacaacgauaucguggcuggcaaccugagcuggccccgcgcgucgaacaacgacuccaacaacgucuacgaucuguggcacgccgcagugaacucccggggcgaguucuucagcgccgacucgccggaccaacuggucgcggccuuccaggacauccucaaccgaauuucgggcaaggaccugccggcaucccgccccgccaucagcucgucccugcaggaagacgacacuggcgacaagcugacccgcuucgccuaccagaccagcuucgccagcgacaagaacugggcuggcgaccugacccgcuacagccugaccacccaggacaaggccaccgugcagaccaagcuguggagcgcgcagagcauccucgacgcgaugcccaacgguggagcuggccgcaagaucaugauggccggauccgguaccucgggccucaaggaguucaccuggggcagccucagcgccgaccagcagcggcaguugaaccgcgauccggaccgcaacgaugucgccgacaccaagggccaggaccgcguggccuuccugcgcggcgaucgccgcaaggagaacagcgacaacuuccgcacccgcaacucgauccucggcgauaucaucaacuccucgccggcgacggucggcaaggcccaguaccugaccuaccuggcccagccgaucgagcccagcgguaacuacuccacguucgcagaagcacagaaaacccgugccccgcggguauacgucggcgccaacgacggcaugcugcacgguuucgauaccgacgguaacgagaccuucgccuucaucccaagcgcggucuucgagaagcuccacaaguugaccgcccgcggcuaccagggcggcgcccaccaguucuacgucgacgguucgccgguggucgccgacgccuucuucggcggcgccuggcauaccgugcugaucggcagccugcgcgccggcggcaagggccuguucgcccucgacgugaccgaucccgccaacaucaagcugcucugggaaaucggcguggaccaggagcccgaccuuggcuacagcuuccccaaacccacggucgcccggcugcacaacggcaagugggccguggucaccggaaacgguuauuccagccugaacgacaaggccgcgcugcugaucaucgaccuggagaccggggccaucacccgcaaacuggaagucaccggcaggaccggcguacccaacggccuauccagcccucgccuggcagacaacaacagcgacggcguagccgacuacgccuacgccggcgaccugcaaggcaaccucuggcgcuucgaccugaucgccggcaaggucaaccaggacgauccguucagccgagccaacgacggcccggcgguggccucgagcuucagggugucuuucgguggccagccgcucuauucggcagucgacuccgccggcgcggcgcaagcgaucaccgccgcgcccucgcugguucgccauccgacacgcaagggcuacaucgugaucuucgguaccggcaaguauuucgagaacgccgacgcccgggccgauaccagccgcgcccagacgcucuacggcaucugggaccagcaaaccaagggcgaagccgcgggcagcacaccccgacugacgcgcggcaaccugcagcagcagacccuggaccuccaggccgacucgaccuucgccucgaccgcucgcaccauucgcaucgccagucagaacccggucaacuggcugaacaaugacggcagcaccaagcaguccggcugguaucuggacuucauggucaacggcacccugaagggcgagaugcugaucgaggacaugaucgccaucggccagguggugcugcugcaaaccaucaccccgaacgaugaccccugugccgacggcgccagcaacuggaccuauggccucgaucccuauaccggcggucgcaccagcuucaccguguucgaccuggcacgccagggcgucguggacucgaaauccgacuacagcuacaacaagcagaacgucgcgguauccgguaccgagcagaaaggccugggaggcuugacgcugagcaccaacgaacagggcaauccggaagucugcuccucgggcgaaugccugaccgugaaccccgguccgaacacccguggccgccagaacuggcgccccaucgaaggaaagaacuga

SEQ ID NO: 87 - RNA, 3636 nt, Pseudomonas aeruginosa
augaagauucucgccauccgccugaagaaccucgccucccucgcuggcgagcaggaaaucgacuucacccgcgaaccgcuguccagcgccggccuguucgccaucaccgguccgaccggcgccggcaagagcaccgugcuggacgcccugugccuggcccuguucggcagcacgccgcggcuggaaagcacuucggccagcagcaagguucccgauggccggaacgagcuguccagcaacgacgaacgcaaccugcugcgccgcgguugcgccagcggcuacgccgaaguggauuucgucggcaucgacggccaccgcuaucgcgcccgcugggaaacccggcgcucccgggacaaggcggacggcgccuugcaaaagagccagcagagccuccaggaccuggagacccagcaaaugcuggcagcgaacaagaaaagcgaguuccgcgaacagcuggagcagaagcucggccucaauuucgcccaguucacucgcgccgugcugcuggcccagagcgaauucagcgccuuccucaaggccagcgacaacgaccgcggcgcauugcuggagaaacucaccgacaccggccuguacagccaauugagcaaagccgccuaucagcgcgccagccaggccgacgagcagcgcaagcaacucgagcaacgccuggaaggcagccugccccuggccgagcaggcccgggccgggcucgaggcggcgcuggaaucccacgcccaggcgcgucuccaggagcaacaggcacugcaacgucuggaaggccagcaacaaugguucaccgaggagcagcggcugcugcaauccugcgagcacgcacaaggccaacuggccgaggccaggcaggccugggacgcccuggcgacggagcgggaaacccugcaauggcuggagcgccuggcuccgguucgcggacugaucgaacgccugaagcaacucgagcaggaacuccggcacuccgagcagcagcagcggcagcgcaccgagcagcaagccgcgggcaccgagcgcuugcaaggauugcaggcccgcuugcaggaggcgcgcgagcgccaggcccaggccgacaaccaucugcgucaggcccaggcgccguugcgcgaggcuuuccagcuggagagcgaggccaggcgccuggagcgaacgcuggccgagcgacaggaacuccaucggcaaucgaaccagcgccacgcccagcaaagcgacgccgcucggcaacuggauauggagcagcagcgccaugucgcggaacaggcgcaacugcaggcggcauugcgcgacagccaggcucucgccgcgcucggcgacgccugggugacccaccagggccagcucgccaccuucgugcaacgucgccagcgcgcgcucgaaagccaggcgcagcuccccgagcuggaaaaaucccuggcccacgccggggaaccgcucgaacgcuugcaggcgcaauggaccgcccuccauggcagcgagccggacgaccuggcggcacgccuggucgaauugcgccggcagaccgauagccuggaacgacaacaagcgcuccacaaggaauggcaacagguccucgaccaacgcgccggucuggcucgacgccugggcgaacucgaccagcguauggucgagcaggagcaggcauugcucgaccugaaacgacaaggcagccaaugcgccgaggaggugaaggcggcggagcaggcccugcaggucacccgcgaguugcuccagcgccaacgucuggcccgcagcgccagcgucgagcaacugcgcgccggccugguggacggcgaggccugcccggucugcggcagccaggagcaucccuaucaccauuccgagcaacugcucgccgcccucggugaacacgacgaccaggagcagguccgcgccgagcagucccucgagcggcugcgacagacccuggucggucugcgcgagggcuauuccagccagcgggaaagacucaaccagagucgccaggagcagcaggaacugacuggccaacuggccgcgcucgaucggcaacuggaccaauggacgcugccggaagaacugcgacuccugcagccguccgcgcaguuggaguggcuggcacaacgccuggacgaccuggcagggcagcgccagcagugccaacgagacuucgaccggcugaucgcccgccagcgccagacccagcaauugcagcaggaacugcgggccgccgagacgauccugcaacagcgccagcaggcgcugacggaacaacggcagcgcuacgaacauuugcagcagcaggucgaggaggacagccagcaauugcguccauugcucuccgacgagcacuggcagcgcuggcaggcagauccgcugcggacuuuccaggcacucggcgaguccaucgagcaacgccggcagcaacaggcgcggcuucagcagaucgaacagcgucugcaggagcucaagcagcgcugcgaugaaucgagcuggcaacugaagcaaagcgacgagcaacgcaacgaagcccgucaggcagaggaaagggcccaggcggaacucgccgaacugaacggacgccucggcgcucaccugggccagcacgccugcgcccaggacuggcagcuaucgcuggagcacgccgcgcaagcggcgcagagcgccgucgagacgcuccaggcgccccuggauucgcugcgcgaggaacaacugcgacucgccgaagcccuggaacaccugcagcagcaacggcagcgccaacaggaugaguuccagcgccuucaggccgacuggcaggccuggcgcgaacgccaggacaaccucgacgacagccgccucgacgcccugcucggccuuuccgaggaacaggcgacgcaauggcgggagcaauugcagcgacugcaagaggagaucacccgccagcagacacuggaagcagagcgccaggcgcaacugcuccagcaucgccggcagcggccggaaaccgaccgcgaggcgcuggaagacaaccugcggcaacagcgcgaacgccuggccgccagcgaacaggccuaccuggagaccuacagccaguugcaggccgacaaccagcgccgcgagcagagccaggcgcugcuugccgaacuggagcgagcccgcgccgaguuccgcagauggggccgccugaacgaacugaucgguucguccagcggcgacaaguuccgccgcaucgcccagggcuacaaccucgaccugcuggugcagcacagcaacgugcaguugcgccaguuggcgcggcgcuaccgccugcagcgcggcggcagcgaacugggccugcuggugguggacaccgagaugggcgacgaacugcgcucgguguauucgcucuccggcggcgagaccuuccugauuucccuggcccuggcgcucggccuggccucgauggcaucgagcaagcugcgcaucgagucgcuguucaucgacgaaggcuucggcagccucgacccggaaucccugcaacuggcgauggaugcccuggacaaccugcaggcccagggacgcaagguggcggugauuucccacguccaggaaaugcacgaacggaucccgguccaggugcggguccagcgcgagggcaacggcaugagcagccugaagguggucggcuga

SEQ ID NO: 88 - RNA, 7407 nt, Pseudomonas aeruginosa
augucgauccaggcgaaaguuaccccuaucgaucagaguauuucuucugcggcugccgucgagguuccggaaaacgggauacucaaacucucccagagcaguaaugucgcgcucgaugucgcaccggagucgguggcgggauacucgaagagcgguucggaccugaucguccagcugaagaccggggaaagcguccggaucgccaacuucuaugcggaaggccagccuuccagccaacuguuccuggccgacaaggacaagcugguggcgguagaucugccgccggucgcugccgacgggccgcugauggccggcuacaucccgcaggaaagccuggccgguuucgagucgcugaccggcgccggugugcucgguggcaugagcgcagggacugcgcugcuggucggugcggcggccaucggcgccgggguggcgauuuccaacagcagcggcggcgguggcggcggcgguucuucggugcccccggacaccacuccgccgaaggcggccagcggccugaagauagcgccugacggcagcagcaucagcggccaggccgaggccggcgcgagcgucggcaucgauaccaauggcgacggcaagccggaccucaccgugaucgccgaugccaacggcaauuucaccgcuccgcugaacccgccgcugaccaauggccagacggucaccgugguggucaccgacccggcuggcaacgccagcccgccggcccaggucaccgcuccggacacuaccgccccggcgccggcuaccgacgugcagguggcgccggacggcagcagcgucaccggcaaggccgaacccggcucgacggugggcgucgauaccgacggcgacggccagccggacaccaccgugguggucggccccggcggcagcuucgagguuccgcugaacccgccgcugaccaauggcgagacggugacggugaucguuaccgacccggccggcaacaacagcaccccggugaccgucgaggcgccggacaccaccgccccggcgccggccaccgacgugcagguggcgccggacggcagcagcgucaccggcaacgcagagccgggcgccaccgucggugucgacaccgauggcgacggccagccggacaccaccgugguggucggucccggcggcagcuucgagguuccgcugaacccgccgcugaccaauggcgagacggugacggugaucguuaccgacccggccggcaacagcagcaccccggucaccgccgaagcccccgacuuccccgacgcgccccaggucaaugccagcaacggcagcguccucagugguacggcggaagcgggcgugaccaucgugaucaccgacggcaacggcaauccgaucggccagaccagcgccgaugccaacggcaacuggagcuucacccccgguagccaacugccggauggcaccguggucaaugugguggccagggacgccgccggcaacagcagcccggcgaccuccaucaccgucgacggcguggcgccgaacgcgccgguggucgagccgagcaacggcagcgaacucagcgggacugccgaaccgggcagcagcgugacccugaccgacggcaauggcaauccgaucggccagaccaccgccgaugccaacggcaacuggucuuucacgccguccaccccguugccggacgguaccguggucaacgugguggccagggaugccgccggcaacagcaguccgccggccagcguuaccguggaugccgucgcgccggccacgcccaccgucgauccgagcaacgguacgacccucagcggcaccgccgagccgggcaguagcgugacccugaccgacggcaacgguaacccgauagggcaggucaccgccgacggcagcggcaacuggaccuucaccccgagcacgccguugcccaacggcacgguggucaacgccacggcuaccgacccguccggcaacgccaguucgccggccagcgucaccguggacgccguggcaccggccacgccaguggucaacccgagcaacggcaccacgcucagcggcaccgccgagccgggcgccaccgugacccugaccgauggcaacggcaaucccaucgggcaggucaccgccgauggcagcggcaacuggagcuucacuccgaccacgccguugcccaacggcaccguggucaacgccacggccaccgacgccuccggcaacaccagugcgggcagcagugucaccguggacucgguagccccggccacgccagugaucaaccccagcaacggcaccacgcucagcggcaccgccgagccgggcagcagcgugacucugaccgauggcaacggcaacccgauuggccaggucaccgccgacggcagcggcaacuggagcuucaccccguccacgccgcuggcggauggaaccguggucaacgccacggccaccgauccggcgggcaacaccagcggccagggcagcaccaccgucgauggcguggcgccgaccacgccgaccgucaaccugagcaacggcagcagccucagcggcacugcggaaccgggcagcacggugauccucaccgacggcaacggcaauccgaucgccgaggucaccgccgacggcagcggcaacuggaccuacaccccguccacgccgaucgccaacggcaccguggucaacgugguggcccaggacgccgccggcaauagcagcccgggcgccagcgucaccguggacucgcaggccccggcggcuccgguggucaacccgagcaacggcacuacgcucagcggcaccgccgagccgggcgcuaccgugacccugaccgacggcaacggcaacccgauuggccaggucaccgccgacggcagcggcaacuggagcuucacaccgggcacgccgcuggccaacggcaccguggucaacgccacggccagcgacccgaccggcaauaccagcgcuccggccagcaccaccguggacucgguggcgccggccgcgccgguggucaauccgagcaacggcgcggagaucagcggcaccgccgaaccgggcgccaccgugacccugaccgauggcagcggcaauccgaucgggcaggucaccgccgacggcagcggcaacuggagcuucaccccguccacgccgcuggcggauggaaccguggucaacgccaccgcuaccgacccggccggcaauaccggcggccagggcagcaccaccguggacgccaucgcgccggccacgccgaccgucaaccugagcaauggcagcagccucagcggcaccgccgagccgggcagcacggugauucucaccgacggcaacggcaauccgaucgccgaggucaccgccgacggcagcggcaacuggaccuacaccccguccacgccgaucgccaacgguacuguggucaacgugguggcccaggacgccuccgguaacagcagcccgccggcgacggugaccgucgauuccagcgcgccgccggcgccggugaucaacccgagcaacggcgucgucaucagcggcaccgccgaggccggugccacggugacccucaccgaugccggcggcaacccgauagggcaggucaccgccgacggcagcggcaacuggagcuucacgccgggcaccccgcuggccaacggcacggugaucgucgccacggccaccgacccgaccggcaauaccggcccgcaggccgccaccacgguggacgcgguggcgccgccggcgccggugaucgauccgagcaacggcacgaccaucagcggcaccgcggaggccggggccaaggugauccucaccgacggcaacggcaacccgaucggcgaaaccaccgccgacggcagcggcaacuggagcuucacgcccggcacgccgcuggccaacggcacgguggucaacgccguggcccaggacccugcgggcaauaccggcccgcagggcagcacuaccguggacgcgguggcgccgaacacgccuguggucaauccgagcaacggcaaccugcucaacgguaccgccgagccgggcagcaccgugaccuugaccgacggcaacggcaacccgaucggccagaccaccgccgauggcagcggcaacuggagcuucacgcccggcucgcaacugcccaacggcaccguggucaacgugaccgcgagcgacgccgccggcaauaccagccuucccgcuaccacgacgguggauuccucgcugccgucgaucccgcagguggauccgagcaacgguucggugaucagcggcaccgcggacgccggcaacaccaucaucaucaccgauggcaacggcaacccgauuggccaggucaccgccgacggcagcggcaacugguccuucacuccaggcaucccgcugccggauggcacgguggucaacgugguggcgcgcagcccaagcaaugucgacagugcgccggcggugaucacuguggauggcguggccccggcggcgccggugaucgauccgagcaacggcaccgagauaagcgguaccgcggaggccggcgcgacggugauccucaccgauggcggcggcaacccgaucggccaggccaccgccgacggcagcggcaacuggacguucaccccgagcaccccgcuggccaacggcaccgugaucaacgccguggcccaggacccggccggcaauaccagcgguccggccagcgucaccgucgaugccaucgccccgccggcgccggugaucaauccgagcaauggagucgucaucagcgguacggcggaagccggggccacggugauccucaccgacggcaacggcaacccgaucggccaggucaccgccgacggcagcggcaacuggagcuucacgcccggcacgccgcuggccaacggcucggugaucaaugcgcuggcccaggacgccgccggcaacaacagcagucccaccagcgccaccgucgacucgcuggcgccagcagccccggugaucgauccgagcaacgguagcgugaucgccgguaccgccgaggcuggugccacggugauccucaccgacggcaacggcaacccgaucggccaggucaccgccgauggcagcggcaacuggagcuucacgcccggcacgccgcuguccaauggcacgguggucaaugcgguggcccaggacgcugccggcaacaccagcggcccggucagcaccacgguggacgcgguggccccggccaccccggugaucgacccgagcaacggugucgaacucagcggcaccgccgaacccggcguccgggugauccucaccgauggcaauggcaauccgaucggccagacccuugccgacggcagcggcaacuggagcuucacgccgggcacgccgcuggccaacggcacgguggucaaugccguggcccaggacccggccggcaauaccagcggcccggccagcaccacgguggacacgguggcuccggccacgccggugaucaaucccagcaacggcagcgugaucaccggcaccgccgaggucggcgccaaggugauccucaccgauggcaacggcaacccgaucggcgagaccaccgccgacggcagugguaacuggaccuucacccccggcacgccgcuggccaacgguacggugaucaacgccgucgccgaggacgccgcgggcaacgccagcgguccggccagcaccacgguggacucgguggcgccguccgcuccgcugcugagcaucagcgccgacggcgcgcugcugaccggcaccgccgagccgaacagccaggugcgcaucguggucaacggcgacaccgccaacccgaucacggucaccgucgacggcgccggcaacuucagccugccguucgcgccgccgcugaucaccggcgagcugaucgccggggucgccgucgacgccgccggcaacgucagcgggccggccaccaucaacgccccggaccuggcgccgccgaccaucagcgugccggaagccgccgauaccuggaucaaugccgcggagaucggcgacgguauccaggucgaugugacgguccguccgaccaugcaggucggccagguggucacggucaaguucgccgggcagaacggcuacgaggccgaggucagccauacccucaccgccggcgacaucgccgccggcaaccugacccugacccugacgccucccggcggcaugggcccguucccggagggugccucgaccgucaccgccgacaucaacggcggcaccgcgucgaccccggugccguucaccaucgacaccauuccgccggcgaccccggugcugucccuggucggcaacauccugaccaucucggcggagccagggaccgaguugacggugaccgucgacgucggcggggugaccgccaccgccacggugaccgccgacaacagcgggcuggcgucgcugaaccugcucaccgaccuggacaucgacuucaguugggaccaguugcucaaugcccaggugucgguggucggacgcgacccggccggcaacccgagcaacacggcgagcaucggcgucggcaccagcaucgagcaaccggugaccaucggcaacuucggccucgacgucagccucaacccgcugaacccgcguuucgguuucagcggaaccaccgagccugacuccagcguggugauccgggucaucaccccggcguugaacgucgaauugcugccgauccaggcggauucguccggaaacuucucgcugaaccugcugagcccgaccauccucacccaguuggggcugaacaucaccgacauccucaaccucggcucgcagaucucguucaaccugguguccaccgacuccaauggcaacgacagcgccgccuacgggaucacccugacccccaacggacugucgcucaauaucggccagaucgaugucaacgguacuuccggcgacgacgugcuguccggcgccaacggcaguucggagcacaucaacggcggcgacggcagcgaccugaucuucaacgugggcaccggcgaucacgugguggccggcaacggcaacgacaccauccagaucaccgcgaccgauuucgucagcaucgauggcggcgccggguucgacacccugguccuggccaacggcaucgaccucgacuacaacgccgucggcgucggcacgcucagcaaccucgagcgcaucgaccucggcaagggcgauucggguagcgugcugacccugaccgcggcggagguggaugccaucaccgaugccaacaacacguugcagaucaccggcgagaacaacgacacccugaacguggugggcgcggugaauaccgguaccacgcaacugaucaacggcauuaccuacgacgucuacaccuucggcaguaccacccugcugaucgaggacaacacgguacaggucguggucuga

SEQ ID NO: 89 - RNA, 10608 nt, Pseudomonas aeruginosa
auggacauccgcagcccgcugaaccagugcaucgcccugucccuggccggcaucuuguuccucaacccgaucgucgccgcggcggcggggcuggcgcuggacaaggccgccggcggcaacaccggccugggccaggcgggcaacggcgugcccaucgucaauaucgccacgcccaacgacgccgggcugucgaacaaccauuuccgcgacuacaacgucggcgccaacgggcugauccucaacaacgcuaccggcaagacccaggguacccagcucggcgggaucauccucggcaaccccaaccucaagggccaggcggcgcaggugauccucaaccaggucaccggcggcaaccgcagcacccuggccggcuacaccgagguggccgggcagucggcgcgggugaucgucgccaacccgcacggcaucaccugccagggcugcggcuucaucaacacgccgcgcgcgacccucaccaccggcaagccgaucauggacggccagcgccuggagcgcuuccagguggacggcggcgacaucgucgucgaaggcgccgaacugaacgucggcaaccucgaacaguucgaccugaucacccgcagcgccaagcucaacgccaagcucuacgcgaagaaccucaacaucgucaccggccgcaacgacguccaggccgacagccugcaggccacgccgcgcgccgccgauggcagcgagaagccgcagcuggcgaucgacagcucggcgcugggcgggauguacgccggggcgauccgccuggucggcaccgagcagggcgugggggugcggcuggccggcgacauggccgccagcggcggcgacauccgcaucgacgccagcggcaagcugagucuggcccaggccuccagccagggcgaccugaagaucgcggcccaggccguggagcugaauggcaagaccuacgccggcggcagcgccgagauccgcagcgcggaggaacuggucaaccggcagagccuggcggcgcgcgaacgcaucgugcuggaggcggcgcauaucgacaacgccggggugaucgaagccggcgucgagccagacgagcgacgcaacgcgcgcggcgaccucgagcugcgcagcggcacccugcgcaacgccggcagccugguggccagccgcgcgcuggaagcgaaggcgagccaggcgcuggacaaccagggcggcagccugaagggggcgaccguccgggucgacgccgggcaccuggacaaccguggcggcaagcugcucgccgagggcgaacugcgggucgaggcgagcagccuggacaaccgccaggacggccuguugcagagccgggaccgcgccguggucaagacccguggcgaucucgacaaccguggcggccaggugaucggccugaacgaucuggaggucggcgcggcgacgcucgacaacggccagcaaggccugcucggcagccagcaguccacccgcgucagcgcccaggcgcuggucaaccggggggacggcgaagucuccggcaagcgcgucgaggcucgcgucgguagccucgacaaucgcggcggcaagcugaucggcgacgaccugcugguggucgccagcggugccaucgacaaccgccucggcuuguucuccgcagccaaccgccucgaccugcgggcgcgcagccuggacaacagcggcaagggcacgcugagcagccggggcggccuggaggucagccucggcggccugcuggacaaccgcgaugaaggcaaccugcucagccagggcgcgcagcgcgugacgguggggcaacuggacaaccgcgccggcggccugcugucgagccgcagcgaguugaacguccacggcgccagccuggacaaccguggcggcgugcugguggccgacgccggccugagcgccacgggaggcgccuucgacaaccgcgacggcggcagcgccagcggcaaggcuggcgugcgcguggaggucgccagccugcgcaacgaccaggguggcaagcugcucagcgauggccgccuggaccucgcagcgaacgccgucggcaacgccggagggcguaucgccgccaagggcgaccugcaggcgacgcuuggcagccuggcccagcaagguggcgaacuggucagcgaaaagacccugaaggucgcggccgacacgcucgacaacagccaguccgggcugaucgccgcgaauggcggcaucgcuaucgaggcgcggcaggucgacaaccgcgccggcgagauuuccagcaccucgaaggucgccgugaacgcccgcgagcaacuggacaaccgcggcggcaaggucaucggcgacagcggccugcgccucaccgugcagcgccugcugaaccaggccaagggggugcuggccgggcgcgacggccugagccuggacggcggcgaacuguucaacggcgacggcggucggcucgacagccagaacagccugagcgugagccucggcggcgugcuggacaaccagggcggcgcgcuggucagcgaaggcagccugacggcgcgcgccgcgcgccuggacaaccguggcgggaccuucuccagcgccggugcgcuggcgcugaccagccaggccgcgcuggacaaccagggcggcaggcugcucagcgaugccggcgugacgcugcagggcgccagccucgacaacagccguuccggcgugaucagcgccaagggcgcgguggauauccgcaccggcguacuggacaacagccgcaacggcggcaucggcagcaacgccggcaucacccugguggccgcccggcuggacaacggccagcagggccgggucagcgccaagggccugcucgacgccaaccugaaaggccucgaccagcgcggaggcggcguccugaucagcgaaaccggcgucacccucgaccucaauggcggcacgcuggucaaccgcgacggcggccugaucgccacgcccggcgcgcugcugcugcgccagcucggcgcgguggacaacggcgccggcggggaaaucuccagcgaccgcgccuucacccucgccgccgccagccuggacaaccgcggcgggcgccugaucggcgccgccaaccugacccugcgcaucgcccaggcccuggacaacagccuggccggggugaucuccggcgccgccggccuggacaucgcggccgcucgccuggacaacagcgccaagggcacccuggccagccgcgccggcaucgaccugcgcgucgauggcgcgcuggacaaccacgccgaaggcaccgucuccggcgcccgccugacgcucgccagcgccucgcuggacaacagcggcaagggccugcucuccggcaacgccggccugagcgucgccacuggcgcgcuggacaacgccgaggguggccaguugaucagccagggcguccuggacgucagcagcgccgaccucgacaaccguggcggcgcccucaguggcaagcagucgcugcgccugagcgccgccaaccuggacaaccguggcggccugcucaccagcgacggcgaacuggaacugacggcagggcgcgucgauuccgccgacggcggcgaaaucuccgcccggggcgaccugcgccugacggucgagcgccuggugcaacgccagggccggcuggucggcgagcgcggcgucagucucgaccugcggggcggcgaccuggacaaccagggcggccugaucagugcccgcggcccgcugagcaucgagcggcugagcguccucgacaaccgccagggcggcgagauuuccagccagcagggcuucgagcugcuggccaggcgcaucgacaacggccagcaggggcgcaucaucagcgccgggaaacugcgccuagacgccgacgcgcugggcaacgccggcgccggccugcucuccggauggcagggccugacggugacaggcgggagccuggacaacagcgccggcggcacccuuucgagcaaggacggcgagcuggccaucagccucggcggcgcgcuggacaaccacggccagggcgcgcuggucagcaagggcgcgcaacggaucgacgccgccagccuggauaacgcccagggcauugucuccggcgaaagcgacgugacccugagcaucgccgggaagcuggacaacggccagggcggccuggucucggcgcagcgcgcgcugagcuucgagcgcgacgauacgcugcugaacaacgccggcggccggaucaacggcggcagccugcugcucaagggcgccagccuggauaacagcgacggccaguugaucagccagggccggcucgacgccauccucggcggcgcccuggucaacaccggcgcggcgcgccuggccagcggcggcgaccugcugcugcgcagcgccagcgucgacaaccgcggcggcaagcuggucagccaggggcugcuggagaucagcgccggcagccucgacaacagcgccuccggcacccucgccagccaggccggcaugagccugcgccugggcggcggcgcccugcgcaaccagcaggacggccugaucuucagccaggccggcgcccucgaugugcaggccggcagccuggacaaccgccagggcacgcuccaggcccagggcgacaaccggcugcguaucggcggcgcgcuggacaaccagggcggccgccuggacagccgggccggcaaccucgaccugcagagcggcagccucgacaacggcgccggcggcgugcucaacagcgccaaggguuggcugaagcuggucaccgggcuguucgacaacagcgccggcgucacccaggcgcagucgcuggagauucgcgccgggcaaggcgugcgcaaccagcagggccaccucucggcgcugggcggcgacaaccgcaucgucaccgccgacuucgacaaccagggcggcggccucuacgccagcggccugcucagccucgacggccagcgcuuccucaaccagggcgcggcggcgggccagggcggcaaggucggcgccgggcgcaucgacuucagccuggccggcgcgcuggccaaccgcuucggccaguuggaaagcgaaagcgagcugcaccugcgcgccgccgcgaucgacaacagcggcggcagccugcgcgcccucggccgcagcggcagcacgcgguuggucgcuggcggccugaacaacgccuacggcgugcuggaaagcgccaaccaggaccucgaccugcaacugggcagccuggccaacgccggugggcgcauccuccacaccggcaauggcaccuucggccuggauuccgggcaggugauccgcgccggcggcgaacugaccaccaauggccugcuggacauccgcgccagcgaauggaccaacagcagcgugcugcaagccggacgccugaaccuggacaucggcaccuuccgccagacggccgagggcaagcuguuggcggugcaguccuucacuggccgcggcggcgacuggagcaacgacggccugcuggccagcgacggcagcuuccgccucgaccugagcggcggcuaccguggcaacggccgcgccaccagccucggcgacuucgcccugaacgccgccagccucgaccucggcaacgccgccagccucgccggcggugccaaugucacgcucggcgccggcaaccugcuggucaaccgugggcggaucaccgccgccggcgaccucguggccagcgccgcgagccugaacaacuacggcacccugggcggcggcggcaaccugcgauugaacgcgcccgcccugcucaacgagcgcggguugcuguucaguggcgccgacaugacccugcgcgccggcgacaucaccaaccucuacggggauguguacagccucggcaggcuggauaucgcccgcgacgaugcgggcaaccgugccgccagccugcgcaaccuuuccggggugaucgagagcggcaaggacuucagccugcgugccagccugaucgagaaccgucgcgccgugcuggaaagcaagucgggccuguacaccgcgaagauggagcagaccgccugcaucgaaggcgucaacgcgggcgacugcagcggcaagcgcaacgccaucuggaccaucacccagcgcgacaagaccgaggucaccgccagcagcgccauggggcaacugcuggccggaggcgacuucgccaucgacggcggcacccugaacaaccuuuccagucugaucggcagcggcggcaaccucaccgccaaccucgaaguccucgacaaccagggccuggaaaccggcgagcuggaaaccauccgcgugcugcguaccgcucgcggcggcgauaucggcggcaucgaccagaagucgcgcaacuucaccaaccucuacugguaccagagcgccaauuucgacccggcgcgcgcgggcgagauccccgccgcgcucaacgcgauccucagcgacugguccuucgaguacgaauucccgagcaaggggccgaccccgaucagcaguggcgaccaguccuacgcagcggugauccaggccgccggcgacgucacggucaaugccagcacgcgcaucgacaacggcgucacccgccccggcuacaccuucgucggcagcggccgccaggugggcgacagcgcggugggcggcagcgggguuucgguggucgugccgcugaccucgcaacugccgcccgaccuggcgcggcgccaggucaacccgguuacccugcccggcuucagccugccccagggugacaacggccuguuccgucucagcucgcgcuuugccgaggacggcaauggcagcgccgcgcucggugccggcgccgaccgcacccagggcgguagcggcgucucggucggccagcaaggcgccggcaacgccgccgguaccuggcagggccagggcgugcgagucgacggccuggcuggcgcggccaacguccagggucagggcggcagcacgcucggcgguagccugccgggcgucgcccggguccagggcgugcccggcaacgccacgccgagcgccagccacaaguaccugaucgagaccaacccggcgcucaccgaacugaagcaguuccucaacucggacuaccugcucagcggccugggcaugaacccggacgauagcaagaagcgucucggcgacggucucuacgagcagcggcugauccgcgacgcggugguggcgcgcaccggccagcgcuacaucgacgggcugagcagcgacgaggcgcuguuccgcuaccugauggacaacgccaucgcuuacaaggaccaacugcaccugcaacugggugugggccugagcgcggagcagauggcggcgcugacccacgacaucgucuggcuggaagaggucgaggugaacggcgagaagguccucgcgccgguggucuaccuggcccaggcggagggucggcuggcacccaacggugcgcugauccagggccgcgacgugaagcuggugagcggcggcgaccugcauaacgucggcacccugcgcgcgcggaacgaccucucggcgacggccgacaaccucgacaacagcggccugaucgaggccggcaagcgccucgaccugcucgccggcgacucgauccgcaaccgccagggcggggucaucgccgggcgugacgugagccucaccgcgcugaccggcgacguaaucaacgaacgcagcgugacccgcuacgacagcgcgcucgacggccgcaccugggaacgcagcuucgccgacagcgccgcgcggguggaggcggcgaacagccugaacguccaggccggacgcgacaucgccaaccucggcggggugcugcagagccgcggcgaccucagccucgacgccggacgcgacgucaccgucgccgccgucgaggaccgccagggccagacccgcuggagcacgucgcggcuccagagcgugacccagcucggcgccgaagucagcgccgggcgggaccugaacgucagcgccggccgcgacuugacggcgguggccagcacccucgaagcgcgccgcgacaucgcccucuccgccgggcgcgacgugacccuggcggcggcggcgaacgaggagcaugccuacagcaagaccaggaaggucaccuaccaggaagacaaggucgcccagcaaggcacccgcguggacgccggcggcgaccuggcgaucaaugccggacaggaccugcgccugaucgcgagccaggccagcgccggcgacgaggccuaccugguggccggcgacaagcuggaacugcuggccgccaacgacagcaacuacuaccuguacgacaagaagaagaaaggcgacuucggccgcaaggaaacccggcgcgacgaagucaccgacgucaaggcggugggcagccagaucagcagcggcggcgaccucacccugcucagcggcggcgaccagaccuaccagggcgcgaagcuggaaucgggcaacgaccuggccaucgucagcggcggcgcggugaccuucgaggcggugaaggaccugcaccaggaaagccacgagaagagcaagggcgaccuggcguggaacagcgccaaggggaaagggcagaccgaugaaacgcuucggcagacccagaucguggcccaggggaaucuggcgaucaaggccguggaagggcugaagaucgaccucaagcauaucgaccagaagaccguaagccagaccaucgacgcgauggugcaggcggauccgcaacuggcguggcugaaggaggccgagcagcgcggggauguggacuggcgcauggugcaggaggugcacgauagcuggaaguacagcaacucgggcauggggccggcgacgcagaucgcugucgccaucgcggcggcagccaucgguggcauggcggcagcgggagcgcucaguggugcaggagugggugccaguagcuucgccaugggcgcaggaguuggugcggcaggaagccugucgggcacggcagcggucagccugaucaacaacaagggcgaucucgggaaggugcugaaagacagcuucaguagugacagucugaagcagauugcuauugcgagccugaccggggggcugacggcugaguacuucgacgggauucuucagaccaagacugauccgcuuacuggaaaggucacgguagaccucagcagccuaucugguguuggucgcuucgcugccaaucaggcgaugcagaacgcuacauccacuguacugagccaggccuugggccagggcgggagccugaacgaggcgcugaagagcgcgcucuacaacaguuucgcggcggcagguuucaacuucgucggcgauaucggccaggaauacagccugaagccaggcgauccuucgauggugaccaugcacgcccugauggguggccuggcggcgcaggucagcgguggcgauuucgccacgggcgccgcggcggcuggcgccaaugaagcgcugguggccaagcuagaccaggccuucaagagcuugagcccugagaaccgugaagccauggucacuauggggucgcaauugguugguguucuggcugcggcgguacgcgauccugaugugacaggcaaagcucuggaaagcgcugcuuggguagcgaagaacucgacgcaauacaacuuccucaaccaucaggauguggccgaucuggauaaugccuugcagaaaugcaagucccagggaaauugccgucagguagaggaagaguucaaggcgcguagcgacgagaaccggcggagguugaauggcugcguggcuguggguaauugcgcggagauucgugcggagaucgaugcggggucuacggcucucaacgagcugguggcccggcaggaaacagcuaauccgggaggaagugacagcgauauagccuacgguuuccugaugggccgaaauguugucgacuggacgacggcuggucaguugcaccuggagcagaccgccaaccucugguggaacgguaauccacaguggcagaaggaagucggugcauaccuagaccagacgggguucaauccguucggaaucggcguuccggcaaugggcggugccgcuggcaagguaacggccaaggcgcucaugaaugcgcugaaggcgggagaguugcccaaaggagagguggccccaggaaaggcuaaucugccuaccauuggggcguuggcggaugcugaggcgggaaugccuuauacccauccaguuaagcucgccgcaaaagcgacugggacagcagggaagauuaagauugaagccggcgcaauaccugacgcaaaugaaguacgugcaggacaaggguuaucuggucuuggguacgauguuacgcaccaaaccacugcgucagcuaaagguauucaagggcagcgaacugcggacuugcauguugauggacucgguuccauugauguguauacgccgaagaaucuugauccgacaaagauaguucgagcgauagagaagaagucgaaucaagccggcggagucuuggugcaggcggacuugccaagcacugacaugucguccauugcugcucguaugugggggaagacuaacgcgcagaguauaaaaacuauauuuuuccagaaaccagacggaucauugguccgauuugaucgaccugcuggaggaggcuga

SEQ ID NO: 90 - RNA, 16884 nt, Pseudomonas aeruginosa
auggacauccgcagcccgcugaaccagugcaucgcccugucccuggccggcauccuguuccucaacccgaucgucgccgcggcggcggggcuggcgcuggacaaggccgccggcggcaacaccggccugggccaggcgggcaacggcgugcccaucgucaauaucgccacgcccaacggcgccgggcugucgaacaaccauuuccgcgacuacaacgucggcgccaacgggcugauccucaacaacgccaccggcaagacccaggguacccagcucggcgggaucauccucggcaaccccaaccucaagggccaggcggcgcaggugauccucaaccaggucaccggcggcaaccgcagcacccuggccggcuacaccgagguggccgggcagucggcgcgggugaucgucgccaacccgcacggcaucaccugccagggcugcggcuucaucaacacgccgcgcgcgacccucaccaccggcaagccgaucauggacggccagcgccuggagcgcuuccagguggacggcggcgacaucgucgucgaaggcgccgaacugaacgucggcaaccucgaacaguucgaccugaucacccgcagcgccaagcucaacgccaagcucuacgcgaagaaccucaacaucgucaccggccgcaacgacguccaggccgacagccugcaggccacgccgcgcgccgccgauggcagcgagaagccacaacuggcgaucgacagcucggcgcugggcgggauguacgccggggcgauccgccuggucggcaccgagcagggcgugggggugaagcuggccggcgacauggccgccagcggcggcgacauccgcaucgacgccagcggcaagcugagccuggcccaggccuccagccagggcgaccugaagaucgcggcccaggccguggagcugaacggcaagaccuacgccggcggcagcgccgagauucgcagcgcggaggaacuggucaaccggcagagccuggcggcgcgcgaacgcaucgcgcuggaggcggcgcauaucgacaacgccggggugaucgaagccggcgucgagccagacgagcgacgcaacgcgcguggcgaccucgagcugcgcagcggcacccugcgcaacgccggcagccugguggccagccgcgcgcuggaagcgaaggcgagccaggcgcuggacaaccagggcggcagccugaagggggcgaccguccgggucgacggcggacaccuggacaaccguggcggcaagcugcucgccgagggcgaacugcgggucgaggcgagcagccuggacaaccgccaggacggccuguugcagagccgggaccgcgccguggucaagacccguggcgaucucgacaaccguggcggccaggucgucggucugaacgaacugcagguccaggcugccgcacuggacaaucgcagugccggucuccuuuccagcaagggagacauggacaucgaguucgcucgucuggacaacagugcgggcggcaagcuggucagcgagcgccguacgcuccugaaggcggaucggcucgauaaucgcagcggucgcauugucgccggccaggaucucgacuugagcucucgguugaucgacaaccgagcgggcgauaucuccagcacgucgagggugguggcgagcgcucgcgaacaguuggacaaccgcgguggcaagaucgucggugacaguggccuggacaucacaacgccacgcaugcucaaccaggacaaggggguacucgccagccgcgaugggcugcgccugagugcuacggaguuguucaacggcgcggggggccugcuguccagccagaaggguaucgacgucucccuggccggugcguucgauaaccaggccggcagccuggacagccggggcuuccugacggugaagucagccuggcucgacaaccagggcgguacgcuauccagcgcaggggcauuggcagugaccagccagggcgcccugaacaaucagggcggcagacuggcgagcgacgccggacuuagcuugagcagcgccagccucgacaacagccaggccggugcgaucaguggcaagggggccguggagauucguaccggcaaccugaacaacagccggaaagccaguaucggcagcgaugcgggacucacccuggucgccgcucggguagacaacagccaggcgggccggaucgccgccaagggugugaucgaugcggaucuccaagggcuggaccagcaugacaggggcaaccuggucagcgauaccggcaucacgcucgaucugaacaagggaagccuggucaaucgcgcucaaggccugaucgccacgccuggcaccuugcuccugcgccaacucggcgugguggacaacagcgguggggaaaucuccagcgaccgcgcguucacucuugccaccuccgcguugaacaaccaggggggacgccugcucagcggcggagcccugaccuugcguaucgcgcaggcccuggacaacagccucgaggggauugucuccggugcuggaggucuggauauccaggcauucguccuggacaaccguaguggcuccaucggcagcaagggcgccaucgauaucggugugacccgccuggaaaacgacgcuggcacacugaucgcugaacgcggccugaagcugguagccgaugaggcgaacaguuccaaggggcguaucgccgccaaugguagccugcaugccaagguuggcacgcugagccagaagggaggagaacugaccagucaggacucgcugacucucgaccugggcauccuaaacaauaacgcuggccguaucgcuggcaaccagggcguggacaucacggcccggcagguggacaacagcgucggcgagauugccagccagggcgugguggcgcugaaccucacugagcagcuggacaaccguggcggcaagaucgucggugacaguggucugggcaucaccgcgccgcacgugcucaaccaggacaaggggguacucgccagccgcgaugggcugcgccugagugcuacggaguuguucaacggcgcggggggccugcuguccagccagaaggguaucgacgucucccuggccggugcguucgauaaccaggccggcagccuggacagccggggcuuccugacggugaagucagccuggcucgacaaccagggcgguacgcuauccagcgcaggggcauuggcagugaccagccagggcgcccugaacaaucagggcggcagacuggcgagcgacgccggacuuagcuugagcagcgccagccucgacaacagccaggccggugcgaucaguggcaagggggccguggagauucguaccggcaaccugaacaacagccggaaagccaguaucggcagcgaugcgggacucacccuggucgccgcucggguagacaacagccaggcgggccggaucgcugccaagggugcgaucgaugcggcucuccaaggguuggaccagcaugacaggggcagccuggucagcgauaccggcaucacgcucgaucugaacaagggaagccuggucaaucgcgcucaaggccugaucgccacgccuggcaccuugcuucugcgccaacucggcgugguggacaacagcgguggggaaaucuccagcgaccgcgcguucacucuugccaccuccgcguugaacaaccaggguggacgccugcucagcgguggagcccugaccuugcguaucgcgcaggcccuggacaacagccucgaggggauugucuccggcgccggaggucuggauauccaggcauucguccuggacaaccguaguggcuccaucggcagcaagggcgccaucgauaucggugugacccgccuggaaaacgacgcuggcacgcugaucgccgaacgcggccugaagcuggcggccgaugaggcgaacaacuccaaggggcguaucgucgccaaggaugaacugcgugccaaacucggugcgcuggugcagaacgggggagagcugacgacucagggcgcgcuggcccucgacgccgacaaagucgacaacggcgcuggucgcaucgccggcaaccgagguguggucaucgaugcccggcagguggacaaccgugccggcgagauugccagccagggcguggcgacgcugaaucucacugagcaacuggacaaccguggcggcaaagucguugcugacaguggucugggcaucaccgcgccacgcgugcucaaccaggacaagggaguaaucgccagccgcgaugggcugcgccugagugguaccgaauuguucaauggcaaugccggacugcucagcagucagagacauauagaggucacucuggacggcgugcuggacaaucagggcaagggcgcgcugcucagcgacgguacccugacggugagcgccgggcgcauacacaaccaggacgccacucuguccagcgccggugcgcugagacugagcagccaggaggcgguggacaaccguggcggcaaguuggugacggacuccagccugcgccugaccagcgccagccuggacaacagccgaucagggaucaucagugccaacgcugcggcggagauccauaccgggguucugaacaacagccagaaaggcaaucuuggcaguaaugacgggcucggccugauugcuacugagguggauaacagccaggaaggucggaucacugccaaaggcaugaucgacgcaaauaucaagggacucgaucagcagggcaaagggcggcuggucaguaaugccggcaucauacucgaccugaacgagggaacccuggccaauggcgcucagggccugaucgccacgccuggaaccuugcuccugcgccaacucggcaugguggacaacagcggcggggaaauuuccagcgaccgagccuucacacucaccaccuccgcgcugaccaaccaggguggccgccugcgcagcggcgguguacugacguugcgcaucgcccaggcucuggacaacagccucgaagguguucucuccggcaccggaggccuggauauccgggcgcuugcccuggacaaccgcaguggcuccaucggcagcaagggcgccgucgauaucgacgugucccguuuggaaaacgaugacggcgaccugcuuagcgaaggucgucugaaacugacugccgagcgagcgaacagugucaggggacggaucgcggccaggggugaccugcacgccagcgugacagccuuuaaccaggcggguggcgaauugagcagcgagggugcgcugaugcucgaggccgauagccucgacaaccgcagcggcggucuggucagugcugauggcaaccugaccguuuccgcccggaggaucgacaaccgugcgggcgaaaucgccagcccgggccaggugacacuggacgucgccgagcaguuggacaaccgaggcggcaaggccaucggcgauagcggacuucgccucgccgcgccacggguacucaaccaggacggcgggguacucgccagucgugaugggcugcgccugaauggcgccgaacuguucaauggcaacggcggccugcucagcagccagcaaagcaucgacgucauucuggacggcguauugggcaaucaggcaggcagcuugagcagccagggacgccugagcgugaagagcggucggcuggacaaccagggcggugcagucuccagcgccgggaccuugucgcuuuccagccagggugcguugaacaaccaggggggcaggguggucaccgacgccggugccguccugcgcagcgccagccucgacaauagccagggcggcaucgucagcgccaagggggccgcggagauccguacuggcagccucaacaauagccagaagggcggcauaggcagcggugccgggcucgcgcuggucgcggaccugguggacaacagccagaacggccggaucacugccaagggugcgaucgaugccaaccugaaggggcuggaucagcagggcagcggcaggcuggucagcgauacggccaucgcgcucgaucugcgcgggggagaacuggucaaccgugcucagggccugaucgccacgccuggagccuugcugcugcggcaacugggugucguggacaacaguggcgguggcgagaucuccagcgaucgaagcuuuacccucgccgcgaccgcgcugagcaaccgggguggccgcgugaucagcggcgacucccugacccugcgcaucgcccaggcacuggacaacagccuccaaggcguucuuuccgcaagcggagggcuggaugucgcugcacucgucuucgacaaccauagcggcaucguugcuagcaagggcgauacacacaucggggugaaccgccuggagaacgaggcaggccgcguggucagcgaaggcgcccuggaucugaccgccaagcaggugagcagcgccaaggggcgcauugccgcgaagggcgaucugcaggucacgguuggcacccuggagcagcaggguggagaacuggccagucaggggacgcugacucucgacgccgauagccuggauaaccgcaauggcggccuggugagcgccgauggcggggucaccgccgaggcacgccagaucgauaaccgcgguggggaaauauccagcguggccaagguggcucuggcuguccgggaacaacuggacaaccgggggggcaaggugaucggcgacagugagcugagccuaaccgugcagcgccugcugaaccaggccaagggugugcucgccagucgcgauggauugcaccuggacggcgcggaacugcucaauggcgauggcggccugcucagcagccaacgccugguggauguaacgcucaguggugcauuggacaaccaggggagcggugcacuggucagcgaagagucgcugacagugaaggccgaccaggucaauaaccaggcggggacuuucuccagugcggguagccugcucguuaccagccggggcgaguugaacaaccaggguggcagguuggugaccgaugcuggagccacccugaacagcacuggcuucgacaacagccgugcgggccuggucagugcgaaaggggcuguggccauucguaccggagcccugaacaacagucagaagggauccauuggcggcaauacgggcgucacccuggucgccggguuggucgacaacggccgggaaggacggaucagcaccaaggguacgcucgacgccaaccugaaaggguugcuucagcaggggggaggcucgcuggucggcgagcgcggugucacccucgaccucaacgguggcacccuggacaaccacgaccucggucugguuucaacgccuggcgcgcuccugcugcgccaacucggcaugguggacaacagcgucggcggagagauauccagcgaccgugcuuuuacccucgccgccaacacacugaacaaucagggcgggcggcugaucagcagcgaagcuuugacccugcgcaucgccaagacacuggacaacagucucaaggggcagguccuggcgaccgacggacuggccaucgagucucaggucuuggacaaccgugcgggaaccaucggcagcaagggugaugcccguaucagcgugaccagccuggacaacgccgaacaaggcagccuggugagugaaggccgccuggagcuuguagccgaccaggugagcaacggcaaccaaggccguaucgccgccagaggcgugcuggaggcggcggucgguacgcugcuccagcaaggcggcgaacuggucagccaggggagccuggaccuucgcgccgacacgcucgacaacagccaguccgggcugaucgccgcgaauggcggcaucgcuaucgaggcgcggcaggucgacaaccgcgccggcgagauuuccagcaccucgaaggucgccgugaacgcccgcgagcaacuggacaaccgcggcggcaaggucaucggcgacagcggccugcgccucaccgugcagcgccugcugaaccaggccaagggggugcuggccgggcgcgacggccugagccuggacggcggcgaacuguucaacggcgacggcggucggcucgacagccagaacagccugagcgugagccucggcggcgugcuggacaaccagggcggcgcgcuggucagcgaaggcagccugacggcgcgcgccgcgcgccuggacaaccguggcgggaccuucuccagcgccggugcgcuggcgcugaccagccaggccgugcuggacaaccagggcggcaggcugcucagcgaugccggugugacgcugaagggcgccagccucgacaacagccguuccggcgugaucagcgccaagggagcgguggauauccgcaccggcguacuggacaacagccgcaacggcggcaucggcagcaacgccggcaucacccugguggccgcccggcuggacaacggccagcagggccgggucagcgccaagggccugcucgacgccaaccugaaaggccucgaccagcgcggaggcggcguucuggucagcgaaaccggcgucacccucgaccucaauggcggcacgcuggucaaccgcgacggcggcuugaucgccacgcccggcgcgcugcugcugcgccagcucggcgcgguggacaacggcgccggcggggaaaucuccagcgaccgcgccuucacccucgccgccgccagccuggacaaccgcggcgggcgccugaucggcgccgacagccugacccugcgcaucgcccaggcccuggacaacagccuggccggggugaucuccggcgccgccggccuggacaucgcggccgcucgccuggacaacagcgccaagggcacccuggccagucgcgccggcaucgaccugcgcgucgacggcgcgcuggacaaccacgccgaaggcaccgucuccggcgcccgccugacgcucgccagcgccucgcuggacaacagcggcaagggccugcucuccggcaacgccggccugagcgucgccacuggcgcgcuggacaacgccgaggguggccaguugaucagccagggcguccuggacgucagcagcgccgaccucgacaaccguggcggcgcccucaguggcaagcagucgcugcgccugagcgccgccaaccuggacaaccguggcggccugcucaccagcgacggcgaacuggaacugacggcagggcgcgucgauuccgccgacggcggcgaaaucuccgcccggggcgaccugcgccugacggucgagcgccuggugcaacgccagggccggcugauuggcgagcgcggcgucagucucgaccugcggggcggcgaccuggacaaccagggcggccugaucagugcccgcggcccgcugagcaucgagcggcugaacguccucgacaaccgccagggcggcgagauuuacagccagcagggcuucgagcugcuggccaggcgcaucgacaacggccagcaggggcgcaucaucagcgccgggaaacugcgccuggacgccgacgcgcugggcaacgccggcgccggccugcucuccggauggcagggccugacggugacaggcgggagccuggacaacagcgccggcggcacccuuucgagcaaggacggcgagcuggccaucagccucggcggcgcgcuggacaaccacggccagggcgcgcuggucagcaagggcgcgcaacggaucgacgccgccagccuggauaacgcccagggcaucgucuccggcgaaagcgacgugacccugagcaucgccgggaagcuggacaacggccagggcggccuggucucggcgcagcgcgcgcugagcuucgagcgcgacgauacgcugcugaacaacgccggcggccggaucaacggcggcagccugcugcucaagggcgccagccuggauaacagcgacggccaguugaucagccagggccggcucgacgccauccucggcggcgcccuggucaacgccggcgcggcgcgccuggccagcggcggcgaccugcugcugcgcagcgccagcgucgacaaccgcggcggcaagcuggucagccaggggcugcuggagaucagcgccggcagccucgacaacagcgccuccggcacccucgccagccaggccgacaugagccugcgccugggcggcggcgcccugcgcaaccagcaggacggccugaucuucagccaggccggcgcccucgaggugcaggccggcagccuggacaaccgccagggcacgcuccaggcccagggcgacaaccggcugcguaucgguggcgcgcuggacaaccaggccggccgccuggacagccgggccggcaaccucgaccugcagagcggcagccucgacaacggcgccggcggcgugcucaacagcgccaaggguuggcugaagcuggucaccgggcuguucgacaacagcgccggcgucacccaggcgcagucgcuggagauucgcgccgggcaaggcgugcgcaaccagcagggccaucucucggcgcugggcggcgacaaccgcaucgucaccgccgacuucgacaaccagggcggcggccucuacgccagcggccugcucagccucgacggccagcgcuuccucaaccagggcgcggcggcgggccagggcggcaaggucggcgccgggcgcaucgacuucagccuggccggcgcgcuggccaaccgcuucggccaguuggaaagcgagagcgagcugcaccugcgcgccgccgcgaucgacaacagcggcggcagccugcgcgcccucggccgcagcggcagcacgcggcuggucgcuggcgaccugaacaacgccuacggcgugcuggaaagcgccaaccaggaccucgaccugcaacugggcagccuggccaacgccggcgggcgcauccuccacacuggcaacggcaccuucggccuggauuccgggcaggugauccgcgccggcggcgaacugaccaccaauggccugcuggacauccgugccagcgaauggaccaacagcagcgugcugcaagccggacgccugaaccuggacaucggcaccuuccgccagacggccgagggcaagcugcuggcggugcaguccuucacuggccgcggcggcgacuggagcaacgacggccugcuggccagcaacggcagcuugcgacucgagcugagcggcggcuaccguggcaacggccgcgccaccagccucggcgacuucgcccugaacgccgccagccucgaccucggcaaugccgccagccucgccggcggcgccaaugucacgcuuggcgccggcaaccugcuggucaaccgugggcggaucaccgcugccggcgaccucguggccagcgccgcgagccugaacaacuacggcacccugggcggcggcggcaaccugcgauugaacgcgcccgcccugcucaacgagcgcggguugcuguucaguggcgccgacaugacccugcgcgccggcgacaucaccaaccucuacggggauguguacagccucggcaggcuggauaucgcccgcgacgaugcggggggcugggcaaaucgcuuggagaacauuuccgggaauuuagagagcacaggugauaugcguuucuccgugaguucacuucucaauagaagggaaacucuagagauugaaggugacuugcagaauagcgcuauuggcguccgcuguacggggugucagcuuucugagagguggggaaaaacuaggucuucgagcgagcuugucuggaucagggaauauaagucuacauugggagauucuucugccgcugcuucaauuacggcuggucgagaucugcuuguuguaggugcaagccugcagaauauugcuucuaauauaagugcuguaagagacgccacgcuaucucugaguaauuucgaaaacaaagguuaugcguuaggggaauaugcggucaggggcguuuauucgccgccgaguaaauuuggcgaagaauugcuuaugcgcauauuggcguauaacgcugucaacgaucccaguuauggggagggauaugcgagcacaggggggagacuuccgaauauucauuauuucgacaagaauuuuaaugaaaaagucucuccgcuggaggucauucauggaaacgggaaaaauggugggccggguuggcaccuguacuucgguaccuuagauguugaguauccggacacagaucgcuggaauaaggcuauuggacgaauaccggcgccgaauuauucaucgaaaaaaacggaugcuauuccagaucuacuuaagggauuggcuccucucgaugaguugacgauuaacaaaggggcgaacucaacgguuggugcugucgugcaagcuggcggucguguaacggugaaugcugcggagaguuucaauaauucuguccuacagggauuucaggccguucaggaaacccaguuaccucaucaggacauagcuguuucaagcacgacgagcgccguagugacucugaagagucaacugccagcggauuuggcaaggcaacagaucaauccucucacccugccgggcuucagccugccucaaggccagaaugggcucuuccgccuggcgucccaaggagcccaggugaaccaggcaaguggugcucugaaauccgccagcgaucucacccagagcggccauggcguaucuguauccgcacagacaggcaguggcgcaaguggcuggaguacccaggcgcgucgugucggcgaugaucgggucaccucgcuugccgguuccgccuaucaaggccggguagcugaggcuaucgaugcgcuacgggcuuccgcgccaaucucgggcgacgggggaaacacuggccguuuccaggccggugagcaccaggcgaccacgggacuggguggacucgucgagggcaaugcaucgggucacagcggcaauggcgucauccucgccgaucugcgcgguggucuacccucguucucaagccuucccgcgucugaucauguucaaggcacagugcccggucacgaugggaauggaacuauucucgccaauuggcagggugcgcaggcgacgguccaggccucgccuucgacagugcguguagaggggguagucuccaguccagguggcaauggcagcauccuugccgaucugccggcugaacagucgucggugcaggcacugccuucggccguuagggcucagggcagccugccucgccucgaagagcggagcgcccuucuugccgagccuccgguugggcagccggcguugcaaacccugccgucgguugcgcgcguugagggcgugcccagcaaugccacaccgagcaacagccacaaguaucugaucgagaccaacccggcgcucaccgagcugaagcaguuccucaacucggacuaccugcucgguggucuggguaucaauccggacgauagcaagaagcgccugggugacggucuauacgagcagcgccugguacgcgaagcgaucguccagcguacggggcagcgcuucaucgccggauugaacagcgacgaagcgauguuccgcuaucugauggacaacgccaucgccagcaaggacguauugggacugaccccuggcgucacccucagcgccgcccagguggcggcgcugacccacgauaucguuuggcuggaagaagucgaggugaauggcgaaaagguccucgcccccguggucuaccuggcccaggccgaggggcgguugggcccgaacggcgcgcugauccaggggcgcgacgugaaccugaucaccggcggggaccugaggaacgccgguacccugcgcgcgcagaacgaccucagcgcgacagccggcaacaucgacaacagcggccugaucgaggccggcaaccgccucgaccugcuggccagcggcuccauccgcaaugaccagggcggcaucauugccgggcgcgagguaagccucucugcccuuaccggagacgucaucaaugaacggacggugacccagcaccaguccuccuacaggggaaccgguaccacugaggcauuugccgauagcgccgcgcguaucgaggcugcgcagaagcugaccguuucggcaggacgcgauguagccaauauuggcggugucaucgacagcaagggcgaccucgccuugcaaggcggcagggauguccugguuucggcugcgguagcggagcggggcuggacggcaggaagccaggcauaccagacccagacgacccagaugggcgccgaggucguggcggggcgcgauaucagcgucagcgccggacgcgauaucagcgucgugggcagccgcaucgacgcucgucgcgacgugacauucgaggcgggucgcgaugugggccuggucgcggcugccaacgaagagcaugccuauggcaagaccaagaaggucacuuuccaggacgacaagaucacccagcaggccacucgcguggacgcuggcggcgaccuggcgaucaaugccggacaggaccugcggcuggucgcgagccaggccagcgccggcgacgaagccuaccugguggccggcgacaagcuggagcugcuggccgcgaacgacagcaguuacuaccucuacgacaagaagagcaaaggcagcuucgguagcaagaagacccggcgcgacgaaaucaccgaugugacggcagugggcagccaaauauccagcggcggcgaccucacccugcucaguggcggcgaccagacuuaccagggcgcgaagcuggaaucgggcaacgaccuggccaucgucagcggcggcgcggugaccuucgaggcgguaaaggaccugcaccaggaaagccacgagaagagcaagggcgaccuggcguggcagucgucgaagggcaagggccagaccgacgaaaccgugcgccagagccagaucguggcccaggggaaucuggcgaucaaggccguggaagggcugaagaucgaccucaagcacaucgaccagaagaccgugagccagaccaucgacgcgauggugcaggcggauccgcaacuggccuggcugaagcagauggagcagcgcggcgauguggauuggcggcgcgugcaggaacugcaugacagcuggaaguacagcaacuccgggcugggcgucggcgcgcaguuggcgauagcgaucguuguggccuacuucacggcgggugcggcgagugcggcauugggaucgauggcgggagugggggcgggcucaggaagcaugauggcugcugccgguagcacugcaaugguccaggccgguacagcaguaggaacagcugccgccggcugggcgaaugcagcuggaacugccguggcuaugggcauggccagcaauggagcgaucagcaccaucaacaaccggggaaaccugggggaugucgucaaggacgugaccuccagcgaugcgcugaggggcuauguagucgcuggcacgacugcggggcugacugccggcgucuacgacaaauggaccucgacccagaccggcaccucgaccgcucuaccgaacaccggggccguggcgcccgccgcaggguugggcaccuggcaaggcgugggccaguucaccucgaaccaguugcugcagaaugguacuucggugcuguuggaccgggcgcugggcggcaagggcagccugggcgaugcguugcaaaacagccuggcaaaugccuuugcggccuacggcuucaagcugauuggcgacaccacccauggcgugcuggacgacggcagccucggcaagaucggcuugcacgcccugaugggaggucuggccgccgaagcggucgguggcgauuuccguaccggagcccuggcugcgggagucaacgaggcgcugguggauagccucgccaagcaauacgccagccugcccaucgaugacaagaagggccugcugaucaugaguucgcaguugaucggcgugcuggcggcuucgacgcagggcgaugcggacgccaagagcuugcagacgggggccuggguggcggggaaugccacccaacacaacuaccucagucauuggcaggaggagaagaagcggcaggaggucgauggcugcaaagacaaacagcucugcaaaaccggaauagaagccaaaugggcaauuauuucggcccagcaggaugucgguaucgucguagguguuggaggaggcaucggucuuucgacagcugaaaccgcaguggguguuuaugagcuggucaagaacuggagggaaaccuaugcagcucuggagcaguuggccacuucgccagaguuccggcagcaauuuggcgauaacuaccugaaggggcuggaggagcgcgccgcauucuugacccaggcauacgaggaugccggcuggcaagguucggucacagcuggugucgagggcgguagguucgcugcggaacuuguuggcguucugacggcagugaaagguggcgcgcagauaaccgccaagcugccaacagcagccaagaaccuggucaacgcgauugcggagucaccuguuuccgguaguaugaguucgcagcuuggggcagugggggauuugggucggcugggugggggagguaaagguuaugucgauauucuuucccacgaagcuaaacagcauauuuuguauggcgacaaaccugggagugguggccauuuguggccggggcaggcagggaagacaguuuucccucaaaacuggucggcagauaagauaguucacgagguuggugauauugcgacguccccuaguaccaaaugguaugcccaaacaggaacuggugggguuuauacaagcaagggugaucccgcuaaauggguugcuuaugagguucgugauggaguucguaugcgcguuguuuaucagcccgcuacaggaaaggugaucacagccuuccccgacaacgcaccuaucccaccuuauaagcccauuaaauag